European Patent Specification EP 3 455 376 B1, published July 31, 2024. Title: A method for producing a DNA probe and a method for analyzing genomic DNA using the DNA probe. Applicant: TOYOTA JIDOSHA KABUSHIKI KAISHA. The sequence listing filed with the application follows.

SEQUENCE LISTING (2046 sequences)

SEQ ID NO: 1 - DNA, 10 bp, Artificial
  synthetic DNA
agacgtcgtt

SEQ ID NO: 2 - DNA, 10 bp, Artificial
  synthetic DNA
gaggcgatat

SEQ ID NO: 3 - DNA, 10 bp, Artificial
  synthetic DNA
gtgcgaacgt

SEQ ID NO: 4 - DNA, 10 bp, Artificial
  synthetic DNA
ttatactgcc

SEQ ID NO: 5 - DNA, 10 bp, Artificial
  synthetic DNA
caagttcgca

SEQ ID NO: 6 - DNA, 10 bp, Artificial
  synthetic DNA
acaaggtagt

SEQ ID NO: 7 - DNA, 10 bp, Artificial
  synthetic DNA
acacagcgac

SEQ ID NO: 8 - DNA, 10 bp, Artificial
  synthetic DNA
ttaccgatgt

SEQ ID NO: 9 - DNA, 10 bp, Artificial
  synthetic DNA
cacagagtcg

SEQ ID NO: 10 - DNA, 10 bp, Artificial
  synthetic DNA
ttcagcgcgt

SEQ ID NO: 11 - DNA, 10 bp, Artificial
  synthetic DNA
aggaccgtga

SEQ ID NO: 12 - DNA, 10 bp, Artificial
  synthetic DNA
gtctgttcgc

SEQ ID NO: 13 - DNA, 10 bp, Artificial
  synthetic DNA
acctgtccac

SEQ ID NO: 14 - DNA, 10 bp, Artificial
  synthetic DNA
ccgcaatgac

SEQ ID NO: 15 - DNA, 10 bp, Artificial
  synthetic DNA
ctgccgatca

SEQ ID NO: 16 - DNA, 10 bp, Artificial
  synthetic DNA
tacacggagc

SEQ ID NO: 17 - DNA, 10 bp, Artificial
  synthetic DNA
ccgcattcat

SEQ ID NO: 18 - DNA, 10 bp, Artificial
  synthetic DNA
gactctagac

SEQ ID NO: 19 - DNA, 10 bp, Artificial
  synthetic DNA
ggagaactta

SEQ ID NO: 20 - DNA, 10 bp, Artificial
  synthetic DNA
tccggtatgc

SEQ ID NO: 21 - DNA, 10 bp, Artificial
  synthetic DNA
ggtcaggagt

SEQ ID NO: 22 - DNA, 10 bp, Artificial
  synthetic DNA
acattggcag

SEQ ID NO: 23 - DNA, 10 bp, Artificial
  synthetic DNA
cgtagactgc

SEQ ID NO: 24 - DNA, 10 bp, Artificial
  synthetic DNA
agactgtact

SEQ ID NO: 25 - DNA, 10 bp, Artificial
  synthetic DNA
tagacgcagt

SEQ ID NO: 26 - DNA, 10 bp, Artificial
  synthetic DNA
ccgataatct

SEQ ID NO: 27 - DNA, 10 bp, Artificial
  synthetic DNA
gagagctagt

SEQ ID NO: 28 - DNA, 10 bp, Artificial
  synthetic DNA
gtaccgcgtt

SEQ ID NO: 29 - DNA, 10 bp, Artificial
  synthetic DNA
gacttgcgca

SEQ ID NO: 30 - DNA, 10 bp, Artificial
  synthetic DNA
cgtgattgcg

SEQ ID NO: 31 - DNA, 10 bp, Artificial
  synthetic DNA
atcgtctctg

SEQ ID NO: 32 - DNA, 10 bp, Artificial
  synthetic DNA
cgtagctacg

SEQ ID NO: 33 - DNA, 10 bp, Artificial
  synthetic DNA
gccgaatagt

SEQ ID NO: 34 - DNA, 10 bp, Artificial
  synthetic DNA
gtacctaggc

SEQ ID NO: 35 - DNA, 10 bp, Artificial
  synthetic DNA
gcttacatga

SEQ ID NO: 36 - DNA, 10 bp, Artificial
  synthetic DNA
tccacgtagt

SEQ ID NO: 37 - DNA, 10 bp, Artificial
  synthetic DNA
agaggccatc

SEQ ID NO: 38 - DNA, 10 bp, Artificial
  synthetic DNA
cggtgatgct

SEQ ID NO: 39 - DNA, 10 bp, Artificial
  synthetic DNA
cactgtgctt

SEQ ID NO: 40 - DNA, 10 bp, Artificial
  synthetic DNA
catgatggct

SEQ ID NO: 41 - DNA, 10 bp, Artificial
  synthetic DNA
gccacacatg

SEQ ID NO: 42 - DNA, 10 bp, Artificial
  synthetic DNA
cacacactgt

SEQ ID NO: 43 - DNA, 10 bp, Artificial
  synthetic DNA
cagaatcata

SEQ ID NO: 44 - DNA, 10 bp, Artificial
  synthetic DNA
atcgtctacg

SEQ ID NO: 45 - DNA, 10 bp, Artificial
  synthetic DNA
cgagcaatac

SEQ ID NO: 46 - DNA, 10 bp, Artificial
  synthetic DNA
acaagcgcac

SEQ ID NO: 47 - DNA, 10 bp, Artificial
  synthetic DNA
gcttagatgt

SEQ ID NO: 48 - DNA, 10 bp, Artificial
  synthetic DNA
tgcattctgg

SEQ ID NO: 49 - DNA, 10 bp, Artificial
  synthetic DNA
tgtcggacca

SEQ ID NO: 50 - DNA, 10 bp, Artificial
  synthetic DNA
aggcactcgt

SEQ ID NO: 51 - DNA, 10 bp, Artificial
  synthetic DNA
ctgcatgtga

SEQ ID NO: 52 - DNA, 10 bp, Artificial
  synthetic DNA
accacgccta

SEQ ID NO: 53 - DNA, 10 bp, Artificial
  synthetic DNA
gaggtcgtac

SEQ ID NO: 54 - DNA, 10 bp, Artificial
  synthetic DNA
aatactctgt

SEQ ID NO: 55 - DNA, 10 bp, Artificial
  synthetic DNA
tgccaactga

SEQ ID NO: 56 - DNA, 10 bp, Artificial
  synthetic DNA
cctgttcggt

SEQ ID NO: 57 - DNA, 10 bp, Artificial
  synthetic DNA
gtagagagtt

SEQ ID NO: 58 - DNA, 10 bp, Artificial
  synthetic DNA
tacagcgtaa

SEQ ID NO: 59 - DNA, 10 bp, Artificial
  synthetic DNA
tgacgtgatg

SEQ ID NO: 60 - DNA, 10 bp, Artificial
  synthetic DNA
agacgtcggt

SEQ ID NO: 61 - DNA, 10 bp, Artificial
  synthetic DNA
cgctaggttc

SEQ ID NO: 62 - DNA, 10 bp, Artificial
  synthetic DNA
gccttatagc

SEQ ID NO: 63 - DNA, 10 bp, Artificial
  synthetic DNA
ccttcgatct

SEQ ID NO: 64 - DNA, 10 bp, Artificial
  synthetic DNA
aggcaacgtg

SEQ ID NO: 65 - DNA, 10 bp, Artificial
  synthetic DNA
tgagcggtgt

SEQ ID NO: 66 - DNA, 10 bp, Artificial
  synthetic DNA
gtgtcgaacg

SEQ ID NO: 67 - DNA, 10 bp, Artificial
  synthetic DNA
cgatgttgcg

SEQ ID NO: 68 - DNA, 10 bp, Artificial
  synthetic DNA
aacaagacac

SEQ ID NO: 69 - DNA, 10 bp, Artificial
  synthetic DNA
gatgctggtt

SEQ ID NO: 70 - DNA, 10 bp, Artificial
  synthetic DNA
accggtagtc

SEQ ID NO: 71 - DNA, 10 bp, Artificial
  synthetic DNA
gtgactagca

SEQ ID NO: 72 - DNA, 10 bp, Artificial
  synthetic DNA
agcctatatt

SEQ ID NO: 73 - DNA, 10 bp, Artificial
  synthetic DNA
tcgtgagctt

SEQ ID NO: 74 - DNA, 10 bp, Artificial
  synthetic DNA
acactatggc

SEQ ID NO: 75 - DNA, 10 bp, Artificial
  synthetic DNA
gactctgtcg

SEQ ID NO: 76 - DNA, 10 bp, Artificial
  synthetic DNA
tcgatgatgc

SEQ ID NO: 77 - DNA, 10 bp, Artificial
  synthetic DNA
cttggacact

SEQ ID NO: 78 - DNA, 10 bp, Artificial
  synthetic DNA
ggctgatcgt

SEQ ID NO: 79 - DNA, 10 bp, Artificial
  synthetic DNA
actcacaggc

SEQ ID NO: 80 - DNA, 10 bp, Artificial
  synthetic DNA
atgtgcgtac

SEQ ID NO: 81 - DNA, 10 bp, Artificial
  synthetic DNA
caccatcgat

SEQ ID NO: 82 - DNA, 10 bp, Artificial
  synthetic DNA
agccattaac

SEQ ID NO: 83 - DNA, 10 bp, Artificial
  synthetic DNA
aatcgactgt

SEQ ID NO: 84 - DNA, 10 bp, Artificial
  synthetic DNA
aatactagcg

SEQ ID NO: 85 - DNA, 10 bp, Artificial
  synthetic DNA
tcgtcactga

SEQ ID NO: 86 - DNA, 10 bp, Artificial
  synthetic DNA
caggctctta

SEQ ID NO: 87 - DNA, 10 bp, Artificial
  synthetic DNA
ggtcggtgat

SEQ ID NO: 88 - DNA, 10 bp, Artificial
  synthetic DNA
cattaggcgt

SEQ ID NO: 89 - DNA, 10 bp, Artificial
  synthetic DNA
actcgcgagt

SEQ ID NO: 90 - DNA, 10 bp, Artificial
  synthetic DNA
ttccgaataa

SEQ ID NO: 91 - DNA, 10 bp, Artificial
  synthetic DNA
tgagcatcgt

SEQ ID NO: 92 - DNA, 10 bp, Artificial
  synthetic DNA
gccacgtaac

SEQ ID NO: 93 - DNA, 10 bp, Artificial
  synthetic DNA
gaactacatg

SEQ ID NO: 94 - DNA, 10 bp, Artificial
  synthetic DNA
tcgtgaggac

SEQ ID NO: 95 - DNA, 10 bp, Artificial
  synthetic DNA
gcggccttaa

SEQ ID NO: 96 - DNA, 10 bp, Artificial
  synthetic DNA
gctaaggacc

SEQ ID NO: 97 - DNA, 10 bp, Artificial
  synthetic DNA
atagccatta

SEQ ID NO: 98 - DNA, 10 bp, Artificial
  synthetic DNA
cagtaatcat

SEQ ID NO: 99 - DNA, 10 bp, Artificial
  synthetic DNA
actccttaat

SEQ ID NO: 100 - DNA, 10 bp, Artificial
  synthetic DNA
tcgaacatta

SEQ ID NO: 101 - DNA, 10 bp, Artificial
  synthetic DNA
attatgaggt

SEQ ID NO: 102 - DNA, 10 bp, Artificial
  synthetic DNA
aatcttagag

SEQ ID NO: 103 - DNA, 10 bp, Artificial
  synthetic DNA
ttagatgatg

SEQ ID NO: 104 - DNA, 10 bp, Artificial
  synthetic DNA
tacatatctg

SEQ ID NO: 105 - DNA, 10 bp, Artificial
  synthetic DNA
tccttaatca

SEQ ID NO: 106 - DNA, 10 bp, Artificial
  synthetic DNA
gttgagatta

SEQ ID NO: 107 - DNA, 10 bp, Artificial
  synthetic DNA
tgttaacgta

SEQ ID NO: 108 - DNA, 10 bp, Artificial
  synthetic DNA
catacagtaa

SEQ ID NO: 109 - DNA, 10 bp, Artificial
  synthetic DNA
cttatacgaa

SEQ ID NO: 110 - DNA, 10 bp, Artificial
  synthetic DNA
agatctatgt

SEQ ID NO: 111 - DNA, 10 bp, Artificial
  synthetic DNA
aagacttagt

SEQ ID NO: 112 - DNA, 10 bp, Artificial
  synthetic DNA
tgcgcaataa

SEQ ID NO: 113 - DNA, 10 bp, Artificial
  synthetic DNA
ttggccatat

SEQ ID NO: 114 - DNA, 10 bp, Artificial
  synthetic DNA
tattacgagg

SEQ ID NO: 115 - DNA, 10 bp, Artificial
  synthetic DNA
ttatgatcgc

SEQ ID NO: 116 - DNA, 10 bp, Artificial
  synthetic DNA
aacttaggag

SEQ ID NO: 117 - DNA, 10 bp, Artificial
  synthetic DNA
tcacaatcgt

SEQ ID NO: 118 - DNA, 10 bp, Artificial
  synthetic DNA
gagtatatgg

SEQ ID NO: 119 - DNA, 10 bp, Artificial
  synthetic DNA
atcaggacaa

SEQ ID NO: 120 - DNA, 10 bp, Artificial
  synthetic DNA
gtactgatag

SEQ ID NO: 121 - DNA, 10 bp, Artificial
  synthetic DNA
cttatactcg

SEQ ID NO: 122 - DNA, 10 bp, Artificial
  synthetic DNA
taacggacta

SEQ ID NO: 123 - DNA, 10 bp, Artificial
  synthetic DNA
gcgttgtata

SEQ ID NO: 124 - DNA, 10 bp, Artificial
  synthetic DNA
cttaagtgct

SEQ ID NO: 125 - DNA, 10 bp, Artificial
  synthetic DNA
atacgactgt

SEQ ID NO: 126 - DNA, 10 bp, Artificial
  synthetic DNA
actgttatcg

SEQ ID NO: 127 - DNA, 10 bp, Artificial
  synthetic DNA
aatcttgacg

SEQ ID NO: 128 - DNA, 10 bp, Artificial
  synthetic DNA
acatcacctt

SEQ ID NO: 129 - DNA, 10 bp, Artificial
  synthetic DNA
ggtatagtac

SEQ ID NO: 130 - DNA, 10 bp, Artificial
  synthetic DNA
ctaatccaca

SEQ ID NO: 131 - DNA, 10 bp, Artificial
  synthetic DNA
gcaccttatt

SEQ ID NO: 132 - DNA, 10 bp, Artificial
  synthetic DNA
attgacggta

SEQ ID NO: 133 - DNA, 10 bp, Artificial
  synthetic DNA
gacatatggt

SEQ ID NO: 134 - DNA, 10 bp, Artificial
  synthetic DNA
gatagtcgta

SEQ ID NO: 135 - DNA, 10 bp, Artificial
  synthetic DNA
caattatcgc

SEQ ID NO: 136 - DNA, 10 bp, Artificial
  synthetic DNA
cttaggtgat

SEQ ID NO: 137 - DNA, 10 bp, Artificial
  synthetic DNA
catactactg

SEQ ID NO: 138 - DNA, 10 bp, Artificial
  synthetic DNA
taacgcgaat

SEQ ID NO: 139 - DNA, 10 bp, Artificial
  synthetic DNA
caagttacga

SEQ ID NO: 140 - DNA, 10 bp, Artificial
  synthetic DNA
aatctcaagg

SEQ ID NO: 141 - DNA, 10 bp, Artificial
  synthetic DNA
gcaatcatca

SEQ ID NO: 142 - DNA, 10 bp, Artificial
  synthetic DNA
tgtaacgttc

SEQ ID NO: 143 - DNA, 10 bp, Artificial
  synthetic DNA
tatcgttggt

SEQ ID NO: 144 - DNA, 10 bp, Artificial
  synthetic DNA
cgcttaagat

SEQ ID NO: 145 - DNA, 10 bp, Artificial
  synthetic DNA
ttagaactgg

SEQ ID NO: 146 - DNA, 10 bp, Artificial
  synthetic DNA
gtcataacgt

SEQ ID NO: 147 - DNA, 10 bp, Artificial
  synthetic DNA
agagcagtat

SEQ ID NO: 148 - DNA, 10 bp, Artificial
  synthetic DNA
caacatcact

SEQ ID NO: 149 - DNA, 10 bp, Artificial
  synthetic DNA
cagaagctta

SEQ ID NO: 150 - DNA, 10 bp, Artificial
  synthetic DNA
aactaacgtg

SEQ ID NO: 151 - DNA, 10 bp, Artificial
  synthetic DNA
ttataccgct

SEQ ID NO: 152 - DNA, 10 bp, Artificial
  synthetic DNA
gaattcgaga

SEQ ID NO: 153 - DNA, 10 bp, Artificial
  synthetic DNA
ttacgtaacc

SEQ ID NO: 154 - DNA, 10 bp, Artificial
  synthetic DNA
gcatggttaa

SEQ ID NO: 155 - DNA, 10 bp, Artificial
  synthetic DNA
gcacctaatt

SEQ ID NO: 156 - DNA, 10 bp, Artificial
  synthetic DNA
tgtaggttgt

SEQ ID NO: 157 - DNA, 10 bp, Artificial
  synthetic DNA
ccatctggaa

SEQ ID NO: 158 - DNA, 10 bp, Artificial
  synthetic DNA
ttcgcgttga

SEQ ID NO: 159 - DNA, 10 bp, Artificial
  synthetic DNA
aaccgaggtt

SEQ ID NO: 160 - DNA, 10 bp, Artificial
  synthetic DNA
gtacgctgtt

SEQ ID NO: 161 - DNA, 10 bp, Artificial
  synthetic DNA
agtatcctgg

SEQ ID NO: 162 - DNA, 10 bp, Artificial
  synthetic DNA
ggttgtacag

SEQ ID NO: 163 - DNA, 10 bp, Artificial
  synthetic DNA
acgtacacca

SEQ ID NO: 164 - DNA, 10 bp, Artificial
  synthetic DNA
tgtcgagcaa

SEQ ID NO: 165 - DNA, 10 bp, Artificial
  synthetic DNA
gtcgtgttac

SEQ ID NO: 166 - DNA, 10 bp, Artificial
  synthetic DNA
gtgcaatagg

SEQ ID NO: 167 - DNA, 10 bp, Artificial
  synthetic DNA
actcgatgct

SEQ ID NO: 168 - DNA, 10 bp, Artificial
  synthetic DNA
gaatcgcgta

SEQ ID NO: 169 - DNA, 10 bp, Artificial
  synthetic DNA
cggtcattgt

SEQ ID NO: 170 - DNA, 10 bp, Artificial
  synthetic DNA
atcaggcgat

SEQ ID NO: 171 - DNA, 10 bp, Artificial
  synthetic DNA
gtaagatgcg

SEQ ID NO: 172 - DNA, 10 bp, Artificial
  synthetic DNA
ggtctcttga

SEQ ID NO: 173 - DNA, 10 bp, Artificial
  synthetic DNA
tcctcgctaa

SEQ ID NO: 174 - DNA, 10 bp, Artificial
  synthetic DNA
ctgcgtgata

SEQ ID NO: 175 - DNA, 10 bp, Artificial
  synthetic DNA
catactcgtc

SEQ ID NO: 176 - DNA, 10 bp, Artificial
  synthetic DNA
atctgagctc

SEQ ID NO: 177 - DNA, 10 bp, Artificial
  synthetic DNA
acggatagtg

SEQ ID NO: 178 - DNA, 10 bp, Artificial
  synthetic DNA
actgcaatgc

SEQ ID NO: 179 - DNA, 10 bp, Artificial
  synthetic DNA
taacgacgtg

SEQ ID NO: 180 - DNA, 10 bp, Artificial
  synthetic DNA
tagactgtcg

SEQ ID NO: 181 - DNA, 10 bp, Artificial
  synthetic DNA
cagcacttca

SEQ ID NO: 182 - DNA, 10 bp, Artificial
  synthetic DNA
aacattcgcc

SEQ ID NO: 183 - DNA, 10 bp, Artificial
  synthetic DNA
actagtgcgt

SEQ ID NO: 184 - DNA, 10 bp, Artificial
  synthetic DNA
acgctgttct

SEQ ID NO: 185 - DNA, 10 bp, Artificial
  synthetic DNA
cgtcgaatgc

SEQ ID NO: 186 - DNA, 10 bp, Artificial
  synthetic DNA
ctctgacggt

SEQ ID NO: 187 - DNA, 10 bp, Artificial
  synthetic DNA
gtcgccatgt

SEQ ID NO: 188 - DNA, 10 bp, Artificial
  synthetic DNA
ggtccacgtt

SEQ ID NO: 189 - DNA, 10 bp, Artificial
  synthetic DNA
cgagcgactt

SEQ ID NO: 190 - DNA, 10 bp, Artificial
  synthetic DNA
ttgacgcgtg

SEQ ID NO: 191 - DNA, 10 bp, Artificial
  synthetic DNA
ctgagagcct

SEQ ID NO: 192 - DNA, 10 bp, Artificial
  synthetic DNA
cgcgctaact

SEQ ID NO: 193 - DNA, 10 bp, Artificial
  synthetic DNA
ggtcgtcaag

SEQ ID NO: 194 - DNA, 10 bp, Artificial
  synthetic DNA
aggttgacca

SEQ ID NO: 195 - DNA, 10 bp, Artificial
  synthetic DNA
taacggcaac

SEQ ID NO: 196 - DNA, 10 bp, Artificial
  synthetic DNA
gaggctggat

SEQ ID NO: 197 - DNA, 10 bp, Artificial
  synthetic DNA
gtgcacacct

SEQ ID NO: 198 - DNA, 10 bp, Artificial
  synthetic DNA
tgaggaccag

SEQ ID NO: 199 - DNA, 10 bp, Artificial
  synthetic DNA
tacttgcgag

SEQ ID NO: 200 - DNA, 10 bp, Artificial
  synthetic DNA
aactgtgaga

SEQ ID NO: 201 - DNA, 10 bp, Artificial
  synthetic DNA
ctccatcaac

SEQ ID NO: 202 - DNA, 10 bp, Artificial
  synthetic DNA
cggactgtta

SEQ ID NO: 203 - DNA, 10 bp, Artificial
  synthetic DNA
taggacagtc

SEQ ID NO: 204 - DNA, 10 bp, Artificial
  synthetic DNA
agaggacaca

SEQ ID NO: 205 - DNA, 10 bp, Artificial
  synthetic DNA
acattcgcgg

SEQ ID NO: 206 - DNA, 10 bp, Artificial
  synthetic DNA
gcttactgca

SEQ ID NO: 207 - DNA, 10 bp, Artificial
  synthetic DNA
caatacgtaa

SEQ ID NO: 208 - DNA, 10 bp, Artificial
  synthetic DNA
agacttgcgc

SEQ ID NO: 209 - DNA, 10 bp, Artificial
  synthetic DNA
gagcggtgtt

SEQ ID NO: 210 - DNA, 10 bp, Artificial
  synthetic DNA
cgtgagaggt

SEQ ID NO: 211 - DNA, 10 bp, Artificial
  synthetic DNA
aatccgtcag

SEQ ID NO: 212 - DNA, 10 bp, Artificial
  synthetic DNA
atacgtaccg

SEQ ID NO: 213 - DNA, 10 bp, Artificial
  synthetic DNA
aactgattcc

SEQ ID NO: 214 - DNA, 10 bp, Artificial
  synthetic DNA
ctgagcgtac

SEQ ID NO: 215 - DNA, 10 bp, Artificial
  synthetic DNA
gtcggattcg

SEQ ID NO: 216 - DNA, 10 bp, Artificial
  synthetic DNA
gccgaccata

SEQ ID NO: 217 - DNA, 10 bp, Artificial
  synthetic DNA
gcagaactaa

SEQ ID NO: 218 - DNA, 10 bp, Artificial
  synthetic DNA
ctaacgaccg

SEQ ID NO: 219 - DNA, 10 bp, Artificial
  synthetic DNA
gctggaccat

SEQ ID NO: 220 - DNA, 10 bp, Artificial
  synthetic DNA
gacgcggtta

SEQ ID NO: 221 - DNA, 10 bp, Artificial
  synthetic DNA
agtggtgagc

SEQ ID NO: 222 - DNA, 10 bp, Artificial
  synthetic DNA
caggcagtca

SEQ ID NO: 223 - DNA, 10 bp, Artificial
  synthetic DNA
tctgacgtca

SEQ ID NO: 224 - DNA, 10 bp, Artificial
  synthetic DNA
tacatgacgt

SEQ ID NO: 225 - DNA, 10 bp, Artificial
  synthetic DNA
tgaggcaacc

SEQ ID NO: 226 - DNA, 10 bp, Artificial
  synthetic DNA
caactgcagt

SEQ ID NO: 227 - DNA, 10 bp, Artificial
  synthetic DNA
cggagatacg

SEQ ID NO: 228 - DNA, 10 bp, Artificial
  synthetic DNA
cttcgcaagt

SEQ ID NO: 229 - DNA, 10 bp, Artificial
  synthetic DNA
ctggcatacg

SEQ ID NO: 230 - DNA, 10 bp, Artificial
  synthetic DNA
taacgttcgc

SEQ ID NO: 231 - DNA, 10 bp, Artificial
  synthetic DNA
ccggcgttaa

SEQ ID NO: 232 - DNA, 10 bp, Artificial
  synthetic DNA
acaagacgcc

SEQ ID NO: 233 - DNA, 10 bp, Artificial
  synthetic DNA
ccattagact

SEQ ID NO: 234 - DNA, 10 bp, Artificial
  synthetic DNA
gtctgtgaca

SEQ ID NO: 235 - DNA, 10 bp, Artificial
  synthetic DNA
ggcattggac

SEQ ID NO: 236 - DNA, 10 bp, Artificial
  synthetic DNA
tcttcgcacg

SEQ ID NO: 237 - DNA, 10 bp, Artificial
  synthetic DNA
tagcctgtgc

SEQ ID NO: 238 - DNA, 10 bp, Artificial
  synthetic DNA
cactgaccta

SEQ ID NO: 239 - DNA, 10 bp, Artificial
  synthetic DNA
ccgcacgatt

SEQ ID NO: 240 - DNA, 10 bp, Artificial
  synthetic DNA
atagcacacg

SEQ ID NO: 241 - DNA, 10 bp, Artificial
  synthetic DNA
gcacgtcata

SEQ ID NO: 242 - DNA, 10 bp, Artificial
  synthetic DNA
aagccgttgg

SEQ ID NO: 243 - DNA, 10 bp, Artificial
  synthetic DNA
cggaccgtta

SEQ ID NO: 244 - DNA, 10 bp, Artificial
  synthetic DNA
tacacagcgt

SEQ ID NO: 245 - DNA, 10 bp, Artificial
  synthetic DNA
cggacttcag

SEQ ID NO: 246 - DNA, 10 bp, Artificial
  synthetic DNA
tagaacgtca

SEQ ID NO: 247 - DNA, 10 bp, Artificial
  synthetic DNA
ggcattggag

SEQ ID NO: 248 - DNA, 10 bp, Artificial
  synthetic DNA
ggcactcgtt

SEQ ID NO: 249 - DNA, 10 bp, Artificial
  synthetic DNA
gtaccgttaa

SEQ ID NO: 250 - DNA, 10 bp, Artificial
  synthetic DNA
aatacgtgtc

SEQ ID NO: 251 - DNA, 10 bp, Artificial
  synthetic DNA
ccattgacgt

SEQ ID NO: 252 - DNA, 10 bp, Artificial
  synthetic DNA
cgtgaatcgc

SEQ ID NO: 253 - DNA, 10 bp, Artificial
  synthetic DNA
atcaacgcgg

SEQ ID NO: 254 - DNA, 10 bp, Artificial
  synthetic DNA
cgccaaggta

SEQ ID NO: 255 - DNA, 10 bp, Artificial
  synthetic DNA
agaagacgcc

SEQ ID NO: 256 - DNA, 10 bp, Artificial
  synthetic DNA
ccgcatagtc

SEQ ID NO: 257 - DNA, 10 bp, Artificial
  synthetic DNA
cttatatgtg

SEQ ID NO: 258 - DNA, 10 bp, Artificial
  synthetic DNA
ggtctcatcg

SEQ ID NO: 259 - DNA, 10 bp, Artificial
  synthetic DNA
ccaccatgtc

SEQ ID NO: 260 - DNA, 10 bp, Artificial
  synthetic DNA
acgaatgtgt

SEQ ID NO: 261 - DNA, 10 bp, Artificial
  synthetic DNA
ggtagtaaca

SEQ ID NO: 262 - DNA, 10 bp, Artificial
  synthetic DNA
gccacttaat

SEQ ID NO: 263 - DNA, 10 bp, Artificial
  synthetic DNA
atattgcgcc

SEQ ID NO: 264 - DNA, 10 bp, Artificial
  synthetic DNA
gaccaatagt

SEQ ID NO: 265 - DNA, 10 bp, Artificial
  synthetic DNA
aacaacacgg

SEQ ID NO: 266 - DNA, 10 bp, Artificial
  synthetic DNA
atagccgatg

SEQ ID NO: 267 - DNA, 10 bp, Artificial
  synthetic DNA
cgagagcata

SEQ ID NO: 268 - DNA, 10 bp, Artificial
  synthetic DNA
cgagacatga

SEQ ID NO: 269 - DNA, 10 bp, Artificial
  synthetic DNA
cgccaagtta

SEQ ID NO: 270 - DNA, 10 bp, Artificial
  synthetic DNA
ttataatcgc

SEQ ID NO: 271 - DNA, 10 bp, Artificial
  synthetic DNA
tagaagtgca

SEQ ID NO: 272 - DNA, 10 bp, Artificial
  synthetic DNA
ggaggcatgt

SEQ ID NO: 273 - DNA, 10 bp, Artificial
  synthetic DNA
gccacttcga

SEQ ID NO: 274 - DNA, 10 bp, Artificial
  synthetic DNA
tccacggtac

SEQ ID NO: 275 - DNA, 10 bp, Artificial
  synthetic DNA
caactatgca

SEQ ID NO: 276 - DNA, 10 bp, Artificial
  synthetic DNA
caaggaggac

SEQ ID NO: 277 - DNA, 10 bp, Artificial
  synthetic DNA
gaggtaccta

SEQ ID NO: 278 - DNA, 10 bp, Artificial
  synthetic DNA
gagcgcataa

SEQ ID NO: 279 - DNA, 10 bp, Artificial
  synthetic DNA
tcgtcacgtg

SEQ ID NO: 280 - DNA, 10 bp, Artificial
  synthetic DNA
aactgtgaca

SEQ ID NO: 281 - DNA, 10 bp, Artificial
  synthetic DNA
tccacgtgag

SEQ ID NO: 282 - DNA, 10 bp, Artificial
  synthetic DNA
acactgctct

SEQ ID NO: 283 - DNA, 10 bp, Artificial
  synthetic DNA
tacggtgagc

SEQ ID NO: 284 - DNA, 10 bp, Artificial
  synthetic DNA
cggactaagt

SEQ ID NO: 285 - DNA, 10 bp, Artificial
  synthetic DNA
aagccacgtt

SEQ ID NO: 286 - DNA, 10 bp, Artificial
  synthetic DNA
caattactcg

SEQ ID NO: 287 - DNA, 10 bp, Artificial
  synthetic DNA
tctggccata

SEQ ID NO: 288 - DNA, 10 bp, Artificial
  synthetic DNA
tcaggctagt

SEQ ID NO: 289 - DNA, 10 bp, Artificial
  synthetic DNA
ttgacccgga

SEQ ID NO: 290 - DNA, 10 bp, Artificial
  synthetic DNA
tttttatggt

SEQ ID NO: 291 - DNA, 10 bp, Artificial
  synthetic DNA
atgtggtgcg

SEQ ID NO: 292 - DNA, 10 bp, Artificial
  synthetic DNA
aaggcgctag

SEQ ID NO: 293 - DNA, 10 bp, Artificial
  synthetic DNA
tccaactttg

SEQ ID NO: 294 - DNA, 10 bp, Artificial
  synthetic DNA
ccatcccatc

SEQ ID NO: 295 - DNA, 10 bp, Artificial
  synthetic DNA
caatacgagg

SEQ ID NO: 296 - DNA, 10 bp, Artificial
  synthetic DNA
gagtgttacc

SEQ ID NO: 297 - DNA, 10 bp, Artificial
  synthetic DNA
gcctcctgta

SEQ ID NO: 298 - DNA, 10 bp, Artificial
  synthetic DNA
cgaaggttgc

SEQ ID NO: 299 - DNA, 10 bp, Artificial
  synthetic DNA
gaggtgctat

SEQ ID NO: 300 - DNA, 10 bp, Artificial
  synthetic DNA
taggataatt

SEQ ID NO: 301 - DNA, 10 bp, Artificial
  synthetic DNA
cgttgtcctc

SEQ ID NO: 302 - DNA, 10 bp, Artificial
  synthetic DNA
tgagaccagc

SEQ ID NO: 303 - DNA, 10 bp, Artificial
  synthetic DNA
tgcccaagct

SEQ ID NO: 304 - DNA, 10 bp, Artificial
  synthetic DNA
tactgaatcg

SEQ ID NO: 305 - DNA, 10 bp, Artificial
  synthetic DNA
ttacatagtc

SEQ ID NO: 306 - DNA, 10 bp, Artificial
  synthetic DNA
acaaaggaaa

SEQ ID NO: 307 - DNA, 10 bp, Artificial
  synthetic DNA
ctcgcttggg

SEQ ID NO: 308 - DNA, 10 bp, Artificial
  synthetic DNA
ccttgcgtca

SEQ ID NO: 309 - DNA, 10 bp, Artificial
  synthetic DNA
taattccgaa

SEQ ID NO: 310 - DNA, 10 bp, Artificial
  synthetic DNA
gtgagcttga

SEQ ID NO: 311 - DNA, 10 bp, Artificial
  synthetic DNA
atgccgattc

SEQ ID NO: 312 - DNA, 10 bp, Artificial
  synthetic DNA
gcttgggctt

SEQ ID NO: 313 - DNA, 10 bp, Artificial
  synthetic DNA
acaaagcgcc

SEQ ID NO: 314 - DNA, 10 bp, Artificial
  synthetic DNA
gaaagctcta

SEQ ID NO: 315 - DNA, 10 bp, Artificial
  synthetic DNA
taccgaccgt

SEQ ID NO: 316 - DNA, 10 bp, Artificial
  synthetic DNA
tcgaagagac

SEQ ID NO: 317 - DNA, 10 bp, Artificial
  synthetic DNA
gtcgcttacg

SEQ ID NO: 318 - DNA, 10 bp, Artificial
  synthetic DNA
gggctctcca

SEQ ID NO: 319 - DNA, 10 bp, Artificial
  synthetic DNA
gcgcccttgt

SEQ ID NO: 320 - DNA, 10 bp, Artificial
  synthetic DNA
ggcaataggc

SEQ ID NO: 321 - DNA, 10 bp, Artificial
  synthetic DNA
caagtcagga

SEQ ID NO: 322 - DNA, 10 bp, Artificial
  synthetic DNA
gggtcgcaat

SEQ ID NO: 323 - DNA, 10 bp, Artificial
  synthetic DNA
cagcaaccta

SEQ ID NO: 324 - DNA, 10 bp, Artificial
  synthetic DNA
ttcccgccac

SEQ ID NO: 325 - DNA, 10 bp, Artificial
  synthetic DNA
tgtgcatttt

SEQ ID NO: 326 - DNA, 10 bp, Artificial
  synthetic DNA
atcaacgacg

SEQ ID NO: 327 - DNA, 10 bp, Artificial
  synthetic DNA
gtgacgtcca

SEQ ID NO: 328 - DNA, 10 bp, Artificial
  synthetic DNA
cgatctagtc

SEQ ID NO: 329 - DNA, 10 bp, Artificial
  synthetic DNA
ttacatcctg

SEQ ID NO: 330 - DNA, 10 bp, Artificial
  synthetic DNA
agccttcaat

SEQ ID NO: 331 - DNA, 10 bp, Artificial
  synthetic DNA
tccatccgat

SEQ ID NO: 332 - DNA, 10 bp, Artificial
  synthetic DNA
gactgggtct

SEQ ID NO: 333 - DNA, 10 bp, Artificial
  synthetic DNA
ttcggtggag

SEQ ID NO: 334 - DNA, 10 bp, Artificial
  synthetic DNA
gaccagcaca

SEQ ID NO: 335 - DNA, 10 bp, Artificial
  synthetic DNA
cattaacgga

SEQ ID NO: 336 - DNA, 10 bp, Artificial
  synthetic DNA
tttttcttga

SEQ ID NO: 337 - DNA, 10 bp, Artificial
  synthetic DNA
cattgcactg

SEQ ID NO: 338 - DNA, 10 bp, Artificial
  synthetic DNA
tgcggcgatc

SEQ ID NO: 339 - DNA, 10 bp, Artificial
  synthetic DNA
atattgcggt

SEQ ID NO: 340 - DNA, 10 bp, Artificial
  synthetic DNA
gacgtcgctc

SEQ ID NO: 341 - DNA, 10 bp, Artificial
  synthetic DNA
tcgcttatcg

SEQ ID NO: 342 - DNA, 10 bp, Artificial
  synthetic DNA
gcgcagacac

SEQ ID NO: 343 - DNA, 10 bp, Artificial
  synthetic DNA
catgtattgt

SEQ ID NO: 344 - DNA, 10 bp, Artificial
  synthetic DNA
tctataacct

SEQ ID NO: 345 - DNA, 10 bp, Artificial
  synthetic DNA
gtggagacaa

SEQ ID NO: 346 - DNA, 10 bp, Artificial
  synthetic DNA
cgaagattat

SEQ ID NO: 347 - DNA, 10 bp, Artificial
  synthetic DNA
tagcaactgc

SEQ ID NO: 348 - DNA, 10 bp, Artificial
  synthetic DNA
ataatcggta

SEQ ID NO: 349 - DNA, 10 bp, Artificial
  synthetic DNA
caggatgggt

SEQ ID NO: 350 - DNA, 10 bp, Artificial
  synthetic DNA
gacgattccc

SEQ ID NO: 351 - DNA, 10 bp, Artificial
  synthetic DNA
cacgccttac

SEQ ID NO: 352 - DNA, 10 bp, Artificial
  synthetic DNA
agttggttcc

SEQ ID NO: 353 - DNA, 10 bp, Artificial
  synthetic DNA
tcttatcagg

SEQ ID NO: 354 - DNA, 10 bp, Artificial
  synthetic DNA
cgagaagttc

SEQ ID NO: 355 - DNA, 10 bp, Artificial
  synthetic DNA
gtggtagaat

SEQ ID NO: 356 - DNA, 10 bp, Artificial
  synthetic DNA
taggcttgtg

SEQ ID NO: 357 - DNA, 10 bp, Artificial
  synthetic DNA
atgcgttacg

SEQ ID NO: 358 - DNA, 10 bp, Artificial
  synthetic DNA
actaccgagg

SEQ ID NO: 359 - DNA, 10 bp, Artificial
  synthetic DNA
cgagttggtg

SEQ ID NO: 360 - DNA, 10 bp, Artificial
  synthetic DNA
ggacgatcaa

SEQ ID NO: 361 - DNA, 10 bp, Artificial
  synthetic DNA
aacagtatgc

SEQ ID NO: 362 - DNA, 10 bp, Artificial
  synthetic DNA
ttggctgatc

SEQ ID NO: 363 - DNA, 10 bp, Artificial
  synthetic DNA
aggattggaa

SEQ ID NO: 364 - DNA, 10 bp, Artificial
  synthetic DNA
catatggaga

SEQ ID NO: 365 - DNA, 10 bp, Artificial
  synthetic DNA
ctgcaggttt

SEQ ID NO: 366 - DNA, 10 bp, Artificial
  synthetic DNA
ctctcttttt

SEQ ID NO: 367 - DNA, 10 bp, Artificial
  synthetic DNA
agtaggggtc

SEQ ID NO: 368 - DNA, 10 bp, Artificial
  synthetic DNA
acaccgcaag

SEQ ID NO: 369 - DNA, 10 bp, Artificial
  synthetic DNA
gaagcgggag

SEQ ID NO: 370 - DNA, 10 bp, Artificial
  synthetic DNA
gatacggact

SEQ ID NO: 371 - DNA, 10 bp, Artificial
  synthetic DNA
tacgacgtgt

SEQ ID NO: 372 - DNA, 10 bp, Artificial
  synthetic DNA
gtgcctcctt

SEQ ID NO: 373 - DNA, 10 bp, Artificial
  synthetic DNA
ggtgactgat

SEQ ID NO: 374 - DNA, 10 bp, Artificial
  synthetic DNA
atatcttacg

SEQ ID NO: 375 - DNA, 10 bp, Artificial
  synthetic DNA
aatcatacgg

SEQ ID NO: 376 - DNA, 10 bp, Artificial
  synthetic DNA
ctcttgggac

SEQ ID NO: 377 - DNA, 10 bp, Artificial
  synthetic DNA
gacgacaaat

SEQ ID NO: 378 - DNA, 10 bp, Artificial
  synthetic DNA
gttgcgaggt

SEQ ID NO: 379 - DNA, 10 bp, Artificial
  synthetic DNA
aaaccgcacc

SEQ ID NO: 380 - DNA, 10 bp, Artificial
  synthetic DNA
gctaacacgt

SEQ ID NO: 381 - DNA, 10 bp, Artificial
  synthetic DNA
atcatgaggg

SEQ ID NO: 382 - DNA, 10 bp, Artificial
  synthetic DNA
gattcacgta

SEQ ID NO: 383 - DNA, 10 bp, Artificial
  synthetic DNA
tctcgaaaag

SEQ ID NO: 384 - DNA, 10 bp, Artificial
  synthetic DNA
ctcgtaacca

SEQ ID NO: 385 - DNA, 10 bp, Artificial
  synthetic DNA
gttacacacg

SEQ ID NO: 386 - DNA, 10 bp, Artificial
  synthetic DNA
cgtgaagggt

SEQ ID NO: 387 - DNA, 10 bp, Artificial
  synthetic DNA
acgagcatct

SEQ ID NO: 388 - DNA, 10 bp, Artificial
  synthetic DNA
acgagggatt

SEQ ID NO: 389 - DNA, 10 bp, Artificial
  synthetic DNA
gcaacgtcgg

SEQ ID NO: 390 - DNA, 10 bp, Artificial
  synthetic DNA
cacggctagg

SEQ ID NO: 391 - DNA, 10 bp, Artificial
  synthetic DNA
cgtgactctc

SEQ ID NO: 392 - DNA, 10 bp, Artificial
  synthetic DNA
tctagacgca

SEQ ID NO: 393 - DNA, 10 bp, Artificial
  synthetic DNA
ctgcgcacat

SEQ ID NO: 394 - DNA, 10 bp, Artificial
  synthetic DNA
atgcttgaca

SEQ ID NO: 395 - DNA, 10 bp, Artificial
  synthetic DNA
tttgtcgaca

SEQ ID NO: 396 - DNA, 10 bp, Artificial
  synthetic DNA
acgtgtcagc

SEQ ID NO: 397 - DNA, 10 bp, Artificial
  synthetic DNA
gaaaacatta

SEQ ID NO: 398 - DNA, 10 bp, Artificial
  synthetic DNA
acattaacgg

SEQ ID NO: 399 - DNA, 10 bp, Artificial
  synthetic DNA
gtacaggtcc

SEQ ID NO: 400 - DNA, 10 bp, Artificial
  synthetic DNA
ctatgtgtac

SEQ ID NO: 401 - DNA, 10 bp, Artificial
  synthetic DNA
gcgtacatta

SEQ ID NO: 402 - DNA, 10 bp, Artificial
  synthetic DNA
gatttgtggc

SEQ ID NO: 403 - DNA, 10 bp, Artificial
  synthetic DNA
tcgcgcgcta

SEQ ID NO: 404 - DNA, 10 bp, Artificial
  synthetic DNA
acaagggcga

SEQ ID NO: 405 - DNA, 10 bp, Artificial
  synthetic DNA
aacgcgcgat

SEQ ID NO: 406 - DNA, 10 bp, Artificial
  synthetic DNA
cgtaaatgcg

SEQ ID NO: 407 - DNA, 10 bp, Artificial
  synthetic DNA
taggcactac

SEQ ID NO: 408 - DNA, 10 bp, Artificial
  synthetic DNA
gcgaggatcg

SEQ ID NO: 409 - DNA, 10 bp, Artificial
  synthetic DNA
cacgtttact

SEQ ID NO: 410 - DNA, 10 bp, Artificial
  synthetic DNA
taccaccacg

SEQ ID NO: 411 - DNA, 10 bp, Artificial
  synthetic DNA
ttaacaggac

SEQ ID NO: 412 - DNA, 10 bp, Artificial
  synthetic DNA
gctgtataac

SEQ ID NO: 413 - DNA, 10 bp, Artificial
  synthetic DNA
gttgctggca

SEQ ID NO: 414 - DNA, 10 bp, Artificial
  synthetic DNA
agtgtggcca

SEQ ID NO: 415 - DNA, 10 bp, Artificial
  synthetic DNA
ctgcggttgt

SEQ ID NO: 416 - DNA, 10 bp, Artificial
  synthetic DNA
tagatcagcg

SEQ ID NO: 417 - DNA, 10 bp, Artificial
  synthetic DNA
ttccggttat

SEQ ID NO: 418 - DNA, 10 bp, Artificial
  synthetic DNA
gataaactgt

SEQ ID NO: 419 - DNA, 10 bp, Artificial
  synthetic DNA
tacagttgcc

SEQ ID NO: 420 - DNA, 10 bp, Artificial
  synthetic DNA
cgatggcgaa

SEQ ID NO: 421 - DNA, 10 bp, Artificial
  synthetic DNA
ccgacgtcag

SEQ ID NO: 422 - DNA, 10 bp, Artificial
  synthetic DNA
tatggtgcaa

SEQ ID NO: 423 - DNA, 10 bp, Artificial
  synthetic DNA
gacgacagtc

SEQ ID NO: 424 - DNA, 10 bp, Artificial
  synthetic DNA
gtcaccgtcc

SEQ ID NO: 425 - DNA, 10 bp, Artificial
  synthetic DNA
ggttttaaca

SEQ ID NO: 426 - DNA, 10 bp, Artificial
  synthetic DNA
gaggacagta

SEQ ID NO: 427 - DNA, 10 bp, Artificial
  synthetic DNA
gttacctaag

SEQ ID NO: 428 - DNA, 10 bp, Artificial
  synthetic DNA
atcacgtgtt

SEQ ID NO: 429 - DNA, 10 bp, Artificial
  synthetic DNA
taaggcctgg

SEQ ID NO: 430 - DNA, 10 bp, Artificial
  synthetic DNA
tgttcgtagc

SEQ ID NO: 431 - DNA, 10 bp, Artificial
  synthetic DNA
tgaggacgtg

SEQ ID NO: 432 - DNA, 10 bp, Artificial
  synthetic DNA
gtgctgtgta

SEQ ID NO: 433 - DNA, 10 bp, Artificial
  synthetic DNA
gagggtacgc

SEQ ID NO: 434 - DNA, 10 bp, Artificial
  synthetic DNA
ccgtgattgt

SEQ ID NO: 435 - DNA, 10 bp, Artificial
  synthetic DNA
aaaatcgcct

SEQ ID NO: 436 - DNA, 10 bp, Artificial
  synthetic DNA
cgatcgcagt

SEQ ID NO: 437 - DNA, 10 bp, Artificial
  synthetic DNA
acgcaataag

SEQ ID NO: 438 - DNA, 10 bp, Artificial
  synthetic DNA
aaggtgcatc

SEQ ID NO: 439 - DNA, 10 bp, Artificial
  synthetic DNA
cgcgtagata

SEQ ID NO: 440 - DNA, 10 bp, Artificial
  synthetic DNA
cgagcagtgc

SEQ ID NO: 441 - DNA, 10 bp, Artificial
  synthetic DNA
atacgtgacg

SEQ ID NO: 442 - DNA, 10 bp, Artificial
  synthetic DNA
agattgcgcg

SEQ ID NO: 443 - DNA, 10 bp, Artificial
  synthetic DNA
acgtgatgcc

SEQ ID NO: 444 - DNA, 10 bp, Artificial
  synthetic DNA
gtacgcatcg

SEQ ID NO: 445 - DNA, 10 bp, Artificial
  synthetic DNA
tcccgactta

SEQ ID NO: 446 - DNA, 10 bp, Artificial
  synthetic DNA
gtttttacac

SEQ ID NO: 447 - DNA, 10 bp, Artificial
  synthetic DNA
cctgagcgtg

SEQ ID NO: 448 - DNA, 10 bp, Artificial
  synthetic DNA
cggcattgta

SEQ ID NO: 449 - DNA, 10 bp, Artificial
  synthetic DNA
tagagtgcgt

SEQ ID NO: 450 - DNA, 10 bp, Artificial
  synthetic DNA
atggccagac

SEQ ID NO: 451 - DNA, 10 bp, Artificial
  synthetic DNA
cttagcatgc

SEQ ID NO: 452 - DNA, 10 bp, Artificial
  synthetic DNA
acaacacctg

SEQ ID NO: 453 - DNA, 10 bp, Artificial
  synthetic DNA
agtgactatc

SEQ ID NO: 454 - DNA, 10 bp, Artificial
  synthetic DNA
catgctacac

SEQ ID NO: 455 - DNA, 10 bp, Artificial
  synthetic DNA
aaagcgggcg

SEQ ID NO: 456 - DNA, 10 bp, Artificial
  synthetic DNA
agatcgccgt

SEQ ID NO: 457 - DNA, 10 bp, Artificial
  synthetic DNA
cgtagatatt

SEQ ID NO: 458 - DNA, 10 bp, Artificial
  synthetic DNA
aatggcagac

SEQ ID NO: 459 - DNA, 10 bp, Artificial
  synthetic DNA
gtataacgtg

SEQ ID NO: 460 - DNA, 10 bp, Artificial
  synthetic DNA
atgtgcgtca

SEQ ID NO: 461 - DNA, 10 bp, Artificial
  synthetic DNA
cctgccaact

SEQ ID NO: 462 - DNA, 10 bp, Artificial
  synthetic DNA
tttataactc

SEQ ID NO: 463 - DNA, 10 bp, Artificial
  synthetic DNA
acggttacgc

SEQ ID NO: 464 - DNA, 10 bp, Artificial
  synthetic DNA
tagcctcttg

SEQ ID NO: 465 - DNA, 10 bp, Artificial
  synthetic DNA
tcgcgaagtt

SEQ ID NO: 466 - DNA, 10 bp, Artificial
  synthetic DNA
gtctacaacc

SEQ ID NO: 467 - DNA, 10 bp, Artificial
  synthetic DNA
gtctactgcg

SEQ ID NO: 468 - DNA, 10 bp, Artificial
  synthetic DNA
gttgcgtctc

SEQ ID NO: 469 - DNA, 10 bp, Artificial
  synthetic DNA
gggccgctaa

SEQ ID NO: 470 - DNA, 10 bp, Artificial
  synthetic DNA
gtacgtcgga

SEQ ID NO: 471 - DNA, 10 bp, Artificial
  synthetic DNA
agcgagagac

SEQ ID NO: 472 - DNA, 10 bp, Artificial
  synthetic DNA
tggctacggt

SEQ ID NO: 473 - DNA, 10 bp, Artificial
  synthetic DNA
aggcatcacg

SEQ ID NO: 474 - DNA, 10 bp, Artificial
  synthetic DNA
tagctcctcg

SEQ ID NO: 475 - DNA, 10 bp, Artificial
  synthetic DNA
ggctagtcag

SEQ ID NO: 476 - DNA, 10 bp, Artificial
  synthetic DNA
ctcactttat

SEQ ID NO: 477 - DNA, 10 bp, Artificial
  synthetic DNA
acggccacgt

SEQ ID NO: 478 - DNA, 10 bp, Artificial
  synthetic DNA
agcgtatatc

SEQ ID NO: 479 - DNA, 10 bp, Artificial
  synthetic DNA
gacacgtcta

SEQ ID NO: 480 - DNA, 10 bp, Artificial
  synthetic DNA
gccagcgtac

SEQ ID NO: 481 - DNA, 10 bp, Artificial
  synthetic DNA
aacattagcg

SEQ ID NO: 482 - DNA, 10 bp, Artificial
  synthetic DNA
agtgtgctat

SEQ ID NO: 483 - DNA, 10 bp, Artificial
  synthetic DNA
cacgagcgtt

SEQ ID NO: 484 - DNA, 10 bp, Artificial
  synthetic DNA
gtaacgccta

SEQ ID NO: 485 - DNA, 10 bp, Artificial
  synthetic DNA
cacatagtac

SEQ ID NO: 486 - DNA, 10 bp, Artificial
  synthetic DNA
cgcgatatcg

SEQ ID NO: 487 - DNA, 10 bp, Artificial
  synthetic DNA
cgttctgtgc

SEQ ID NO: 488 - DNA, 10 bp, Artificial
  synthetic DNA
ctgatcgcat

SEQ ID NO: 489 - DNA, 10 bp, Artificial
  synthetic DNA
tggcgtgaga

SEQ ID NO: 490 - DNA, 10 bp, Artificial
  synthetic DNA
ttgccaggct

SEQ ID NO: 491 - DNA, 10 bp, Artificial
  synthetic DNA
gttatacaca

SEQ ID NO: 492 - DNA, 10 bp, Artificial
  synthetic DNA
agtgccaact

SEQ ID NO: 493 - DNA, 10 bp, Artificial
  synthetic DNA
tcacgtagca

SEQ ID NO: 494 - DNA, 10 bp, Artificial
  synthetic DNA
taattcagcg

SEQ ID NO: 495 - DNA, 10 bp, Artificial
  synthetic DNA
aagtatcgtc

SEQ ID NO: 496 - DNA, 10 bp, Artificial
  synthetic DNA
cacagttact

SEQ ID NO: 497 - DNA, 10 bp, Artificial
  synthetic DNA
ccttaccgtg

SEQ ID NO: 498 - DNA, 10 bp, Artificial
  synthetic DNA
acggtgtcgt

SEQ ID NO: 499 - DNA, 10 bp, Artificial
  synthetic DNA
cgcgtaagac

SEQ ID NO: 500 - DNA, 10 bp, Artificial
  synthetic DNA
ttcgcaccag

SEQ ID NO: 501 - DNA, 10 bp, Artificial
  synthetic DNA
cacgaacaga

SEQ ID NO: 502 - DNA, 10 bp, Artificial
  synthetic DNA
gttggacatt

SEQ ID NO: 503 - DNA, 10 bp, Artificial
  synthetic DNA
ggtgcttaag

SEQ ID NO: 504 - DNA, 10 bp, Artificial
  synthetic DNA
tcggtctcgt

SEQ ID NO: 505 - DNA, 10 bp, Artificial
  synthetic DNA
tctagtacgc

SEQ ID NO: 506 - DNA, 10 bp, Artificial
  synthetic DNA
ttaggccgag

SEQ ID NO: 507 - DNA, 10 bp, Artificial
  synthetic DNA
cgtcaagagc

SEQ ID NO: 508 - DNA, 10 bp, Artificial
  synthetic DNA
acatgtctac

SEQ ID NO: 509 - DNA, 10 bp, Artificial
  synthetic DNA
atcgttacgt

SEQ ID NO: 510 - DNA, 10 bp, Artificial
  synthetic DNA
acggatcgtt

SEQ ID NO: 511 - DNA, 10 bp, Artificial
  synthetic DNA
aatcttggcg

SEQ ID NO: 512 - DNA, 10 bp, Artificial
  synthetic DNA
agtatctggt

SEQ ID NO: 513 - DNA, 10 bp, Artificial
  synthetic DNA
caaccgacgt

SEQ ID NO: 514 - DNA, 10 bp, Artificial
  synthetic DNA
tggtaacgcg

SEQ ID NO: 515 - DNA, 10 bp, Artificial
  synthetic DNA
gtgcagacat

SEQ ID NO: 516 - DNA, 10 bp, Artificial
  synthetic DNA
gtctagttgc

SEQ ID NO: 517 - DNA, 10 bp, Artificial
  synthetic DNA
caattcgacg

SEQ ID NO: 518 - DNA, 10 bp, Artificial
  synthetic DNA
cttagcacct

SEQ ID NO: 519 - DNA, 10 bp, Artificial
  synthetic DNA
taatgtcgca

SEQ ID NO: 520 - DNA, 10 bp, Artificial
  synthetic DNA
caatcggtac

SEQ ID NO: 521 - DNA, 10 bp, Artificial
  synthetic DNA
agcacgcatt

SEQ ID NO: 522 - DNA, 10 bp, Artificial
  synthetic DNA
aggtcctcgt

SEQ ID NO: 523 - DNA, 10 bp, Artificial
  synthetic DNA
ttgtgcctgc

SEQ ID NO: 524 - DNA, 10 bp, Artificial
  synthetic DNA
accgcctgta

SEQ ID NO: 525 - DNA, 10 bp, Artificial
  synthetic DNA
gtacgtcagg

SEQ ID NO: 526 - DNA, 10 bp, Artificial
  synthetic DNA
gcacacaact

SEQ ID NO: 527 - DNA, 10 bp, Artificial
  synthetic DNA
tgagcactta

SEQ ID NO: 528 - DNA, 10 bp, Artificial
  synthetic DNA
gtgccgcata

SEQ ID NO: 529 - DNA, 10 bp, Artificial
  synthetic DNA
atgttttcgc

SEQ ID NO: 530 - DNA, 10 bp, Artificial
  synthetic DNA
acacttaggt

SEQ ID NO: 531 - DNA, 10 bp, Artificial
  synthetic DNA
cgtgccgtga

SEQ ID NO: 532 - DNA, 10 bp, Artificial
  synthetic DNA
ttactaatca

SEQ ID NO: 533 - DNA, 10 bp, Artificial
  synthetic DNA
gtggcaggta

SEQ ID NO: 534 - DNA, 10 bp, Artificial
  synthetic DNA
gcgcgatatg

SEQ ID NO: 535 - DNA, 10 bp, Artificial
  synthetic DNA
gaacgacgtt

SEQ ID NO: 536 - DNA, 10 bp, Artificial
  synthetic DNA
atcaggagtg

SEQ ID NO: 537 - DNA, 10 bp, Artificial
  synthetic DNA
gccagtaagt

SEQ ID NO: 538 - DNA, 10 bp, Artificial
  synthetic DNA
gcaagaagca

SEQ ID NO: 539 - DNA, 10 bp, Artificial
  synthetic DNA
aactccgcca

SEQ ID NO: 540 - DNA, 10 bp, Artificial
  synthetic DNA
acttgagcct

SEQ ID NO: 541 - DNA, 10 bp, Artificial
  synthetic DNA
cgtgatcgtg

SEQ ID NO: 542 - DNA, 10 bp, Artificial
  synthetic DNA
aattagcgaa

SEQ ID NO: 543 - DNA, 10 bp, Artificial
  synthetic DNA
acttccttag

SEQ ID NO: 544 - DNA, 10 bp, Artificial
  synthetic DNA
tgtgctgata

SEQ ID NO: 545 - DNA, 10 bp, Artificial
  synthetic DNA
aggcggctga

SEQ ID NO: 546 - DNA, 10 bp, Artificial
  synthetic DNA
cgtttagagc

SEQ ID NO: 547 - DNA, 10 bp, Artificial
  synthetic DNA
acgcgtctaa

SEQ ID NO: 548 - DNA, 10 bp, Artificial
  synthetic DNA
gcgaatgtac

SEQ ID NO: 549 - DNA, 10 bp, Artificial
  synthetic DNA
cgtgatccaa

SEQ ID NO: 550 - DNA, 10 bp, Artificial
  synthetic DNA
caaccagatg

SEQ ID NO: 551 - DNA, 10 bp, Artificial
  synthetic DNA
accattaacc

SEQ ID NO: 552 - DNA, 10 bp, Artificial
  synthetic DNA
cgattcacgt

SEQ ID NO: 553 - DNA, 10 bp, Artificial
  synthetic DNA
ctagaacctg

SEQ ID NO: 554 - DNA, 10 bp, Artificial
  synthetic DNA
cctaacgaca

SEQ ID NO: 555 - DNA, 10 bp, Artificial
  synthetic DNA
gacgtgcatg

SEQ ID NO: 556 - DNA, 10 bp, Artificial
  synthetic DNA
atgtaacctt

SEQ ID NO: 557 - DNA, 10 bp, Artificial
  synthetic DNA
gatacagtcg

SEQ ID NO: 558 - DNA, 10 bp, Artificial
  synthetic DNA
cgtatgtctc

SEQ ID NO: 559 - DNA, 10 bp, Artificial
  synthetic DNA
agattatcga

SEQ ID NO: 560 - DNA, 10 bp, Artificial
  synthetic DNA
atactggtaa

SEQ ID NO: 561 - DNA, 10 bp, Artificial
  synthetic DNA
gttgagtagc

SEQ ID NO: 562 - DNA, 10 bp, Artificial
  synthetic DNA
accattatca

SEQ ID NO: 563 - DNA, 10 bp, Artificial
  synthetic DNA
cacacttcag

SEQ ID NO: 564 - DNA, 10 bp, Artificial
  synthetic DNA
gactagcggt

SEQ ID NO: 565 - DNA, 10 bp, Artificial
  synthetic DNA
aattgtcgag

SEQ ID NO: 566 - DNA, 10 bp, Artificial
  synthetic DNA
ctaaggacgt

SEQ ID NO: 567 - DNA, 10 bp, Artificial
  synthetic DNA
attacgatga

SEQ ID NO: 568 - DNA, 10 bp, Artificial
  synthetic DNA
attgaagact

SEQ ID NO: 569 - DNA, 10 bp, Artificial
  synthetic DNA
gcttgtacgt

SEQ ID NO: 570 - DNA, 10 bp, Artificial
  synthetic DNA
cctacgtcac

SEQ ID NO: 571 - DNA, 10 bp, Artificial
  synthetic DNA
cacaacttag

SEQ ID NO: 572 - DNA, 10 bp, Artificial
  synthetic DNA
gcggttcatc

SEQ ID NO: 573 - DNA, 10 bp, Artificial
  synthetic DNA
gtactcatct

SEQ ID NO: 574 - DNA, 10 bp, Artificial
  synthetic DNA
gtgcatcagt

SEQ ID NO: 575 - DNA, 10 bp, Artificial
  synthetic DNA
tcacatccta

SEQ ID NO: 576 - DNA, 10 bp, Artificial
  synthetic DNA
cacgcgctat

SEQ ID NO: 577 - DNA, 8 bp, Artificial
  synthetic DNA
ctatcttg

SEQ ID NO: 578 - DNA, 8 bp, Artificial
  synthetic DNA
aagtgcgt

SEQ ID NO: 579 - DNA, 8 bp, Artificial
  synthetic DNA
acatgcga

SEQ ID NO: 580 - DNA, 8 bp, Artificial
  synthetic DNA
accaatgg

SEQ ID NO: 581 - DNA, 8 bp, Artificial
  synthetic DNA
tgcgttga

SEQ ID NO: 582 - DNA, 8 bp, Artificial
  synthetic DNA
gacatgtc

SEQ ID NO: 583 - DNA, 8 bp, Artificial
  synthetic DNA
ttgtgcgt

SEQ ID NO: 584 - DNA, 8 bp, Artificial
  synthetic DNA
acatcgca

SEQ ID NO: 585 - DNA, 8 bp, Artificial
  synthetic DNA
gaagacga

SEQ ID NO: 586 - DNA, 8 bp, Artificial
  synthetic DNA
tcgataga

SEQ ID NO: 587 - DNA, 8 bp, Artificial
  synthetic DNA
tcttgcaa

SEQ ID NO: 588 - DNA, 8 bp, Artificial
  synthetic DNA
agcaagtt

SEQ ID NO: 589 - DNA, 8 bp, Artificial
  synthetic DNA
ttcatgga

SEQ ID NO: 590 - DNA, 8 bp, Artificial
  synthetic DNA
tcaattcg

SEQ ID NO: 591 - DNA, 8 bp, Artificial
  synthetic DNA
cggtatgt

SEQ ID NO: 592 - DNA, 8 bp, Artificial
  synthetic DNA
accactac

SEQ ID NO: 593 - DNA, 8 bp, Artificial
  synthetic DNA
tcgcttat

SEQ ID NO: 594 - DNA, 8 bp, Artificial
  synthetic DNA
tctcgact

SEQ ID NO: 595 - DNA, 8 bp, Artificial
  synthetic DNA
gaatcggt

SEQ ID NO: 596 - DNA, 8 bp, Artificial
  synthetic DNA
gttacaag

SEQ ID NO: 597 - DNA, 8 bp, Artificial
  synthetic DNA
ctgtgtag

SEQ ID NO: 598 - DNA, 8 bp, Artificial
  synthetic DNA
tggtagaa

SEQ ID NO: 599 - DNA, 8 bp, Artificial
  synthetic DNA
atactgcg

SEQ ID NO: 600 - DNA, 8 bp, Artificial
  synthetic DNA
aactcgtc

SEQ ID NO: 601 - DNA, 8 bp, Artificial
  synthetic DNA
atatgtgc

SEQ ID NO: 602 - DNA, 8 bp, Artificial
  synthetic DNA
aagttgcg

SEQ ID NO: 603 - DNA, 8 bp, Artificial
  synthetic DNA
gatcatgt

SEQ ID NO: 604 - DNA, 8 bp, Artificial
  synthetic DNA
ttgttgct

SEQ ID NO: 605 - DNA, 8 bp, Artificial
  synthetic DNA
cctcttag

SEQ ID NO: 606 - DNA, 8 bp, Artificial
  synthetic DNA
tcacagct

SEQ ID NO: 607 - DNA, 8 bp, Artificial
  synthetic DNA
agattgac

SEQ ID NO: 608 - DNA, 8 bp, Artificial
  synthetic DNA
agcctgat

SEQ ID NO: 609 - DNA, 8 bp, Artificial
  synthetic DNA
cgtcaagt

SEQ ID NO: 610 - DNA, 8 bp, Artificial
  synthetic DNA
aagtagac

SEQ ID NO: 611 - DNA, 8 bp, Artificial
  synthetic DNA
tcagacaa

SEQ ID NO: 612 - DNA, 8 bp, Artificial
  synthetic DNA
tccttgac

SEQ ID NO: 613 - DNA, 8 bp, Artificial
  synthetic DNA
gtagctgt

SEQ ID NO: 614 - DNA, 8 bp, Artificial
  synthetic DNA
cgtcgtaa

SEQ ID NO: 615 - DNA, 8 bp, Artificial
  synthetic DNA
ccaatgga

SEQ ID NO: 616 - DNA, 8 bp, Artificial
  synthetic DNA
ttgagaga

SEQ ID NO: 617 - DNA, 8 bp, Artificial
  synthetic DNA
acaacacc

SEQ ID NO: 618 - DNA, 8 bp, Artificial
  synthetic DNA
tctagtac

SEQ ID NO: 619 - DNA, 8 bp, Artificial
  synthetic DNA
gaggaagt

SEQ ID NO: 620 - DNA, 8 bp, Artificial
  synthetic DNA
gcgtattg

SEQ ID NO: 621 - DNA, 8 bp, Artificial
  synthetic DNA
aagtagct

SEQ ID NO: 622 - DNA, 8 bp, Artificial
  synthetic DNA
tgaacctt

SEQ ID NO: 623 - DNA, 8 bp, Artificial
  synthetic DNA
tgtgttac

SEQ ID NO: 624 - DNA, 8 bp, Artificial
  synthetic DNA
taacctga

SEQ ID NO: 625 - DNA, 8 bp, Artificial
  synthetic DNA
gctattcc

SEQ ID NO: 626 - DNA, 8 bp, Artificial
  synthetic DNA
gttagatg

SEQ ID NO: 627 - DNA, 8 bp, Artificial
  synthetic DNA
caggataa

SEQ ID NO: 628 - DNA, 8 bp, Artificial
  synthetic DNA
accgtagt

SEQ ID NO: 629 - DNA, 8 bp, Artificial
  synthetic DNA
ccgtgtat

SEQ ID NO: 630 - DNA, 8 bp, Artificial
  synthetic DNA
tccactct

SEQ ID NO: 631 - DNA, 8 bp, Artificial
  synthetic DNA
tagctcat

SEQ ID NO: 632 - DNA, 8 bp, Artificial
  synthetic DNA
cgctaata

SEQ ID NO: 633 - DNA, 8 bp, Artificial
  synthetic DNA
tacctctg

SEQ ID NO: 634 - DNA, 8 bp, Artificial
  synthetic DNA
tgcactac

SEQ ID NO: 635 - DNA, 8 bp, Artificial
  synthetic DNA
cttggaag

SEQ ID NO: 636 - DNA, 8 bp, Artificial
  synthetic DNA
aatgcacg

SEQ ID NO: 637 - DNA, 8 bp, Artificial
  synthetic DNA
cactgtta

SEQ ID NO: 638 - DNA, 8 bp, Artificial
  synthetic DNA
tcgactag

SEQ ID NO: 639 - DNA, 8 bp, Artificial
  synthetic DNA
ctaggtta

SEQ ID NO: 640 - DNA, 8 bp, Artificial
  synthetic DNA
gcagatgt

SEQ ID NO: 641 - DNA, 8 bp, Artificial
  synthetic DNA
agttcaga

SEQ ID NO: 642 - DNA, 8 bp, Artificial
  synthetic DNA
ctccatca

SEQ ID NO: 643 - DNA, 8 bp, Artificial
  synthetic DNA
tggttacg

SEQ ID NO: 644 - DNA, 8 bp, Artificial
  synthetic DNA
acgtagca

SEQ ID NO: 645 - DNA, 8 bp, Artificial
  synthetic DNA
ctcttcca

SEQ ID NO: 646 - DNA, 8 bp, Artificial
  synthetic DNA
cgtcagat

SEQ ID NO: 647 - DNA, 8 bp, Artificial
  synthetic DNA
tggatcat

SEQ ID NO: 648 - DNA, 8 bp, Artificial
  synthetic DNA
atatcgac

SEQ ID NO: 649 - DNA, 8 bp, Artificial
  synthetic DNA
ttgtggag

SEQ ID NO: 650 - DNA, 8 bp, Artificial
  synthetic DNA
ttagagca

SEQ ID NO: 651 - DNA, 8 bp, Artificial
  synthetic DNA
taactacc

SEQ ID NO: 652 - DNA, 8 bp, Artificial
  synthetic DNA
ctatgagg

SEQ ID NO: 653 - DNA, 8 bp, Artificial
  synthetic DNA
cttctcac

SEQ ID NO: 654 - DNA, 8 bp, Artificial
  synthetic DNA
cgttctct

SEQ ID NO: 655 - DNA, 8 bp, Artificial
  synthetic DNA
gtcactat

SEQ ID NO: 656 - DNA, 8 bp, Artificial
  synthetic DNA
tcgttagc

SEQ ID NO: 657 - DNA, 8 bp, Artificial
  synthetic DNA
atcgtgta

SEQ ID NO: 658 - DNA, 8 bp, Artificial
  synthetic DNA
gagagcaa

SEQ ID NO: 659 - DNA, 8 bp, Artificial
  synthetic DNA
agacgcaa

SEQ ID NO: 660 - DNA, 8 bp, Artificial
  synthetic DNA
tccagtta

SEQ ID NO: 661 - DNA, 8 bp, Artificial
  synthetic DNA
aatgccac

SEQ ID NO: 662 - DNA, 8 bp, Artificial
  synthetic DNA
atcacgtg

SEQ ID NO: 663 - DNA, 8 bp, Artificial
  synthetic DNA
actgtgca

SEQ ID NO: 664 - DNA, 8 bp, Artificial
  synthetic DNA
tcactgca

SEQ ID NO: 665 - DNA, 8 bp, Artificial
  synthetic DNA
gcatccaa

SEQ ID NO: 666 - DNA, 8 bp, Artificial
  synthetic DNA
agcactat

SEQ ID NO: 667 - DNA, 8 bp, Artificial
  synthetic DNA
cgaaggat

SEQ ID NO: 668 - DNA, 8 bp, Artificial
  synthetic DNA
ccttgtgt

SEQ ID NO: 669 - DNA, 8 bp, Artificial
  synthetic DNA
tgcggata

SEQ ID NO: 670 - DNA, 8 bp, Artificial
  synthetic DNA
aggaatgg

SEQ ID NO: 671 - DNA, 8 bp, Artificial
  synthetic DNA
atcgtaac

SEQ ID NO: 672 - DNA, 8 bp, Artificial
  synthetic DNA
gaatgtct

SEQ ID NO: 673 - DNA, 9 bp, Artificial
  synthetic DNA
ttgctacat

SEQ ID NO: 674 - DNA, 9 bp, Artificial
  synthetic DNA
taacgtatg

SEQ ID NO: 675 - DNA, 9 bp, Artificial
  synthetic DNA
cagtatgta

SEQ ID NO: 676 - DNA, 9 bp, Artificial
  synthetic DNA
tcaataacg

SEQ ID NO: 677 - DNA, 9 bp, Artificial
  synthetic DNA
cacacttat

SEQ ID NO: 678 - DNA, 9 bp, Artificial
  synthetic DNA
gactgtaat

SEQ ID NO: 679 - DNA, 9 bp, Artificial
  synthetic DNA
tatacactg

SEQ ID NO: 680 - DNA, 9 bp, Artificial
  synthetic DNA
actgcatta

SEQ ID NO: 681 - DNA, 9 bp, Artificial
  synthetic DNA
acattaagc

SEQ ID NO: 682 - DNA, 9 bp, Artificial
  synthetic DNA
catattacg

SEQ ID NO: 683 - DNA, 9 bp, Artificial
  synthetic DNA
atatctacg

SEQ ID NO: 684 - DNA, 9 bp, Artificial
  synthetic DNA
agtaactgt

SEQ ID NO: 685 - DNA, 9 bp, Artificial
  synthetic DNA
atgacgtta

SEQ ID NO: 686 - DNA, 9 bp, Artificial
  synthetic DNA
attatgcga

SEQ ID NO: 687 - DNA, 9 bp, Artificial
  synthetic DNA
agtatacac

SEQ ID NO: 688 - DNA, 9 bp, Artificial
  synthetic DNA
ttagcgtta

SEQ ID NO: 689 - DNA, 9 bp, Artificial
  synthetic DNA
tatgacact

SEQ ID NO: 690 - DNA, 9 bp, Artificial
  synthetic DNA
attaacgct

SEQ ID NO: 691 - DNA, 9 bp, Artificial
  synthetic DNA
taggacaat

SEQ ID NO: 692 - DNA, 9 bp, Artificial
  synthetic DNA
aagacgtta

SEQ ID NO: 693 - DNA, 9 bp, Artificial
  synthetic DNA
tataagcgt

SEQ ID NO: 694 - DNA, 9 bp, Artificial
  synthetic DNA
atacctggc

SEQ ID NO: 695 - DNA, 9 bp, Artificial
  synthetic DNA
ctcgagatc

SEQ ID NO: 696 - DNA, 9 bp, Artificial
  synthetic DNA
atggtgagg

SEQ ID NO: 697 - DNA, 9 bp, Artificial
  synthetic DNA
atgtcgacg

SEQ ID NO: 698 - DNA, 9 bp, Artificial
  synthetic DNA
gacgtctga

SEQ ID NO: 699 - DNA, 9 bp, Artificial
  synthetic DNA
tacactgcg

SEQ ID NO: 700 - DNA, 9 bp, Artificial
  synthetic DNA
atcgtcagg

SEQ ID NO: 701 - DNA, 9 bp, Artificial
  synthetic DNA
tgcacgtac

SEQ ID NO: 702 - DNA, 9 bp, Artificial
  synthetic DNA
gtcgtgcat

SEQ ID NO: 703 - DNA, 9 bp, Artificial
  synthetic DNA
gagtgttac

SEQ ID NO: 704 - DNA, 9 bp, Artificial
  synthetic DNA
agactgtac

SEQ ID NO: 705 - DNA, 9 bp, Artificial
  synthetic DNA
tgcgactta

SEQ ID NO: 706 - DNA, 9 bp, Artificial
  synthetic DNA
tgtccgtaa

SEQ ID NO: 707 - DNA, 9 bp, Artificial
  synthetic DNA
gtaatcgag

SEQ ID NO: 708 - DNA, 9 bp, Artificial
  synthetic DNA
gtaccttag

SEQ ID NO: 709 - DNA, 9 bp, Artificial
  synthetic DNA
atcacgtgt

SEQ ID NO: 710 - DNA, 9 bp, Artificial
  synthetic DNA
acttagcgt

SEQ ID NO: 711 - DNA, 9 bp, Artificial
  synthetic DNA
gtaatcgtg

SEQ ID NO: 712 - DNA, 9 bp, Artificial
  synthetic DNA
atgccgtta

SEQ ID NO: 713 - DNA, 9 bp, Artificial
  synthetic DNA
ataacgtgc

SEQ ID NO: 714 - DNA, 9 bp, Artificial
  synthetic DNA
ctacgttgt

SEQ ID NO: 715 - DNA, 9 bp, Artificial
  synthetic DNA
tatgacgca

SEQ ID NO: 716 - DNA, 9 bp, Artificial
  synthetic DNA
ccgataaca

SEQ ID NO: 717 - DNA, 9 bp, Artificial
  synthetic DNA
atgcgcata

SEQ ID NO: 718 - DNA, 9 bp, Artificial
  synthetic DNA
gataagcgt

SEQ ID NO: 719 - DNA, 9 bp, Artificial
  synthetic DNA
atatctgcg

SEQ ID NO: 720 - DNA, 9 bp, Artificial
  synthetic DNA
acttagacg

SEQ ID NO: 721 - DNA, 9 bp, Artificial
  synthetic DNA
atcaccgta

SEQ ID NO: 722 - DNA, 9 bp, Artificial
  synthetic DNA
taagacacg

SEQ ID NO: 723 - DNA, 9 bp, Artificial
  synthetic DNA
aatgccgta

SEQ ID NO: 724 - DNA, 9 bp, Artificial
  synthetic DNA
aatcacgtg

SEQ ID NO: 725 - DNA, 9 bp, Artificial
  synthetic DNA
tcgttagtc

SEQ ID NO: 726 - DNA, 9 bp, Artificial
  synthetic DNA
catcatgtc

SEQ ID NO: 727 - DNA, 9 bp, Artificial
  synthetic DNA
taagacggt

SEQ ID NO: 728 - DNA, 9 bp, Artificial
  synthetic DNA
tgcatagtg

SEQ ID NO: 729 - DNA, 9 bp, Artificial
  synthetic DNA
gagcgttat

SEQ ID NO: 730 - DNA, 9 bp, Artificial
  synthetic DNA
tgccttaca

SEQ ID NO: 731 - DNA, 9 bp, Artificial
  synthetic DNA
ttcgcgtta

SEQ ID NO: 732 - DNA, 9 bp, Artificial
  synthetic DNA
gtgttaacg

SEQ ID NO: 733 - DNA, 9 bp, Artificial
  synthetic DNA
gacactgaa

SEQ ID NO: 734 - DNA, 9 bp, Artificial
  synthetic DNA
ctgttatcg

SEQ ID NO: 735 - DNA, 9 bp, Artificial
  synthetic DNA
ggtcgttat

SEQ ID NO: 736 - DNA, 9 bp, Artificial
  synthetic DNA
cgagagtat

SEQ ID NO: 737 - DNA, 9 bp, Artificial
  synthetic DNA
atacagtcc

SEQ ID NO: 738 - DNA, 9 bp, Artificial
  synthetic DNA
aattcacgc

SEQ ID NO: 739 - DNA, 9 bp, Artificial
  synthetic DNA
tatgtgcac

SEQ ID NO: 740 - DNA, 9 bp, Artificial
  synthetic DNA
gatgacgta

SEQ ID NO: 741 - DNA, 9 bp, Artificial
  synthetic DNA
gatgcgata

SEQ ID NO: 742 - DNA, 9 bp, Artificial
  synthetic DNA
gagcgatta

SEQ ID NO: 743 - DNA, 9 bp, Artificial
  synthetic DNA
tgtcacaga

SEQ ID NO: 744 - DNA, 9 bp, Artificial
  synthetic DNA
tactaaccg

SEQ ID NO: 745 - DNA, 9 bp, Artificial
  synthetic DNA
cataacgag

SEQ ID NO: 746 - DNA, 9 bp, Artificial
  synthetic DNA
cgtatacct

SEQ ID NO: 747 - DNA, 9 bp, Artificial
  synthetic DNA
tatcacgtg

SEQ ID NO: 748 - DNA, 9 bp, Artificial
  synthetic DNA
gaacgttac

SEQ ID NO: 749 - DNA, 9 bp, Artificial
  synthetic DNA
gtcgtatac

SEQ ID NO: 750 - DNA, 9 bp, Artificial
  synthetic DNA
atgtcgaca

SEQ ID NO: 751 - DNA, 9 bp, Artificial
  synthetic DNA
atacagcac

SEQ ID NO: 752 - DNA, 9 bp, Artificial
  synthetic DNA
tacttacgc

SEQ ID NO: 753 - DNA, 9 bp, Artificial
  synthetic DNA
aactacggt

SEQ ID NO: 754 - DNA, 9 bp, Artificial
  synthetic DNA
tagaacggt

SEQ ID NO: 755 - DNA, 9 bp, Artificial
  synthetic DNA
gaatgtcac

SEQ ID NO: 756 - DNA, 9 bp, Artificial
  synthetic DNA
tgtacgtct

SEQ ID NO: 757 - DNA, 9 bp, Artificial
  synthetic DNA
aacattgcg

SEQ ID NO: 758 - DNA, 9 bp, Artificial
  synthetic DNA
ttgaacgct

SEQ ID NO: 759 - DNA, 9 bp, Artificial
  synthetic DNA
aatcaggac

SEQ ID NO: 760 - DNA, 9 bp, Artificial
  synthetic DNA
attcgcaca

SEQ ID NO: 761 - DNA, 9 bp, Artificial
  synthetic DNA
ccatgtact

SEQ ID NO: 762 - DNA, 9 bp, Artificial
  synthetic DNA
tgtcctgtt

SEQ ID NO: 763 - DNA, 9 bp, Artificial
  synthetic DNA
taattgcgc

SEQ ID NO: 764 - DNA, 9 bp, Artificial
  synthetic DNA
gatagtgtg

SEQ ID NO: 765 - DNA, 9 bp, Artificial
  synthetic DNA
atagacgca

SEQ ID NO: 766 - DNA, 9 bp, Artificial
  synthetic DNA
tgtaccgtt

SEQ ID NO: 767 - DNA, 9 bp, Artificial
  synthetic DNA
attgtcgca

SEQ ID NO: 768 - DNA, 9 bp, Artificial
  synthetic DNA
gtcacgtaa

SEQ ID NO: 769 - DNA, 11 bp, Artificial
  synthetic DNA
ttacactatgc

SEQ ID NO: 770 - DNA, 11 bp, Artificial
  synthetic DNA
gcgatagtcgt

SEQ ID NO: 771 - DNA, 11 bp, Artificial
  synthetic DNA
ctattcacagt

SEQ ID NO: 772 - DNA, 11 bp, Artificial
  synthetic DNA
agagtcactgt

SEQ ID NO: 773 - DNA, 11 bp, Artificial
  synthetic DNA
agagtcgaagc

SEQ ID NO: 774 - DNA, 11 bp, Artificial
  synthetic DNA
ctgaatatgtg

SEQ ID NO: 775 - DNA, 11 bp, Artificial
  synthetic DNA
actccacagga

SEQ ID NO: 776 - DNA, 11 bp, Artificial
  synthetic DNA
atcctcgtaag

SEQ ID NO: 777 - DNA, 11 bp, Artificial
  synthetic DNA
taccatcgcct

SEQ ID NO: 778 - DNA, 11 bp, Artificial
  synthetic DNA
aacgcctataa

SEQ ID NO: 779 - DNA, 11 bp, Artificial
  synthetic DNA
ctgtcgaactt

SEQ ID NO: 780 - DNA, 11 bp, Artificial
  synthetic DNA
tcagatgtccg

SEQ ID NO: 781 - DNA, 11 bp, Artificial
  synthetic DNA
ctgcttatcgt

SEQ ID NO: 782 - DNA, 11 bp, Artificial
  synthetic DNA
acattcgcaca

SEQ ID NO: 783 - DNA, 11 bp, Artificial
  synthetic DNA
ccttaatgcat

SEQ ID NO: 784 - DNA, 11 bp, Artificial
  synthetic DNA
ggctagctact

SEQ ID NO: 785 - DNA, 11 bp, Artificial
  synthetic DNA
ttccagttggc

SEQ ID NO: 786 - DNA, 11 bp, Artificial
  synthetic DNA
gagtcacaagg

SEQ ID NO: 787 - DNA, 11 bp, Artificial
  synthetic DNA
cagaaggttca

SEQ ID NO: 788 - DNA, 11 bp, Artificial
  synthetic DNA
tcaacgtgcag

SEQ ID NO: 789 - DNA, 11 bp, Artificial
  synthetic DNA
caagcttacta

SEQ ID NO: 790 - DNA, 11 bp, Artificial
  synthetic DNA
agaactcgttg

SEQ ID NO: 791 - DNA, 11 bp, Artificial
  synthetic DNA
ccgatacagag

SEQ ID NO: 792 - DNA, 11 bp, Artificial
  synthetic DNA
gtacgctgatc

SEQ ID NO: 793 - DNA, 11 bp, Artificial
  synthetic DNA
tcctcagtgaa

SEQ ID NO: 794 - DNA, 11 bp, Artificial
  synthetic DNA
gagccaacatt

SEQ ID NO: 795 - DNA, 11 bp, Artificial
  synthetic DNA
gagatcgatgg

SEQ ID NO: 796 - DNA, 11 bp, Artificial
  synthetic DNA
atcgtcagctg

SEQ ID NO: 797 - DNA, 11 bp, Artificial
  synthetic DNA
gaagcacacgt

SEQ ID NO: 798 - DNA, 11 bp, Artificial
  synthetic DNA
atcacgcaacc

SEQ ID NO: 799 - DNA, 11 bp, Artificial
  synthetic DNA
tcgaatagtcg

SEQ ID NO: 800 - DNA, 11 bp, Artificial
  synthetic DNA
tattaccgtct

SEQ ID NO: 801 - DNA, 11 bp, Artificial
  synthetic DNA
cagtcacgaca

SEQ ID NO: 802 - DNA, 11 bp, Artificial
  synthetic DNA
ttactcgacgt

SEQ ID NO: 803 - DNA, 11 bp, Artificial
  synthetic DNA
gcaatgttgaa

SEQ ID NO: 804 - DNA, 11 bp, Artificial
  synthetic DNA
gacacgagcaa

SEQ ID NO: 805 - DNA, 11 bp, Artificial
  synthetic DNA
cgagattacaa

SEQ ID NO: 806 - DNA, 11 bp, Artificial
  synthetic DNA
taccgactaca

SEQ ID NO: 807 - DNA, 11 bp, Artificial
  synthetic DNA
accgttgccat

SEQ ID NO: 808 - DNA, 11 bp, Artificial
  synthetic DNA
atgtaatcgcc

SEQ ID NO: 809 - DNA, 11 bp, Artificial
  synthetic DNA
aagcctgatgt

SEQ ID NO: 810 - DNA, 11 bp, Artificial
  synthetic DNA
aagtaacgtgg

SEQ ID NO: 811 - DNA, 11 bp, Artificial
  synthetic DNA
gtagaggttgg

SEQ ID NO: 812 - DNA, 11 bp, Artificial
  synthetic DNA
ctcttgcctca

SEQ ID NO: 813 - DNA, 11 bp, Artificial
  synthetic DNA
atcgtgaagtg

SEQ ID NO: 814 - DNA, 11 bp, Artificial
  synthetic DNA
accagcactat

SEQ ID NO: 815 - DNA, 11 bp, Artificial
  synthetic DNA
caccagaatgt

SEQ ID NO: 816 - DNA, 11 bp, Artificial
  synthetic DNA
gagtgaacaac

SEQ ID NO: 817 - DNA, 11 bp, Artificial
  synthetic DNA
taacgttacgc

SEQ ID NO: 818 - DNA, 11 bp, Artificial
  synthetic DNA
cttggatcttg

SEQ ID NO: 819 - DNA, 11 bp, Artificial
  synthetic DNA
gttccaacgtt

SEQ ID NO: 820 - DNA, 11 bp, Artificial
  synthetic DNA
caaggaccgta

SEQ ID NO: 821 - DNA, 11 bp, Artificial
  synthetic DNA
gacttcacgca

SEQ ID NO: 822 - DNA, 11 bp, Artificial
  synthetic DNA
cacactactgg

SEQ ID NO: 823 - DNA, 11 bp, Artificial
  synthetic DNA
tcagatgaatc

SEQ ID NO: 824 - DNA, 11 bp, Artificial
  synthetic DNA
tatggatctgg

SEQ ID NO: 825 - DNA, 11 bp, Artificial
  synthetic DNA
tcttaggtgtg

SEQ ID NO: 826 - DNA, 11 bp, Artificial
  synthetic DNA
tgtcagcgtca

SEQ ID NO: 827 - DNA, 11 bp, Artificial
  synthetic DNA
gtctaggacag

SEQ ID NO: 828 - DNA, 11 bp, Artificial
  synthetic DNA
gcctcttcata

SEQ ID NO: 829 - DNA, 11 bp, Artificial
  synthetic DNA
agaagtgttac

SEQ ID NO: 830 - DNA, 11 bp, Artificial
  synthetic DNA
catgaggcttg

SEQ ID NO: 831 - DNA, 11 bp, Artificial
  synthetic DNA
tggattgctca

SEQ ID NO: 832 - DNA, 11 bp, Artificial
  synthetic DNA
atctacctaag

SEQ ID NO: 833 - DNA, 11 bp, Artificial
  synthetic DNA
atgagcagtga

SEQ ID NO: 834 - DNA, 11 bp, Artificial
  synthetic DNA
ccaggagatac

SEQ ID NO: 835 - DNA, 11 bp, Artificial
  synthetic DNA
ccgttatactt

SEQ ID NO: 836 - DNA, 11 bp, Artificial
  synthetic DNA
ctcagtacaag

SEQ ID NO: 837 - DNA, 11 bp, Artificial
  synthetic DNA
ggtgatcgtag

SEQ ID NO: 838 - DNA, 11 bp, Artificial
  synthetic DNA
cgaacgagaca

SEQ ID NO: 839 - DNA, 11 bp, Artificial
  synthetic DNA
actacgagctt

SEQ ID NO: 840 - DNA, 11 bp, Artificial
  synthetic DNA
ttgccacagca

SEQ ID NO: 841 - DNA, 11 bp, Artificial
  synthetic DNA
gtcaactctac

SEQ ID NO: 842 - DNA, 11 bp, Artificial
  synthetic DNA
tggactgtgtc

SEQ ID NO: 843 - DNA, 11 bp, Artificial
  synthetic DNA
ggaatggactt

SEQ ID NO: 844 - DNA, 11 bp, Artificial
  synthetic DNA
cgagaacataa

SEQ ID NO: 845 - DNA, 11 bp, Artificial
  synthetic DNA
acctggtcagt

SEQ ID NO: 846 - DNA, 11 bp, Artificial
  synthetic DNA
cgaacgacaca

SEQ ID NO: 847 - DNA, 11 bp, Artificial
  synthetic DNA
agtctagccat

SEQ ID NO: 848 - DNA, 11 bp, Artificial
  synthetic DNA
aggcctagatg

SEQ ID NO: 849 - DNA, 11 bp, Artificial
  synthetic DNA
ggtgcgttagt

SEQ ID NO: 850 - DNA, 11 bp, Artificial
  synthetic DNA
attgtgtccga

SEQ ID NO: 851 - DNA, 11 bp, Artificial
  synthetic DNA
gcagacattaa

SEQ ID NO: 852 - DNA, 11 bp, Artificial
  synthetic DNA
attggctcatg

SEQ ID NO: 853 - DNA, 11 bp, Artificial
  synthetic DNA
gaggttacatg

SEQ ID NO: 854 - DNA, 11 bp, Artificial
  synthetic DNA
cctataggacc

SEQ ID NO: 855 - DNA, 11 bp, Artificial
  synthetic DNA
ttagacggtct

SEQ ID NO: 856 - DNA, 11 bp, Artificial
  synthetic DNA
gattgacgcac

SEQ ID NO: 857 - DNA, 11 bp, Artificial
  synthetic DNA
aagacacctcg

SEQ ID NO: 858 - DNA, 11 bp, Artificial
  synthetic DNA
tcgaataatcg

SEQ ID NO: 859 - DNA, 11 bp, Artificial
  synthetic DNA
tctatgtcgga

SEQ ID NO: 860 - DNA, 11 bp, Artificial
  synthetic DNA
tcgcatgaacc

SEQ ID NO: 861 - DNA, 11 bp, Artificial
  synthetic DNA
tgttatgtctc

SEQ ID NO: 862 - DNA, 11 bp, Artificial
  synthetic DNA
tggatcctaca

SEQ ID NO: 863 - DNA, 11 bp, Artificial
  synthetic DNA
atcgttcagcc

SEQ ID NO: 864 - DNA, 11 bp, Artificial
  synthetic DNA
taccgcaagca

SEQ ID NO: 865 - DNA, 12 bp, Artificial
  synthetic DNA
gctgttgaaccg

SEQ ID NO: 866 - DNA, 12 bp, Artificial
  synthetic DNA
atactccgagat

SEQ ID NO: 867 - DNA, 12 bp, Artificial
  synthetic DNA
cttaaggagcgc

SEQ ID NO: 868 - DNA, 12 bp, Artificial
  synthetic DNA
tatactacaagc

SEQ ID NO: 869 - DNA, 12 bp, Artificial
  synthetic DNA
tagtggtcgtca

SEQ ID NO: 870 - DNA, 12 bp, Artificial
  synthetic DNA
gtgcttcaggag

SEQ ID NO: 871 - DNA, 12 bp, Artificial
  synthetic DNA
gacgcatacctc

SEQ ID NO: 872 - DNA, 12 bp, Artificial
  synthetic DNA
cctacctgtgga

SEQ ID NO: 873 - DNA, 12 bp, Artificial
  synthetic DNA
gcggtcacatat

SEQ ID NO: 874 - DNA, 12 bp, Artificial
  synthetic DNA
ctgcattcacga

SEQ ID NO: 875 - DNA, 12 bp, Artificial
  synthetic DNA
tggatccttcat

SEQ ID NO: 876 - DNA, 12 bp, Artificial
  synthetic DNA
ttgtgctggact

SEQ ID NO: 877 - DNA, 12 bp, Artificial
  synthetic DNA
attgagagctat

SEQ ID NO: 878 - DNA, 12 bp, Artificial
  synthetic DNA
tcgctaatgtag

SEQ ID NO: 879 - DNA, 12 bp, Artificial
  synthetic DNA
ctactggcacaa

SEQ ID NO: 880 - DNA, 12 bp, Artificial
  synthetic DNA
agagccagtcgt

SEQ ID NO: 881 - DNA, 12 bp, Artificial
  synthetic DNA
aatactggctaa

SEQ ID NO: 882 - DNA, 12 bp, Artificial
  synthetic DNA
ctgcatgcataa

SEQ ID NO: 883 - DNA, 12 bp, Artificial
  synthetic DNA
ttgtcacaactc

SEQ ID NO: 884 - DNA, 12 bp, Artificial
  synthetic DNA
tgctaactctcc

SEQ ID NO: 885 - DNA, 12 bp, Artificial
  synthetic DNA
tctctagttcgg

SEQ ID NO: 886 - DNA, 12 bp, Artificial
  synthetic DNA
ttacgtccgcaa

SEQ ID NO: 887 - DNA, 12 bp, Artificial
  synthetic DNA
gtgttgctacca

SEQ ID NO: 888 - DNA, 12 bp, Artificial
  synthetic DNA
cgcatgtatgcc

SEQ ID NO: 889 - DNA, 12 bp, Artificial
  synthetic DNA
cctgttctgatt

SEQ ID NO: 890 - DNA, 12 bp, Artificial
  synthetic DNA
taagatgcttga

SEQ ID NO: 891 - DNA, 12 bp, Artificial
  synthetic DNA
atatatctcagc

SEQ ID NO: 892 - DNA, 12 bp, Artificial
  synthetic DNA
ttcctcgtggtt

SEQ ID NO: 893 - DNA, 12 bp, Artificial
  synthetic DNA
atgtcgatctag

SEQ ID NO: 894 - DNA, 12 bp, Artificial
  synthetic DNA
catccactaatc

SEQ ID NO: 895 - DNA, 12 bp, Artificial
  synthetic DNA
gcctctggtaac

SEQ ID NO: 896 - DNA, 12 bp, Artificial
  synthetic DNA
agtcaagagatt

SEQ ID NO: 897 - DNA, 12 bp, Artificial
  synthetic DNA
actgaggcgttc

SEQ ID NO: 898 - DNA, 12 bp, Artificial
  synthetic DNA
taaggctgacat

SEQ ID NO: 899 - DNA, 12 bp, Artificial
  synthetic DNA
agttcgcataca

SEQ ID NO: 900 - DNA, 12 bp, Artificial
  synthetic DNA
gcagaattgcga

SEQ ID NO: 901 - DNA, 12 bp, Artificial
  synthetic DNA
ggttatgaagaa

SEQ ID NO: 902 - DNA, 12 bp, Artificial
  synthetic DNA
agaagtcgcctc

SEQ ID NO: 903 - DNA, 12 bp, Artificial
  synthetic DNA
ttcgcgttattg

SEQ ID NO: 904 - DNA, 12 bp, Artificial
  synthetic DNA
tacctggtcggt

SEQ ID NO: 905 - DNA, 12 bp, Artificial
  synthetic DNA
ggttaccgagga

SEQ ID NO: 906 - DNA, 12 bp, Artificial
  synthetic DNA
acacacttctag

SEQ ID NO: 907 - DNA, 12 bp, Artificial
  synthetic DNA
ggaagtgattaa

SEQ ID NO: 908 - DNA, 12 bp, Artificial
  synthetic DNA
tccatcagataa

SEQ ID NO: 909 - DNA, 12 bp, Artificial
  synthetic DNA
tgtctgtatcat

SEQ ID NO: 910 - DNA, 12 bp, Artificial
  synthetic DNA
aattggctatag

SEQ ID NO: 911 - DNA, 12 bp, Artificial
  synthetic DNA
acgtcggaaggt

SEQ ID NO: 912 - DNA, 12 bp, Artificial
  synthetic DNA
aggcatccgttg

SEQ ID NO: 913 - DNA, 12 bp, Artificial
  synthetic DNA
accgtcgcttga

SEQ ID NO: 914 - DNA, 12 bp, Artificial
  synthetic DNA
taccgtcaagtg

SEQ ID NO: 915 - DNA, 12 bp, Artificial
  synthetic DNA
ctcgatatagtt

SEQ ID NO: 916 - DNA, 12 bp, Artificial
  synthetic DNA
cgtcaacgtggt

SEQ ID NO: 917 - DNA, 12 bp, Artificial
  synthetic DNA
tagtcaacgtag

SEQ ID NO: 918 - DNA, 12 bp, Artificial
  synthetic DNA
tgagtaggtcag

SEQ ID NO: 919 - DNA, 12 bp, Artificial
  synthetic DNA
cttggcatgtac

SEQ ID NO: 920 - DNA, 12 bp, Artificial
  synthetic DNA
tgccgagacttc

SEQ ID NO: 921 - DNA, 12 bp, Artificial
  synthetic DNA
ctaagacttaag

SEQ ID NO: 922 - DNA, 12 bp, Artificial
  synthetic DNA
ttctcgtgtgcg

SEQ ID NO: 923 - DNA, 12 bp, Artificial
  synthetic DNA
cacctgcacgat

SEQ ID NO: 924 - DNA, 12 bp, Artificial
  synthetic DNA
attaagcctaag

SEQ ID NO: 925 - DNA, 12 bp, Artificial
  synthetic DNA
ggtggaaccatg

SEQ ID NO: 926 - DNA, 12 bp, Artificial
  synthetic DNA
actaacgcgact

SEQ ID NO: 927 - DNA, 12 bp, Artificial
  synthetic DNA
cagttgtgctat

SEQ ID NO: 928 - DNA, 12 bp, Artificial
  synthetic DNA
acgctgttagca

SEQ ID NO: 929 - DNA, 12 bp, Artificial
  synthetic DNA
gtcaacgctaag

SEQ ID NO: 930 - DNA, 12 bp, Artificial
  synthetic DNA
agcttaggtatg

SEQ ID NO: 931 - DNA, 12 bp, Artificial
  synthetic DNA
cgcaggacgatt

SEQ ID NO: 932 - DNA, 12 bp, Artificial
  synthetic DNA
aaccggctgtct

SEQ ID NO: 933 - DNA, 12 bp, Artificial
  synthetic DNA
gttgctcacgtg

SEQ ID NO: 934 - DNA, 12 bp, Artificial
  synthetic DNA
gaatcttccgcg

SEQ ID NO: 935 - DNA, 12 bp, Artificial
  synthetic DNA
agagcgtacacg

SEQ ID NO: 936 - DNA, 12 bp, Artificial
  synthetic DNA
aaggctaatgtc

SEQ ID NO: 937 - DNA, 12 bp, Artificial
  synthetic DNA
tctatgtagacg

SEQ ID NO: 938 - DNA, 12 bp, Artificial
  synthetic DNA
agacggtctagt

SEQ ID NO: 939 - DNA, 12 bp, Artificial
  synthetic DNA
ttggtcacacgc

SEQ ID NO: 940 - DNA, 12 bp, Artificial
  synthetic DNA
gtcgatatatgg

SEQ ID NO: 941 - DNA, 12 bp, Artificial
  synthetic DNA
aacatggatacg

SEQ ID NO: 942 - DNA, 12 bp, Artificial
  synthetic DNA
ttcgcagttcct

SEQ ID NO: 943 - DNA, 12 bp, Artificial
  synthetic DNA
cgcatgttgtgc

SEQ ID NO: 944 - DNA, 12 bp, Artificial
  synthetic DNA
tgttaagttgga

SEQ ID NO: 945 - DNA, 12 bp, Artificial
  synthetic DNA
caagtgtgatga

SEQ ID NO: 946 - DNA, 12 bp, Artificial
  synthetic DNA
ctggtaccacgt

SEQ ID NO: 947 - DNA, 12 bp, Artificial
  synthetic DNA
cgctaggatcac

SEQ ID NO: 948 - DNA, 12 bp, Artificial
  synthetic DNA
tgctcattacgg

SEQ ID NO: 949 - DNA, 12 bp, Artificial
  synthetic DNA
tgctcagtaaca

SEQ ID NO: 950 - DNA, 12 bp, Artificial
  synthetic DNA
acgatcatagcc

SEQ ID NO: 951 - DNA, 12 bp, Artificial
  synthetic DNA
acgatacgtgga

SEQ ID NO: 952 - DNA, 12 bp, Artificial
  synthetic DNA
gttcgatgatgg

SEQ ID NO: 953 - DNA, 12 bp, Artificial
  synthetic DNA
aagagctgtgcc

SEQ ID NO: 954 - DNA, 12 bp, Artificial
  synthetic DNA
ggttggatcaac

SEQ ID NO: 955 - DNA, 12 bp, Artificial
  synthetic DNA
gcgcgcttatga

SEQ ID NO: 956 - DNA, 12 bp, Artificial
  synthetic DNA
cgtcgatcatca

SEQ ID NO: 957 - DNA, 12 bp, Artificial
  synthetic DNA
gagactgcactc

SEQ ID NO: 958 - DNA, 12 bp, Artificial
  synthetic DNA
gatagatcgcat

SEQ ID NO: 959 - DNA, 12 bp, Artificial
  synthetic DNA
ggccatcatcag

SEQ ID NO: 960 - DNA, 12 bp, Artificial
  synthetic DNA
ggtgttccactg

SEQ ID NO: 961 - DNA, 14 bp, Artificial
  synthetic DNA
agctatacagaggt

SEQ ID NO: 962 - DNA, 14 bp, Artificial
  synthetic DNA
aggccgttctgtct

SEQ ID NO: 963 - DNA, 14 bp, Artificial
  synthetic DNA
cattggtctgctat

SEQ ID NO: 964 - DNA, 14 bp, Artificial
  synthetic DNA
ctacatacgcgcca

SEQ ID NO: 965 - DNA, 14 bp, Artificial
  synthetic DNA
gcttaacggcgctt

SEQ ID NO: 966 - DNA, 14 bp, Artificial
  synthetic DNA
tacgatactccacc

SEQ ID NO: 967 - DNA, 14 bp, Artificial
  synthetic DNA
accggcataagaag

SEQ ID NO: 968 - DNA, 14 bp, Artificial
  synthetic DNA
ggatgcttcgataa

SEQ ID NO: 969 - DNA, 14 bp, Artificial
  synthetic DNA
gtgtacctgaatgt

SEQ ID NO: 970 - DNA, 14 bp, Artificial
  synthetic DNA
cgcggatacacaga

SEQ ID NO: 971 - DNA, 14 bp, Artificial
  synthetic DNA
ttccacggcactgt

SEQ ID NO: 972 - DNA, 14 bp, Artificial
  synthetic DNA
tagccaggcaacaa

SEQ ID NO: 973 - DNA, 14 bp, Artificial
  synthetic DNA
agcgtcaacacgta

SEQ ID NO: 974 - DNA, 14 bp, Artificial
  synthetic DNA
taacgctactcgcg

SEQ ID NO: 975 - DNA, 14 bp, Artificial
  synthetic DNA
tagatagacgatct

SEQ ID NO: 976 - DNA, 14 bp, Artificial
  synthetic DNA
actcttgcaatgct

SEQ ID NO: 977 - DNA, 14 bp, Artificial
  synthetic DNA
actcggttaggtcg

SEQ ID NO: 978 - DNA, 14 bp, Artificial
  synthetic DNA
cattatctacgcat

SEQ ID NO: 979 - DNA, 14 bp, Artificial
  synthetic DNA
cacaccggcgatta

SEQ ID NO: 980 - DNA, 14 bp, Artificial
  synthetic DNA
tacgcagtactgtg

SEQ ID NO: 981 - DNA, 14 bp, Artificial
  synthetic DNA
caagcgcgtgaatg

SEQ ID NO: 982 - DNA, 14 bp, Artificial
  synthetic DNA
gaatggactgacga

SEQ ID NO: 983 - DNA, 14 bp, Artificial
  synthetic DNA
ctagcgctgaagtt

SEQ ID NO: 984 - DNA, 14 bp, Artificial
  synthetic DNA
tgcggcagaccaat

SEQ ID NO: 985 - DNA, 14 bp, Artificial
  synthetic DNA
aaggcatagagatt

SEQ ID NO: 986 - DNA, 14 bp, Artificial
  synthetic DNA
ttctcctcgccatg

SEQ ID NO: 987 - DNA, 14 bp, Artificial
  synthetic DNA
tcattggtcgtgaa

SEQ ID NO: 988 - DNA, 14 bp, Artificial
  synthetic DNA
attacgctatacga

SEQ ID NO: 989 - DNA, 14 bp, Artificial
  synthetic DNA
atgatcctccacgg

SEQ ID NO: 990 - DNA, 14 bp, Artificial
  synthetic DNA
cgtcgttagtaatc

SEQ ID NO: 991 - DNA, 14 bp, Artificial
  synthetic DNA
tgcacatagtctca

SEQ ID NO: 992 - DNA, 14 bp, Artificial
  synthetic DNA
gtcaaggagtcacg

SEQ ID NO: 993 - DNA, 14 bp, Artificial
  synthetic DNA
ggttggaatcttgc

SEQ ID NO: 994 - DNA, 14 bp, Artificial
  synthetic DNA
catcggtgcactca

SEQ ID NO: 995 - DNA, 14 bp, Artificial
  synthetic DNA
aatgcactagacgt

SEQ ID NO: 996 - DNA, 14 bp, Artificial
  synthetic DNA
tacagtcaggctcg

SEQ ID NO: 997 - DNA, 14 bp, Artificial
  synthetic DNA
agagaagcttagcc

SEQ ID NO: 998 - DNA, 14 bp, Artificial
  synthetic DNA
ccataggatcgtat

SEQ ID NO: 999 - DNA, 14 bp, Artificial
  synthetic DNA
ttgtgctacacctg

SEQ ID NO: 1000 - DNA, 14 bp, Artificial
  synthetic DNA
ctccagtaatacta

SEQ ID NO: 1001 - DNA, 14 bp, Artificial
  synthetic DNA
tgatgccgatgtgg

SEQ ID NO: 1002 - DNA, 14 bp, Artificial
  synthetic DNA
gtcataccgcttaa

SEQ ID NO: 1003 - DNA, 14 bp, Artificial
  synthetic DNA
acgttctcttgaga

SEQ ID NO: 1004 - DNA, 14 bp, Artificial
  synthetic DNA
cagccatatcgtgt

SEQ ID NO: 1005 - DNA, 14 bp, Artificial
  synthetic DNA
ttgaacgtagcaat

SEQ ID NO: 1006 - DNA, 14 bp, Artificial
  synthetic DNA
acaatcgcggtaat

SEQ ID NO: 1007 - DNA, 14 bp, Artificial
  synthetic DNA
gttcctgtagatcc

SEQ ID NO: 1008 - DNA, 14 bp, Artificial
  synthetic DNA
agagccttacggca

SEQ ID NO: 1009 - DNA, 14 bp, Artificial
  synthetic DNA
aatatggcgccacc

SEQ ID NO: 1010 - DNA, 14 bp, Artificial
  synthetic DNA
accatataggttcg

SEQ ID NO: 1011 - DNA, 14 bp, Artificial
  synthetic DNA
atgcaccacagctg

SEQ ID NO: 1012 - DNA, 14 bp, Artificial
  synthetic DNA
ctactattgaacag

SEQ ID NO: 1013 - DNA, 14 bp, Artificial
  synthetic DNA
tgccatcactctag

SEQ ID NO: 1014 - DNA, 14 bp, Artificial
  synthetic DNA
gcgaacgagaatcg

SEQ ID NO: 1015 - DNA, 14 bp, Artificial
  synthetic DNA
gaatcaaggagacc

SEQ ID NO: 1016 - DNA, 14 bp, Artificial
  synthetic DNA
caacatctatgcag

SEQ ID NO: 1017 - DNA, 14 bp, Artificial
  synthetic DNA
caatccgtcatgga

SEQ ID NO: 1018 - DNA, 14 bp, Artificial
  synthetic DNA
agctcttagccata

SEQ ID NO: 1019 - DNA, 14 bp, Artificial
  synthetic DNA
aacaaggcaactgg

SEQ ID NO: 1020 - DNA, 14 bp, Artificial
  synthetic DNA
gtcgtcgctcctat

SEQ ID NO: 1021 - DNA, 14 bp, Artificial
  synthetic DNA
gtcatcattagatg

SEQ ID NO: 1022 - DNA, 14 bp, Artificial
  synthetic DNA
gcactaagtagcag

SEQ ID NO: 1023 - DNA, 14 bp, Artificial
  synthetic DNA
accttaccggacct

SEQ ID NO: 1024 - DNA, 14 bp, Artificial
  synthetic DNA
gctcaggtatgtca

SEQ ID NO: 1025 - DNA, 14 bp, Artificial
  synthetic DNA
tgtcacgagttagt

SEQ ID NO: 1026 - DNA, 14 bp, Artificial
  synthetic DNA
cagatgacttacgt

SEQ ID NO: 1027 - DNA, 14 bp, Artificial
  synthetic DNA
gaagtagcgattga

SEQ ID NO: 1028 - DNA, 14 bp, Artificial
  synthetic DNA
gcaggcaatctgta

SEQ ID NO: 1029 - DNA, 14 bp, Artificial
  synthetic DNA
ccttatacaacaag

SEQ ID NO: 1030 - DNA, 14 bp, Artificial
  synthetic DNA
ccttagattgattg

SEQ ID NO: 1031 - DNA, 14 bp, Artificial
  synthetic DNA
agccacgagtgata

SEQ ID NO: 1032 - DNA, 14 bp, Artificial
  synthetic DNA
ggatgactcgtgac

SEQ ID NO: 1033 - DNA, 14 bp, Artificial
  synthetic DNA
cttcgttcgccatt

SEQ ID NO: 1034 - DNA, 14 bp, Artificial
  synthetic DNA
tcttgcgtattgat

SEQ ID NO: 1035 - DNA, 14 bp, Artificial
  synthetic DNA
cttaacgtggtggc

SEQ ID NO: 1036 - DNA, 14 bp, Artificial
  synthetic DNA
tgctgttacggaag

SEQ ID NO: 1037 - DNA, 14 bp, Artificial
  synthetic DNA
ctgaattagttctc

SEQ ID NO: 1038 - DNA, 14 bp, Artificial
  synthetic DNA
cctccaagtacaga

SEQ ID NO: 1039 - DNA, 14 bp, Artificial
  synthetic DNA
ctggtaattcgcgg

SEQ ID NO: 1040 - DNA, 14 bp, Artificial
  synthetic DNA
cgactgcaatctgg

SEQ ID NO: 1041 - DNA, 14 bp, Artificial
  synthetic DNA
tggatcgcgattgg

SEQ ID NO: 1042 - DNA, 14 bp, Artificial
  synthetic DNA
cgactattcctgcg

SEQ ID NO: 1043 - DNA, 14 bp, Artificial
  synthetic DNA
caagtaggtccgtc

SEQ ID NO: 1044 - DNA, 14 bp, Artificial
  synthetic DNA
agtaatcagtgttc

SEQ ID NO: 1045 - DNA, 14 bp, Artificial
  synthetic DNA
ttattctcactacg

SEQ ID NO: 1046 - DNA, 14 bp, Artificial
  synthetic DNA
catgtcttcttcgt

SEQ ID NO: 1047 - DNA, 14 bp, Artificial
  synthetic DNA
aggcacataccatc

SEQ ID NO: 1048 - DNA, 14 bp, Artificial
  synthetic DNA
aggttagaggatgt

SEQ ID NO: 1049 - DNA, 14 bp, Artificial
  synthetic DNA
caactggcaagtgc

SEQ ID NO: 1050 - DNA, 14 bp, Artificial
  synthetic DNA
cgctcacatagagg

SEQ ID NO: 1051 - DNA, 14 bp, Artificial
  synthetic DNA
gcaatgtcgagatc

SEQ ID NO: 1052 - DNA, 14 bp, Artificial
  synthetic DNA
gttctgtggtgctc

SEQ ID NO: 1053 - DNA, 14 bp, Artificial
  synthetic DNA
aagtgatcagacta

SEQ ID NO: 1054 - DNA, 14 bp, Artificial
  synthetic DNA
attgaaggattcca

SEQ ID NO: 1055 - DNA, 14 bp, Artificial
  synthetic DNA
acgccatgctacta

SEQ ID NO: 1056 - DNA, 14 bp, Artificial
  synthetic DNA
ctgaagatgtctgc

SEQ ID NO: 1057 - DNA, 16 bp, Artificial
  synthetic DNA
gacaatctctgccgat

SEQ ID NO: 1058 - DNA, 16 bp, Artificial
  synthetic DNA
ggtccgcctaatgtaa

SEQ ID NO: 1059 - DNA, 16 bp, Artificial
  synthetic DNA
agccacaggcaattcc

SEQ ID NO: 1060 - DNA, 16 bp, Artificial
  synthetic DNA
atctcaagttctcaac

SEQ ID NO: 1061 - DNA, 16 bp, Artificial
  synthetic DNA
tgtaacgcatacgacg

SEQ ID NO: 1062 - DNA, 16 bp, Artificial
  synthetic DNA
tatctcgaataccagc

SEQ ID NO: 1063 - DNA, 16 bp, Artificial
  synthetic DNA
accgcaacacaggcaa

SEQ ID NO: 1064 - DNA, 16 bp, Artificial
  synthetic DNA
ggccagtaacatgact

SEQ ID NO: 1065 - DNA, 16 bp, Artificial
  synthetic DNA
gtgaacagttaaggtg

SEQ ID NO: 1066 - DNA, 16 bp, Artificial
  synthetic DNA
ccaggatccgtattgc

SEQ ID NO: 1067 - DNA, 16 bp, Artificial
  synthetic DNA
gacctagcactagacc

SEQ ID NO: 1068 - DNA, 16 bp, Artificial
  synthetic DNA
cgccatcctattcacg

SEQ ID NO: 1069 - DNA, 16 bp, Artificial
  synthetic DNA
aagtgcagtaatggaa

SEQ ID NO: 1070 - DNA, 16 bp, Artificial
  synthetic DNA
tcaacgcgttcgtcta

SEQ ID NO: 1071 - DNA, 16 bp, Artificial
  synthetic DNA
agcggccactatctaa

SEQ ID NO: 1072 - DNA, 16 bp, Artificial
  synthetic DNA
ctcggcgccatataga

SEQ ID NO: 1073 - DNA, 16 bp, Artificial
  synthetic DNA
cgataacttagaagaa

SEQ ID NO: 1074 - DNA, 16 bp, Artificial
  synthetic DNA
cataggatgtgacgcc

SEQ ID NO: 1075 - DNA, 16 bp, Artificial
  synthetic DNA
ggcttgtcgtcgtatc

SEQ ID NO: 1076 - DNA, 16 bp, Artificial
  synthetic DNA
cttgtctgaatattag

SEQ ID NO: 1077 - DNA, 16 bp, Artificial
  synthetic DNA
acagttcgagtgtcgg

SEQ ID NO: 1078 - DNA, 16 bp, Artificial
  synthetic DNA
ctctaacctgtgacgt

SEQ ID NO: 1079 - DNA, 16 bp, Artificial
  synthetic DNA
cgcgctaattcaacaa

SEQ ID NO: 1080 - DNA, 16 bp, Artificial
  synthetic DNA
actcacgaatgcggca

SEQ ID NO: 1081 - DNA, 16 bp, Artificial
  synthetic DNA
aatcttcggcattcat

SEQ ID NO: 1082 - DNA, 16 bp, Artificial
  synthetic DNA
aagtatcaggatcgcg

SEQ ID NO: 1083 - DNA, 16 bp, Artificial
  synthetic DNA
agtaactctgcagaca

SEQ ID NO: 1084 - DNA, 16 bp, Artificial
  synthetic DNA
ggattgaacattgtgc

SEQ ID NO: 1085 - DNA, 16 bp, Artificial
  synthetic DNA
gtgatgctcacgcatc

SEQ ID NO: 1086 - DNA, 16 bp, Artificial
  synthetic DNA
cgtagcgtaacggata

SEQ ID NO: 1087 - DNA, 16 bp, Artificial
  synthetic DNA
tgcgatgcaccgttag

SEQ ID NO: 1088 - DNA, 16 bp, Artificial
  synthetic DNA
ccagtatgctctcagg

SEQ ID NO: 1089 - DNA, 16 bp, Artificial
  synthetic DNA
aatgacgttgaagcct

SEQ ID NO: 1090 - DNA, 16 bp, Artificial
  synthetic DNA
tcgattctataggagt

SEQ ID NO: 1091 - DNA, 16 bp, Artificial
  synthetic DNA
cgataggttcagctat

SEQ ID NO: 1092 - DNA, 16 bp, Artificial
  synthetic DNA
ccatgttgatagaata

SEQ ID NO: 1093 - DNA, 16 bp, Artificial
  synthetic DNA
gagccacttctacagg

SEQ ID NO: 1094 - DNA, 16 bp, Artificial
  synthetic DNA
gcgaactctcggtaat

SEQ ID NO: 1095 - DNA, 16 bp, Artificial
  synthetic DNA
gacctgagtagctggt

SEQ ID NO: 1096 - DNA, 16 bp, Artificial
  synthetic DNA
cgagtctattagcctg

SEQ ID NO: 1097 - DNA, 16 bp, Artificial
  synthetic DNA
gtagtgccatacacct

SEQ ID NO: 1098 - DNA, 16 bp, Artificial
  synthetic DNA
ccagtggtctatagca

SEQ ID NO: 1099 - DNA, 16 bp, Artificial
  synthetic DNA
gtcagtgcgttattgc

SEQ ID NO: 1100 - DNA, 16 bp, Artificial
  synthetic DNA
agtgtcggagtgacga

SEQ ID NO: 1101 - DNA, 16 bp, Artificial
  synthetic DNA
aatctccgctatagtt

SEQ ID NO: 1102 - DNA, 16 bp, Artificial
  synthetic DNA
cgagtaggtctgactt

SEQ ID NO: 1103 - DNA, 16 bp, Artificial
  synthetic DNA
ctgtcgctctaataac

SEQ ID NO: 1104 - DNA, 16 bp, Artificial
  synthetic DNA
gctgtcaatataactg

SEQ ID NO: 1105 - DNA, 16 bp, Artificial
  synthetic DNA
agctcaagttgaatcc

SEQ ID NO: 1106 - DNA, 16 bp, Artificial
  synthetic DNA
aattcatgctcctaac

SEQ ID NO: 1107 - DNA, 16 bp, Artificial
  synthetic DNA
ccaaggtctggtgata

SEQ ID NO: 1108 - DNA, 16 bp, Artificial
  synthetic DNA
ctccacgtatcttgaa

SEQ ID NO: 1109 - DNA, 16 bp, Artificial
  synthetic DNA
tagccgaacaacactt

SEQ ID NO: 1110 - DNA, 16 bp, Artificial
  synthetic DNA
agtacacgacatatgc

SEQ ID NO: 1111 - DNA, 16 bp, Artificial
  synthetic DNA
acgttctagactcctg

SEQ ID NO: 1112 - DNA, 16 bp, Artificial
  synthetic DNA
cgactcaagcactgct

SEQ ID NO: 1113 - DNA, 16 bp, Artificial
  synthetic DNA
tgaagctcacgattaa

SEQ ID NO: 1114 - DNA, 16 bp, Artificial
  synthetic DNA
tatctaacgtatggta

SEQ ID NO: 1115 - DNA, 16 bp, Artificial
  synthetic DNA
tataccatgttccttg

SEQ ID NO: 1116 - DNA, 16 bp, Artificial
  synthetic DNA
ttcctacgatgacttc

SEQ ID NO: 1117 - DNA, 16 bp, Artificial
  synthetic DNA
ctctccaatatgtgcc

SEQ ID NO: 1118 - DNA, 16 bp, Artificial
  synthetic DNA
gagtagagtcttgcca

SEQ ID NO: 1119 - DNA, 16 bp, Artificial
  synthetic DNA
gcgagatgtggtccta

SEQ ID NO: 1120 - DNA, 16 bp, Artificial
  synthetic DNA
aagctacacggaccac

SEQ ID NO: 1121 - DNA, 16 bp, Artificial
  synthetic DNA
atacaactggcaaccg

SEQ ID NO: 1122 - DNA, 16 bp, Artificial
  synthetic DNA
cggtagatgctatgct

SEQ ID NO: 1123 - DNA, 16 bp, Artificial
  synthetic DNA
tcttgaccggtcatca

SEQ ID NO: 1124 - DNA, 16 bp, Artificial
  synthetic DNA
agatcgtgcatgcgat

SEQ ID NO: 1125 - DNA, 16 bp, Artificial
  synthetic DNA
tcctcgagacagcctt

SEQ ID NO: 1126 - DNA, 16 bp, Artificial
  synthetic DNA
tagccggtaccactta

SEQ ID NO: 1127 - DNA, 16 bp, Artificial
  synthetic DNA
gtaaggcagcgtgcaa

SEQ ID NO: 1128 - DNA, 16 bp, Artificial
  synthetic DNA
tagtctgctcctggtc

SEQ ID NO: 1129 - DNA, 16 bp, Artificial
  synthetic DNA
tggattatagcagcag

SEQ ID NO: 1130 - DNA, 16 bp, Artificial
  synthetic DNA
aagaatgatcagacat

SEQ ID NO: 1131 - DNA, 16 bp, Artificial
  synthetic DNA
cagcgctatatacctc

SEQ ID NO: 1132 - DNA, 16 bp, Artificial
  synthetic DNA
gagtagtacctccacc

SEQ ID NO: 1133 - DNA, 16 bp, Artificial
  synthetic DNA
gacgtgatcctctaga

SEQ ID NO: 1134 - DNA, 16 bp, Artificial
  synthetic DNA
gttccgttcactacga

SEQ ID NO: 1135 - DNA, 16 bp, Artificial
  synthetic DNA
tgcaagcaccaggatg

SEQ ID NO: 1136 - DNA, 16 bp, Artificial
  synthetic DNA
ttagttggcggctgag

SEQ ID NO: 1137 - DNA, 16 bp, Artificial
  synthetic DNA
cagatgcagacatacg

SEQ ID NO: 1138 - DNA, 16 bp, Artificial
  synthetic DNA
gacgcttgatgattat

SEQ ID NO: 1139 - DNA, 16 bp, Artificial
  synthetic DNA
tggatcacgactagga

SEQ ID NO: 1140 - DNA, 16 bp, Artificial
  synthetic DNA
ctcgtcggtataacgc

SEQ ID NO: 1141 - DNA, 16 bp, Artificial
  synthetic DNA
aagcacggatgcgatt

SEQ ID NO: 1142 - DNA, 16 bp, Artificial
  synthetic DNA
agatcttccggtgaac

SEQ ID NO: 1143 - DNA, 16 bp, Artificial
  synthetic DNA
ggacaatagcaacctg

SEQ ID NO: 1144 - DNA, 16 bp, Artificial
  synthetic DNA
gataatcggttccaat

SEQ ID NO: 1145 - DNA, 16 bp, Artificial
  synthetic DNA
ctcaagctacagttgt

SEQ ID NO: 1146 - DNA, 16 bp, Artificial
  synthetic DNA
gttggcatgatgtaga

SEQ ID NO: 1147 - DNA, 16 bp, Artificial
  synthetic DNA
cagcatgaggtaagtg

SEQ ID NO: 1148 - DNA, 16 bp, Artificial
  synthetic DNA
gcctcatcacacgtca

SEQ ID NO: 1149 - DNA, 16 bp, Artificial
  synthetic DNA
tcgatactacacatcg

SEQ ID NO: 1150 - DNA, 16 bp, Artificial
  synthetic DNA
tacacgaggcttgatc

SEQ ID NO: 1151 - DNA, 16 bp, Artificial
  synthetic DNA
ttctcgtgtccgcatt

SEQ ID NO: 1152 - DNA, 16 bp, Artificial
  synthetic DNA
ggtgaagcaacagcat

SEQ ID NO: 1153 - DNA, 18 bp, Artificial
  synthetic DNA
cgaaccgactgtacagtt

SEQ ID NO: 1154 - DNA, 18 bp, Artificial
  synthetic DNA
ccgactgcggataagtta

SEQ ID NO: 1155 - DNA, 18 bp, Artificial
  synthetic DNA
cgacaggtaggtaagcag

SEQ ID NO: 1156 - DNA, 18 bp, Artificial
  synthetic DNA
tgatacgttggtatacag

SEQ ID NO: 1157 - DNA, 18 bp, Artificial
  synthetic DNA
ctactatagaatacgtag

SEQ ID NO: 1158 - DNA, 18 bp, Artificial
  synthetic DNA
agactgtggcaatggcat

SEQ ID NO: 1159 - DNA, 18 bp, Artificial
  synthetic DNA
ggaagactgatacaacga

SEQ ID NO: 1160 - DNA, 18 bp, Artificial
  synthetic DNA
tatgcacatatagcgctt

SEQ ID NO: 1161 - DNA, 18 bp, Artificial
  synthetic DNA
catggtaatcgaccgagg

SEQ ID NO: 1162 - DNA, 18 bp, Artificial
  synthetic DNA
gtcattgccgtcattgcc

SEQ ID NO: 1163 - DNA, 18 bp, Artificial
  synthetic DNA
cctaagaactccgaagct

SEQ ID NO: 1164 - DNA, 18 bp, Artificial
  synthetic DNA
tcgctcaccgtactagga

SEQ ID NO: 1165 - DNA, 18 bp, Artificial
  synthetic DNA
tattactgtcacagcagg

SEQ ID NO: 1166 - DNA, 18 bp, Artificial
  synthetic DNA
tgagacaggctacgagtc

SEQ ID NO: 1167 - DNA, 18 bp, Artificial
  synthetic DNA
aagctatgcgaacacgtt

SEQ ID NO: 1168 - DNA, 18 bp, Artificial
  synthetic DNA
aacggaggagtgagccaa

SEQ ID NO: 1169 - DNA, 18 bp, Artificial
  synthetic DNA
ccactatggacatcatgg

SEQ ID NO: 1170 - DNA, 18 bp, Artificial
  synthetic DNA
atggtggtggatagctcg

SEQ ID NO: 1171 - DNA, 18 bp, Artificial
  synthetic DNA
tcaccggttacacatcgc

SEQ ID NO: 1172 - DNA, 18 bp, Artificial
  synthetic DNA
aagatactgagatatgga

SEQ ID NO: 1173 - DNA, 18 bp, Artificial
  synthetic DNA
gacctgttcttgaactag

SEQ ID NO: 1174 - DNA, 18 bp, Artificial
  synthetic DNA
aagtagagctctcggtta

SEQ ID NO: 1175 - DNA, 18 bp, Artificial
  synthetic DNA
ctatgttcttactctctt

SEQ ID NO: 1176 - DNA, 18 bp, Artificial
  synthetic DNA
caaggctataagcggtta

SEQ ID NO: 1177 - DNA, 18 bp, Artificial
  synthetic DNA
gaagctaattaaccgata

SEQ ID NO: 1178 - DNA, 18 bp, Artificial
  synthetic DNA
ttcacgtctgccaagcac

SEQ ID NO: 1179 - DNA, 18 bp, Artificial
  synthetic DNA
atcgtatagatcgagaca

SEQ ID NO: 1180 - DNA, 18 bp, Artificial
  synthetic DNA
gtcacagattcacatcat

SEQ ID NO: 1181 - DNA, 18 bp, Artificial
  synthetic DNA
gtgcctgtgaactatcag

SEQ ID NO: 1182 - DNA, 18 bp, Artificial
  synthetic DNA
cagcgtacaagatagtcg

SEQ ID NO: 1183 - DNA, 18 bp, Artificial
  synthetic DNA
gcatggcatggtagacct

SEQ ID NO: 1184 - DNA, 18 bp, Artificial
  synthetic DNA
ggtatgctactcttcgca

SEQ ID NO: 1185 - DNA, 18 bp, Artificial
  synthetic DNA
atgttcagtcacaagcga

SEQ ID NO: 1186 - DNA, 18 bp, Artificial
  synthetic DNA
taggaagtgtgtaatagc

SEQ ID NO: 1187 - DNA, 18 bp, Artificial
  synthetic DNA
aatccatgtagctgtacg

SEQ ID NO: 1188 - DNA, 18 bp, Artificial
  synthetic DNA
ccagattcactggcatag

SEQ ID NO: 1189 - DNA, 18 bp, Artificial
  synthetic DNA
ttgtctctacgtaatatc

SEQ ID NO: 1190 - DNA, 18 bp, Artificial
  synthetic DNA
gtggtgcttgtgacaatt

SEQ ID NO: 1191 - DNA, 18 bp, Artificial
  synthetic DNA
cagcctacttggctgaga

SEQ ID NO: 1192 - DNA, 18 bp, Artificial
  synthetic DNA
tactcaatgcatctgtgt

SEQ ID NO: 1193 - DNA, 18 bp, Artificial
  synthetic DNA
tgtagagagacgaatata

SEQ ID NO: 1194 - DNA, 18 bp, Artificial
  synthetic DNA
gcctacaaccatcctact

SEQ ID NO: 1195 - DNA, 18 bp, Artificial
  synthetic DNA
gcgtggcattgagattca

SEQ ID NO: 1196 - DNA, 18 bp, Artificial
  synthetic DNA
gcatgccagctaactgag

SEQ ID NO: 1197 - DNA, 18 bp, Artificial
  synthetic DNA
gcgagtaatccggttgga

SEQ ID NO: 1198 - DNA, 18 bp, Artificial
  synthetic DNA
gcctctaccagaacgtca

SEQ ID NO: 1199 - DNA, 18 bp, Artificial
  synthetic DNA
gtcagcagaagactgacc

SEQ ID NO: 1200 - DNA, 18 bp, Artificial
  synthetic DNA
gataacagacgtagcagg

SEQ ID NO: 1201 - DNA, 18 bp, Artificial
  synthetic DNA
caggagatcgcatgtcgt

SEQ ID NO: 1202 - DNA, 18 bp, Artificial
  synthetic DNA
ctggaaggaatggagcca

SEQ ID NO: 1203 - DNA, 18 bp, Artificial
  synthetic DNA
attggttctctaccacaa

SEQ ID NO: 1204 - DNA, 18 bp, Artificial
  synthetic DNA
ctcattgttgacggctca

SEQ ID NO: 1205 - DNA, 18 bp, Artificial
  synthetic DNA
ttcaggactgtagttcat

SEQ ID NO: 1206 - DNA, 18 bp, Artificial
  synthetic DNA
agaccgcactaactcaag

SEQ ID NO: 1207 - DNA, 18 bp, Artificial
  synthetic DNA
ggaatattgtgcagaccg

SEQ ID NO: 1208 - DNA, 18 bp, Artificial
  synthetic DNA
cctattactaatagctca

SEQ ID NO: 1209 - DNA, 18 bp, Artificial
  synthetic DNA
atggcatgagtacttcgg

SEQ ID NO: 1210 - DNA, 18 bp, Artificial
  synthetic DNA
gacacgtatgcgtctagc

SEQ ID NO: 1211 - DNA, 18 bp, Artificial
  synthetic DNA
gaaggtacggaatctgtt

SEQ ID NO: 1212 - DNA, 18 bp, Artificial
  synthetic DNA
tataacgtccgacactgt

SEQ ID NO: 1213 - DNA, 18 bp, Artificial
  synthetic DNA
gctaatacattaccgccg

SEQ ID NO: 1214 - DNA, 18 bp, Artificial
  synthetic DNA
gaagccaacactcctgac

SEQ ID NO: 1215 - DNA, 18 bp, Artificial
  synthetic DNA
cgaataacgagctgtgat

SEQ ID NO: 1216 - DNA, 18 bp, Artificial
  synthetic DNA
gcctaccgatcgcactta

SEQ ID NO: 1217 - DNA, 18 bp, Artificial
  synthetic DNA
ctgaggagaatagcctgc

SEQ ID NO: 1218 - DNA, 18 bp, Artificial
  synthetic DNA
cagcatggacagtacttc

SEQ ID NO: 1219 - DNA, 18 bp, Artificial
  synthetic DNA
ggtatagagccttcctta

SEQ ID NO: 1220 - DNA, 18 bp, Artificial
  synthetic DNA
cgctctgcatatatagca

SEQ ID NO: 1221 - DNA, 18 bp, Artificial
  synthetic DNA
cggctctactatgctcgt

SEQ ID NO: 1222 - DNA, 18 bp, Artificial
  synthetic DNA
cctaatgcgaagctcacc

SEQ ID NO: 1223 - DNA, 18 bp, Artificial
  synthetic DNA
acaaccggtgaggcagta

SEQ ID NO: 1224 - DNA, 18 bp, Artificial
  synthetic DNA
ttggttcgaaccaaccgc

SEQ ID NO: 1225 - DNA, 18 bp, Artificial
  synthetic DNA
atactaggttgaactaag

SEQ ID NO: 1226 - DNA, 18 bp, Artificial
  synthetic DNA
gcgttgagagtaacatat

SEQ ID NO: 1227 - DNA, 18 bp, Artificial
  synthetic DNA
agttgtataataagcgtc

SEQ ID NO: 1228 - DNA, 18 bp, Artificial
  synthetic DNA
gtatgatgccgtccaatt

SEQ ID NO: 1229 - DNA, 18 bp, Artificial
  synthetic DNA
ggactctctgaagagtct

SEQ ID NO: 1230 - DNA, 18 bp, Artificial
  synthetic DNA
ggactctcttgacttgaa

SEQ ID NO: 1231 - DNA, 18 bp, Artificial
  synthetic DNA
gataacagtgcttcgtcc

SEQ ID NO: 1232 - DNA, 18 bp, Artificial
  synthetic DNA
ggccattatagatgaact

SEQ ID NO: 1233 - DNA, 18 bp, Artificial
  synthetic DNA
atagagagcacagagcag

SEQ ID NO: 1234 - DNA, 18 bp, Artificial
  synthetic DNA
gtgtgagtgtatcataac

SEQ ID NO: 1235 - DNA, 18 bp, Artificial
  synthetic DNA
ataaccttagtgcgcgtc

SEQ ID NO: 1236 - DNA, 18 bp, Artificial
  synthetic DNA
ccgactgatatgcatgga

SEQ ID NO: 1237 - DNA, 18 bp, Artificial
  synthetic DNA
ggatatctgatcgcatca

SEQ ID NO: 1238 - DNA, 18 bp, Artificial
  synthetic DNA
cagcattaacgaggcgaa

SEQ ID NO: 1239 - DNA, 18 bp, Artificial
  synthetic DNA
gcgaggcctacatattcg

SEQ ID NO: 1240 - DNA, 18 bp, Artificial
  synthetic DNA
cgataagtggtaaggtct

SEQ ID NO: 1241 - DNA, 18 bp, Artificial
  synthetic DNA
agatcctgagtcgagcaa

SEQ ID NO: 1242 - DNA, 18 bp, Artificial
  synthetic DNA
aagatataacgagaccga

SEQ ID NO: 1243 - DNA, 18 bp, Artificial
  synthetic DNA
ccgactgattgagaacgt

SEQ ID NO: 1244 - DNA, 18 bp, Artificial
  synthetic DNA
tcggcttatatgacacgt

SEQ ID NO: 1245 - DNA, 18 bp, Artificial
  synthetic DNA
aataacgtacgccggagg

SEQ ID NO: 1246 - DNA, 18 bp, Artificial
  synthetic DNA
aacacagcattgcgcacg

SEQ ID NO: 1247 - DNA, 18 bp, Artificial
  synthetic DNA
gtagtctgacagcaacaa

SEQ ID NO: 1248 - DNA, 18 bp, Artificial
  synthetic DNA
agaatgacttgagctgct

SEQ ID NO: 1249 - DNA, 20 bp, Artificial
  synthetic DNA
actggtagtaacgtccacct

SEQ ID NO: 1250 - DNA, 20 bp, Artificial
  synthetic DNA
agactggttgttattcgcct

SEQ ID NO: 1251 - DNA, 20 bp, Artificial
  synthetic DNA
tatcattgacagcgagctca

SEQ ID NO: 1252 - DNA, 20 bp, Artificial
  synthetic DNA
tggagtctgaagaaggactc

SEQ ID NO: 1253 - DNA, 20 bp, Artificial
  synthetic DNA
catctggactacggcaacga

SEQ ID NO: 1254 - DNA, 20 bp, Artificial
  synthetic DNA
aactgtcataagacagacaa

SEQ ID NO: 1255 - DNA, 20 bp, Artificial
  synthetic DNA
cctcaacatgacatacaccg

SEQ ID NO: 1256 - DNA, 20 bp, Artificial
  synthetic DNA
caataccgttcgcgattcta

SEQ ID NO: 1257 - DNA, 20 bp, Artificial
  synthetic DNA
gcgtctacgttgattcggcc

SEQ ID NO: 1258 - DNA, 20 bp, Artificial
  synthetic DNA
tgaacagaggcacttgcagg

SEQ ID NO: 1259 - DNA, 20 bp, Artificial
  synthetic DNA
cgactagaacctactactgc

SEQ ID NO: 1260 - DNA, 20 bp, Artificial
  synthetic DNA
gcaccgcacgtggagagata

SEQ ID NO: 1261 - DNA, 20 bp, Artificial
  synthetic DNA
ctgagagaccgactgatgcg

SEQ ID NO: 1262 - DNA, 20 bp, Artificial
  synthetic DNA
tcgtccttctacttaatgat

SEQ ID NO: 1263 - DNA, 20 bp, Artificial
  synthetic DNA
caagctataccatccgaatt

SEQ ID NO: 1264 - DNA, 20 bp, Artificial
  synthetic DNA
caatacgtatagtcttagat

SEQ ID NO: 1265 - DNA, 20 bp, Artificial
  synthetic DNA
ccatccacagtgacctatgt

SEQ ID NO: 1266 - DNA, 20 bp, Artificial
  synthetic DNA
tatccgttggagaaggttca

SEQ ID NO: 1267 - DNA, 20 bp, Artificial
  synthetic DNA
cgcctaggtacctgagtacg

SEQ ID NO: 1268 - DNA, 20 bp, Artificial
  synthetic DNA
cagagtgctcgtgttcgcga

SEQ ID NO: 1269 - DNA, 20 bp, Artificial
  synthetic DNA
cgcttggacatccttaagaa

SEQ ID NO: 1270 - DNA, 20 bp, Artificial
  synthetic DNA
gaccgcatgattagtcttac

SEQ ID NO: 1271 - DNA, 20 bp, Artificial
  synthetic DNA
cttggccgtagtcactcagt

SEQ ID NO: 1272 - DNA, 20 bp, Artificial
  synthetic DNA
gatagcgatattcagttcgc

SEQ ID NO: 1273 - DNA, 20 bp, Artificial
  synthetic DNA
atccaacactaagacaacca

SEQ ID NO: 1274 - DNA, 20 bp, Artificial
  synthetic DNA
ccattctgttgcgtgtcctc

SEQ ID NO: 1275 - DNA, 20 bp, Artificial
  synthetic DNA
acattctgtacgcttgcagc

SEQ ID NO: 1276 - DNA, 20 bp, Artificial
  synthetic DNA
tgctgaacgccaatcgctta

SEQ ID NO: 1277 - DNA, 20 bp, Artificial
  synthetic DNA
tcctctacaagaatattgcg

SEQ ID NO: 1278 - DNA, 20 bp, Artificial
  synthetic DNA
cgaccaacgcagcctgattc

SEQ ID NO: 1279 - DNA, 20 bp, Artificial
  synthetic DNA
attgcgagcttgagtagcgc

SEQ ID NO: 1280 - DNA, 20 bp, Artificial
  synthetic DNA
aaggtgcgagcataggaatc

SEQ ID NO: 1281 - DNA, 20 bp, Artificial
  synthetic DNA
cacttaagtgtgatatagat

SEQ ID NO: 1282 - DNA, 20 bp, Artificial
  synthetic DNA
atcggtatgctgacctagac

SEQ ID NO: 1283 - DNA, 20 bp, Artificial
  synthetic DNA
tacaatctcgaatgcaggat

SEQ ID NO: 1284 - DNA, 20 bp, Artificial
  synthetic DNA
ccatatgaagcgcagccgtc

SEQ ID NO: 1285 - DNA, 20 bp, Artificial
  synthetic DNA
cgtctcgtggacattcgagg

SEQ ID NO: 1286 - DNA, 20 bp, Artificial
  synthetic DNA
ccgagtacagaagcgtggaa

SEQ ID NO: 1287 - DNA, 20 bp, Artificial
  synthetic DNA
ttacgtggtcgacaggcagt

SEQ ID NO: 1288 - DNA, 20 bp, Artificial
  synthetic DNA
agctgcaatctgcatgatta

SEQ ID NO: 1289 - DNA, 20 bp, Artificial
  synthetic DNA
acctgccgaagcagcctaca

SEQ ID NO: 1290 - DNA, 20 bp, Artificial
  synthetic DNA
aacatgataaccacatggtt

SEQ ID NO: 1291 - DNA, 20 bp, Artificial
  synthetic DNA
atccgactgattgaattacc

SEQ ID NO: 1292 - DNA, 20 bp, Artificial
  synthetic DNA
tcacgctgactcttatcagg

SEQ ID NO: 1293 - DNA, 20 bp, Artificial
  synthetic DNA
gcgcgctcgaagtacaacat

SEQ ID NO: 1294 - DNA, 20 bp, Artificial
  synthetic DNA
acagccagatgcgttgttcc

SEQ ID NO: 1295 - DNA, 20 bp, Artificial
  synthetic DNA
ggagctctgacctgcaagaa

SEQ ID NO: 1296 - DNA, 20 bp, Artificial
  synthetic DNA
aacattagcctcaagtaaga

SEQ ID NO: 1297 - DNA, 20 bp, Artificial
  synthetic DNA
tgtgattatgccgaatgagg

SEQ ID NO: 1298 - DNA, 20 bp, Artificial
  synthetic DNA
gagtaataatccaatcagta

SEQ ID NO: 1299 - DNA, 20 bp, Artificial
  synthetic DNA
ctccttggcgacagctgaac

SEQ ID NO: 1300 - DNA, 20 bp, Artificial
  synthetic DNA
ttacgcacacatacacagac

SEQ ID NO: 1301 - DNA, 20 bp, Artificial
  synthetic DNA
acgccgtatggcgacttagg

SEQ ID NO: 1302 - DNA, 20 bp, Artificial
  synthetic DNA
agaacgacaattacgatggc

SEQ ID NO: 1303 - DNA, 20 bp, Artificial
  synthetic DNA
tgctaacgtaccactgccac

SEQ ID NO: 1304 - DNA, 20 bp, Artificial
  synthetic DNA
catccagaatgtctatcata

SEQ ID NO: 1305 - DNA, 20 bp, Artificial
  synthetic DNA
ggagaacgcctatagcactc

SEQ ID NO: 1306 - DNA, 20 bp, Artificial
  synthetic DNA
acctcttgtgacggccagtc

SEQ ID NO: 1307 - DNA, 20 bp, Artificial
  synthetic DNA
tgccataacttggcataaga

SEQ ID NO: 1308 - DNA, 20 bp, Artificial
  synthetic DNA
acaattgtctgaccacgctc

SEQ ID NO: 1309 - DNA, 20 bp, Artificial
  synthetic DNA
tcgtcaccttcacagaacga

SEQ ID NO: 1310 - DNA, 20 bp, Artificial
  synthetic DNA
agcagcagatgatgatccaa

SEQ ID NO: 1311 - DNA, 20 bp, Artificial
  synthetic DNA
tcgtgccttggattccagga

SEQ ID NO: 1312 - DNA, 20 bp, Artificial
  synthetic DNA
tgttatagccacgatactat

SEQ ID NO: 1313 - DNA, 20 bp, Artificial
  synthetic DNA
aatctcacctgtaccttccg

SEQ ID NO: 1314 - DNA, 20 bp, Artificial
  synthetic DNA
gagtagcggaagcgttagcg

SEQ ID NO: 1315 - DNA, 20 bp, Artificial
  synthetic DNA
aatactccggcgaggtatac

SEQ ID NO: 1316 - DNA, 20 bp, Artificial
  synthetic DNA
ttcgcatccttgcacgaaca

SEQ ID NO: 1317 - DNA, 20 bp, Artificial
  synthetic DNA
aaccggctaatactactggc

SEQ ID NO: 1318 - DNA, 20 bp, Artificial
  synthetic DNA
ctagcatcttagacaccaga

SEQ ID NO: 1319 - DNA, 20 bp, Artificial
  synthetic DNA
tagttgcgtgatacaagata

SEQ ID NO: 1320 - DNA, 20 bp, Artificial
  synthetic DNA
tcgtctcgacacagttggtc

SEQ ID NO: 1321 - DNA, 20 bp, Artificial
  synthetic DNA
tccgttcgcgtgcgaactga

SEQ ID NO: 1322 - DNA, 20 bp, Artificial
  synthetic DNA
tctgactctggtgtacagtc

SEQ ID NO: 1323 - DNA, 20 bp, Artificial
  synthetic DNA
acagcgcaattatatcctgt

SEQ ID NO: 1324 - DNA, 20 bp, Artificial
  synthetic DNA
agatccgtacgtgagactag

SEQ ID NO: 1325 - DNA, 20 bp, Artificial
  synthetic DNA
tacattgaagcatccgaaca

SEQ ID NO: 1326 - DNA, 20 bp, Artificial
  synthetic DNA
ctcctgagagatcaacgcca

SEQ ID NO: 1327 - DNA, 20 bp, Artificial
  synthetic DNA
tcacctcgaatgagttcgtt

SEQ ID NO: 1328 - DNA, 20 bp, Artificial
  synthetic DNA
tagcgacttaaggtccaagc

SEQ ID NO: 1329 - DNA, 20 bp, Artificial
  synthetic DNA
agtacgtattgccgtgcaag

SEQ ID NO: 1330 - DNA, 20 bp, Artificial
  synthetic DNA
agccacgaaccgacgtcata

SEQ ID NO: 1331 - DNA, 20 bp, Artificial
  synthetic DNA
tgatgtgtacgctactacta

SEQ ID NO: 1332 - DNA, 20 bp, Artificial
  synthetic DNA
ccactgtgtgcagcagacga

SEQ ID NO: 1333 - DNA, 20 bp, Artificial
  synthetic DNA
ctattgtacagcgaacgctg

SEQ ID NO: 1334 - DNA, 20 bp, Artificial
  synthetic DNA
ctccgatatcgcacggatcg

SEQ ID NO: 1335 - DNA, 20 bp, Artificial
  synthetic DNA
aacttatcgtcggacgcatg

SEQ ID NO: 1336 - DNA, 20 bp, Artificial
  synthetic DNA
tatcctaattcgtgccggtc

SEQ ID NO: 1337 - DNA, 20 bp, Artificial
  synthetic DNA
acagccttcctgtgtggact

SEQ ID NO: 1338 - DNA, 20 bp, Artificial
  synthetic DNA
cctccgtgaggatcgtacca

SEQ ID NO: 1339 - DNA, 20 bp, Artificial
  synthetic DNA
gctctaagtaacagaactaa

SEQ ID NO: 1340 - DNA, 20 bp, Artificial
  synthetic DNA
gacttaccgcgcgttctggt

SEQ ID NO: 1341 - DNA, 20 bp, Artificial
  synthetic DNA
tctgaggatacacatgtgga

SEQ ID NO: 1342 - DNA, 20 bp, Artificial
  synthetic DNA
tgtaatcacactggtgtcgg

SEQ ID NO: 1343 - DNA, 20 bp, Artificial
  synthetic DNA
cactaggcggcagacataca

SEQ ID NO: 1344 - DNA, 20 bp, Artificial
  synthetic DNA
ctagagcacagtaccacgtt

SEQ ID NO: 1345 - DNA, 22 bp, Artificial
  synthetic DNA
ttcagaggtctacgcttccggt

SEQ ID NO: 1346 - DNA, 22 bp, Artificial
  synthetic DNA
aacacagactgcgttatgccaa

SEQ ID NO: 1347 - DNA, 22 bp, Artificial
  synthetic DNA
tgctgagttctatacagcagtg

SEQ ID NO: 1348 - DNA, 22 bp, Artificial
  synthetic DNA
acctattatatgatagcgtcat

SEQ ID NO: 1349 - DNA, 22 bp, Artificial
  synthetic DNA
atcgtgagctacagtgaatgca

SEQ ID NO: 1350 - DNA, 22 bp, Artificial
  synthetic DNA
cgtgatgtatccggccttgcag

SEQ ID NO: 1351 - DNA, 22 bp, Artificial
  synthetic DNA
tcttctggtcctagagttgtgc

SEQ ID NO: 1352 - DNA, 22 bp, Artificial
  synthetic DNA
tgatgtcggcggcggatcagat

SEQ ID NO: 1353 - DNA, 22 bp, Artificial
  synthetic DNA
tcggccttagcgttcagcatcc

SEQ ID NO: 1354 - DNA, 22 bp, Artificial
  synthetic DNA
ttaagtaggtcagccactgcac

SEQ ID NO: 1355 - DNA, 22 bp, Artificial
  synthetic DNA
ccaggtgagttgatctgacacc

SEQ ID NO: 1356 - DNA, 22 bp, Artificial
  synthetic DNA
tatactattactgtgttcgatc

SEQ ID NO: 1357 - DNA, 22 bp, Artificial
  synthetic DNA
ccgcagtatgtctagtgttgtc

SEQ ID NO: 1358 - DNA, 22 bp, Artificial
  synthetic DNA
gtctaccgcgtacgaagctctc

SEQ ID NO: 1359 - DNA, 22 bp, Artificial
  synthetic DNA
atgcgagtccgtggtcgatcct

SEQ ID NO: 1360 - DNA, 22 bp, Artificial
  synthetic DNA
tggtagattggtgtgagaacta

SEQ ID NO: 1361 - DNA, 22 bp, Artificial
  synthetic DNA
aggttcgtcgatcaactgctaa

SEQ ID NO: 1362 - DNA, 22 bp, Artificial
  synthetic DNA
acgacaagcatcctgcgatatc

SEQ ID NO: 1363 - DNA, 22 bp, Artificial
  synthetic DNA
ttgaatcacagagagcgtgatt

SEQ ID NO: 1364 - DNA, 22 bp, Artificial
  synthetic DNA
gtacttagtgcttacgtcagct

SEQ ID NO: 1365 - DNA, 22 bp, Artificial
  synthetic DNA
gattattaaggccaagctcata

SEQ ID NO: 1366 - DNA, 22 bp, Artificial
  synthetic DNA
gcatgcagagacgtactcatcg

SEQ ID NO: 1367 - DNA, 22 bp, Artificial
  synthetic DNA
tagcggatggtgtcctggcact

SEQ ID NO: 1368 - DNA, 22 bp, Artificial
  synthetic DNA
tacggctgccaacttaataact

SEQ ID NO: 1369 - DNA, 22 bp, Artificial
  synthetic DNA
ctcatatgacaacttctatagt

SEQ ID NO: 1370 - DNA, 22 bp, Artificial
  synthetic DNA
caagcaatagttgtcggccacc

SEQ ID NO: 1371 - DNA, 22 bp, Artificial
  synthetic DNA
ttcagcaatccgtactgctaga

SEQ ID NO: 1372 - DNA, 22 bp, Artificial
  synthetic DNA
tgagacgttgctgacattctcc

SEQ ID NO: 1373 - DNA, 22 bp, Artificial
  synthetic DNA
gttccgatgagttagatgtata

SEQ ID NO: 1374 - DNA, 22 bp, Artificial
  synthetic DNA
ttgacgcttggaggagtacaag

SEQ ID NO: 1375 - DNA, 22 bp, Artificial
  synthetic DNA
ttcatgttacctccacattgtg

SEQ ID NO: 1376 - DNA, 22 bp, Artificial
  synthetic DNA
gagcacgtgccagattgcaacc

SEQ ID NO: 1377 - DNA, 22 bp, Artificial
  synthetic DNA
ggtcgacaagcacaagccttct

SEQ ID NO: 1378 - DNA, 22 bp, Artificial
  synthetic DNA
taggcaggtaagatgaccgact

SEQ ID NO: 1379 - DNA, 22 bp, Artificial
  synthetic DNA
cgaggcatgccaagtcgccaat

SEQ ID NO: 1380 - DNA, 22 bp, Artificial
  synthetic DNA
agtgttgataggcggatgagag

SEQ ID NO: 1381 - DNA, 22 bp, Artificial
  synthetic DNA
ttcggtctagacctctcacaat

SEQ ID NO: 1382 - DNA, 22 bp, Artificial
  synthetic DNA
gtgacgctcatatcttgccacc

SEQ ID NO: 1383 - DNA, 22 bp, Artificial
  synthetic DNA
gatgtaattctacgcgcggact

SEQ ID NO: 1384 - DNA, 22 bp, Artificial
  synthetic DNA
gatggcgatgttgcattacatg

SEQ ID NO: 1385 - DNA, 22 bp, Artificial
  synthetic DNA
tatgctctgaattaacgtagaa

SEQ ID NO: 1386 - DNA, 22 bp, Artificial
  synthetic DNA
aggcaatatggtgatccgtagc

SEQ ID NO: 1387 - DNA, 22 bp, Artificial
  synthetic DNA
tgacagcgatgcatacagtagt

SEQ ID NO: 1388 - DNA, 22 bp, Artificial
  synthetic DNA
ttctgctaacggtatccaatac

SEQ ID NO: 1389 - DNA, 22 bp, Artificial
  synthetic DNA
gagtcgtccatacgatctagga

SEQ ID NO: 1390 - DNA, 22 bp, Artificial
  synthetic DNA
agacggactcaacgccaattcc

SEQ ID NO: 1391 - DNA, 22 bp, Artificial
  synthetic DNA
gtagtgttgagcggaccgagct

SEQ ID NO: 1392 - DNA, 22 bp, Artificial
  synthetic DNA
aatataactagatcatagccag

SEQ ID NO: 1393 - DNA, 22 bp, Artificial
  synthetic DNA
tcaatcggagaatacagaacgt

SEQ ID NO: 1394 - DNA, 22 bp, Artificial
  synthetic DNA
atctccgtcgtccgaaccaaca

SEQ ID NO: 1395 - DNA, 22 bp, Artificial
  synthetic DNA
taggcgttcagcggtatgctta

SEQ ID NO: 1396 - DNA, 22 bp, Artificial
  synthetic DNA
tgcgtgctatacaacctatacg

SEQ ID NO: 1397 - DNA, 22 bp, Artificial
  synthetic DNA
atggccggcatacatctgtatg

SEQ ID NO: 1398 - DNA, 22 bp, Artificial
  synthetic DNA
tgatgctgacataacactgaat

SEQ ID NO: 1399 - DNA, 22 bp, Artificial
  synthetic DNA
atccaaggtacctgaacatcct

SEQ ID NO: 1400 - DNA, 22 bp, Artificial
  synthetic DNA
tagtgacgaccaggtgagcctc

SEQ ID NO: 1401 - DNA, 22 bp, Artificial
  synthetic DNA
aggaggatccgtcaagtcgacc

SEQ ID NO: 1402 - DNA, 22 bp, Artificial
  synthetic DNA
agagtatgccagatcgtgaggc

SEQ ID NO: 1403 - DNA, 22 bp, Artificial
  synthetic DNA
ccactcactaggatggctgcgt

SEQ ID NO: 1404 - DNA, 22 bp, Artificial
  synthetic DNA
tatccaacctgttatagcgatt

SEQ ID NO: 1405 - DNA, 22 bp, Artificial
  synthetic DNA
tcttgcagtgagttgagtctgc

SEQ ID NO: 1406 - DNA, 22 bp, Artificial
  synthetic DNA
ccactgttgtacatacacctgg

SEQ ID NO: 1407 - DNA, 22 bp, Artificial
  synthetic DNA
atgcgcgtaggccactaagtcc

SEQ ID NO: 1408 - DNA, 22 bp, Artificial
  synthetic DNA
acagcggtctacaaccgactgc

SEQ ID NO: 1409 - DNA, 22 bp, Artificial
  synthetic DNA
tcgcgctccagacaattgcagc

SEQ ID NO: 1410 - DNA, 22 bp, Artificial
  synthetic DNA
ccggtagaccaggagtggtcat

SEQ ID NO: 1411 - DNA, 22 bp, Artificial
  synthetic DNA
atctcctaacctagagccatct

SEQ ID NO: 1412 - DNA, 22 bp, Artificial
  synthetic DNA
ccacatcgaatctaacaactac

SEQ ID NO: 1413 - DNA, 22 bp, Artificial
  synthetic DNA
tagtcttattgaatacgtccta

SEQ ID NO: 1414 - DNA, 22 bp, Artificial
  synthetic DNA
tccttaagccttggaactggcg

SEQ ID NO: 1415 - DNA, 22 bp, Artificial
  synthetic DNA
ccgtgatggattgacgtagagg

SEQ ID NO: 1416 - DNA, 22 bp, Artificial
  synthetic DNA
gcctggataacagatgtcttag

SEQ ID NO: 1417 - DNA, 22 bp, Artificial
  synthetic DNA
ctcgacctataatcttctgcca

SEQ ID NO: 1418 - DNA, 22 bp, Artificial
  synthetic DNA
agctacttctccttcctaatca

SEQ ID NO: 1419 - DNA, 22 bp, Artificial
  synthetic DNA
acacgctattgccttccagtta

SEQ ID NO: 1420 - DNA, 22 bp, Artificial
  synthetic DNA
aagcctgtgcatgcaatgagaa

SEQ ID NO: 1421 - DNA, 22 bp, Artificial
  synthetic DNA
tcgttggttatagcacaacttc

SEQ ID NO: 1422 - DNA, 22 bp, Artificial
  synthetic DNA
gcgatgccttccaacataccaa

SEQ ID NO: 1423 - DNA, 22 bp, Artificial
  synthetic DNA
ccaccgttagcacgtgctacgt

SEQ ID NO: 1424 - DNA, 22 bp, Artificial
  synthetic DNA
gttaccacaatgccgccatcaa

SEQ ID NO: 1425 - DNA, 22 bp, Artificial
  synthetic DNA
ggtgcattaagaacgaactacc

SEQ ID NO: 1426 - DNA, 22 bp, Artificial
  synthetic DNA
tccttccggataatgccgattc

SEQ ID NO: 1427 - DNA, 22 bp, Artificial
  synthetic DNA
aaccgcaacttctagcggaaga

SEQ ID NO: 1428 - DNA, 22 bp, Artificial
  synthetic DNA
tccttaagcagttgaacctagg

SEQ ID NO: 1429 - DNA, 22 bp, Artificial
  synthetic DNA
tactaagtcagataagatcaga

SEQ ID NO: 1430 - DNA, 22 bp, Artificial
  synthetic DNA
ttcgccataactagatgaatgc

SEQ ID NO: 1431 - DNA, 22 bp, Artificial
  synthetic DNA
aagaagttagacgcggtggctg

SEQ ID NO: 1432 - DNA, 22 bp, Artificial
  synthetic DNA
gtatctgatcgaagagcggtgg

SEQ ID NO: 1433 - DNA, 22 bp, Artificial
  synthetic DNA
tcaagagctacgaagtaagtcc

SEQ ID NO: 1434 - DNA, 22 bp, Artificial
  synthetic DNA
cgagtacacagcagcataccta

SEQ ID NO: 1435 - DNA, 22 bp, Artificial
  synthetic DNA
ctcgataagttactctgctaga

SEQ ID NO: 1436 - DNA, 22 bp, Artificial
  synthetic DNA
atggtgctggttctccgtctgt

SEQ ID NO: 1437 - DNA, 22 bp, Artificial
  synthetic DNA
tcaagcggtccaaggctgagac

SEQ ID NO: 1438 - DNA, 22 bp, Artificial
  synthetic DNA
tgtcctgctctgttgctaccgt

SEQ ID NO: 1439 - DNA, 22 bp, Artificial
  synthetic DNA
agtcatatcgcgtcacacgttg

SEQ ID NO: 1440 - DNA, 22 bp, Artificial
  synthetic DNA
ggtgaataaggacatgagaagc

SEQ ID NO: 1441 - DNA, 24 bp, Artificial
  synthetic DNA
cctgatcttatctagtagagactc

SEQ ID NO: 1442 - DNA, 24 bp, Artificial
  synthetic DNA
ttctgtgtaggtgtgccaatcacc

SEQ ID NO: 1443 - DNA, 24 bp, Artificial
  synthetic DNA
gacttccagatgcttaagacgaca

SEQ ID NO: 1444 - DNA, 24 bp, Artificial
  synthetic DNA
gtccttcgacggagaacatccgag

SEQ ID NO: 1445 - DNA, 24 bp, Artificial
  synthetic DNA
cttggttagtgtaccgtcaacgtc

SEQ ID NO: 1446 - DNA, 24 bp, Artificial
  synthetic DNA
aagcggcatgtgcctaatcgacgt

SEQ ID NO: 1447 - DNA, 24 bp, Artificial
  synthetic DNA
cgaccgtcgttacacggaatccga

SEQ ID NO: 1448 - DNA, 24 bp, Artificial
  synthetic DNA
tcgcaagtgtgccgttctgttcat

SEQ ID NO: 1449 - DNA, 24 bp, Artificial
  synthetic DNA
cgtactgaagttcggagtcgccgt

SEQ ID NO: 1450 - DNA, 24 bp, Artificial
  synthetic DNA
ccactacagaatggtagcagatca

SEQ ID NO: 1451 - DNA, 24 bp, Artificial
  synthetic DNA
agtaggagagaggcctacacaaca

SEQ ID NO: 1452 - DNA, 24 bp, Artificial
  synthetic DNA
agccaagatactcgttcggtatgg

SEQ ID NO: 1453 - DNA, 24 bp, Artificial
  synthetic DNA
gttccgagtacattgaatcctggc

SEQ ID NO: 1454 - DNA, 24 bp, Artificial
  synthetic DNA
aggcgtacgagttattgccagagg

SEQ ID NO: 1455 - DNA, 24 bp, Artificial
  synthetic DNA
gtggcatcacacatatctcagcat

SEQ ID NO: 1456 - DNA, 24 bp, Artificial
  synthetic DNA
gagaccgatatgttgatgccagaa

SEQ ID NO: 1457 - DNA, 24 bp, Artificial
  synthetic DNA
caactgtagccagtcgattgctat

SEQ ID NO: 1458 - DNA, 24 bp, Artificial
  synthetic DNA
tatcaatgcaatgagaggatgcag

SEQ ID NO: 1459 - DNA, 24 bp, Artificial
  synthetic DNA
gtatgctcggctccaagtactgtt

SEQ ID NO: 1460 - DNA, 24 bp, Artificial
  synthetic DNA
agagactcttataggcttgacgga

SEQ ID NO: 1461 - DNA, 24 bp, Artificial
  synthetic DNA
acttaacagatatggatcatcgcc

SEQ ID NO: 1462 - DNA, 24 bp, Artificial
  synthetic DNA
aatcagagcgagtctcgcttcagg

SEQ ID NO: 1463 - DNA, 24 bp, Artificial
  synthetic DNA
accaccgaggaacaggtgcgacaa

SEQ ID NO: 1464 - DNA, 24 bp, Artificial
  synthetic DNA
tggtacatgtcaaccgtaagcctg

SEQ ID NO: 1465 - DNA, 24 bp, Artificial
  synthetic DNA
cgtgccgcggtgttcttgtatatg

SEQ ID NO: 1466 - DNA, 24 bp, Artificial
  synthetic DNA
gacaagcgcgcgtgagacatatca

SEQ ID NO: 1467 - DNA, 24 bp, Artificial
  synthetic DNA
agtgcactccgaacaagagttagt

SEQ ID NO: 1468 - DNA, 24 bp, Artificial
  synthetic DNA
cctcattaccgcgttaggagtccg

SEQ ID NO: 1469 - DNA, 24 bp, Artificial
  synthetic DNA
tgcttattgcttagttgctatctc

SEQ ID NO: 1470 - DNA, 24 bp, Artificial
  synthetic DNA
gcgtgatcctgttctattcgttag

SEQ ID NO: 1471 - DNA, 24 bp, Artificial
  synthetic DNA
ggccagaactatgacgagtataag

SEQ ID NO: 1472 - DNA, 24 bp, Artificial
  synthetic DNA
gatggcgactatctaattgcaatg

SEQ ID NO: 1473 - DNA, 24 bp, Artificial
  synthetic DNA
tagtaaccatagctctgtacaact

SEQ ID NO: 1474 - DNA, 24 bp, Artificial
  synthetic DNA
cgtgatcgccaatacacatgtcgc

SEQ ID NO: 1475 - DNA, 24 bp, Artificial
  synthetic DNA
taataacggatcgatatgcacgcg

SEQ ID NO: 1476 - DNA, 24 bp, Artificial
  synthetic DNA
atcatcgcgctaatactatctgaa

SEQ ID NO: 1477 - DNA, 24 bp, Artificial
  synthetic DNA
cacgtgcgtgcaggtcactagtat

SEQ ID NO: 1478 - DNA, 24 bp, Artificial
  synthetic DNA
aggtccaatgccgagcgatcagaa

SEQ ID NO: 1479 - DNA, 24 bp, Artificial
  synthetic DNA
cagcataacaacgagccaggtcag

SEQ ID NO: 1480 - DNA, 24 bp, Artificial
  synthetic DNA
atggcgtccaatactccgacctat

SEQ ID NO: 1481 - DNA, 24 bp, Artificial
  synthetic DNA
aggaacatcgtgaataatgaagac

SEQ ID NO: 1482 - DNA, 24 bp, Artificial
  synthetic DNA
tctcgacgttcatgtaattaagga

SEQ ID NO: 1483 - DNA, 24 bp, Artificial
  synthetic DNA
tcgcggttaaccttacttagacga

SEQ ID NO: 1484 - DNA, 24 bp, Artificial
  synthetic DNA
atcatatctacggctctggcgccg

SEQ ID NO: 1485 - DNA, 24 bp, Artificial
  synthetic DNA
gcagatggagaccagaggtacagg

SEQ ID NO: 1486 - DNA, 24 bp, Artificial
  synthetic DNA
agacagaagattaccacgtgctat

SEQ ID NO: 1487 - DNA, 24 bp, Artificial
  synthetic DNA
ccacggacaacatgccgcttaact

SEQ ID NO: 1488 - DNA, 24 bp, Artificial
  synthetic DNA
cttgaagtctcaagctatgagaga

SEQ ID NO: 1489 - DNA, 24 bp, Artificial
  synthetic DNA
acagcagtcgtgcttaggtcactg

SEQ ID NO: 1490 - DNA, 24 bp, Artificial
  synthetic DNA
aggtgttaatgaacgtaggtgaga

SEQ ID NO: 1491 - DNA, 24 bp, Artificial
  synthetic DNA
agccactatgttcaaggctgagcc

SEQ ID NO: 1492 - DNA, 24 bp, Artificial
  synthetic DNA
gcaggcggtgtcgtgtgacaatga

SEQ ID NO: 1493 - DNA, 24 bp, Artificial
  synthetic DNA
agccattgctacagaggttactta

SEQ ID NO: 1494 - DNA, 24 bp, Artificial
  synthetic DNA
acaatcgaacctacactgagtccg

SEQ ID NO: 1495 - DNA, 24 bp, Artificial
  synthetic DNA
ccgatctcaataggtaccacgaac

SEQ ID NO: 1496 - DNA, 24 bp, Artificial
  synthetic DNA
gatacgtggcgctatgctaattaa

SEQ ID NO: 1497 - DNA, 24 bp, Artificial
  synthetic DNA
agagagatggcacacattgacgtc

SEQ ID NO: 1498 - DNA, 24 bp, Artificial
  synthetic DNA
ctcaactcatccttgtagccgatg

SEQ ID NO: 1499 - DNA, 24 bp, Artificial
  synthetic DNA
gtggaataacgcgatacgactctt

SEQ ID NO: 1500 - DNA, 24 bp, Artificial
  synthetic DNA
atctaccatgcgaatgctctctag

SEQ ID NO: 1501 - DNA, 24 bp, Artificial
  synthetic DNA
atacgcacgcctgacacaaggacc

SEQ ID NO: 1502 - DNA, 24 bp, Artificial
  synthetic DNA
gtccactctcagtgtgtagagtcc

SEQ ID NO: 1503 - DNA, 24 bp, Artificial
  synthetic DNA
aatatatccagattctctgtgcag

SEQ ID NO: 1504 - DNA, 24 bp, Artificial
  synthetic DNA
ccttccgccacatgttcgacaagg

SEQ ID NO: 1505 - DNA, 24 bp, Artificial
  synthetic DNA
actgtgccatcatccgaggagcca

SEQ ID NO: 1506 - DNA, 24 bp, Artificial
  synthetic DNA
tctatgccgctatggcgtcgtgta

SEQ ID NO: 1507 - DNA, 24 bp, Artificial
  synthetic DNA
cgtaacctaaggtaatatgtctgc

SEQ ID NO: 1508 - DNA, 24 bp, Artificial
  synthetic DNA
tactgaccgtatcaagattactaa

SEQ ID NO: 1509 - DNA, 24 bp, Artificial
  synthetic DNA
tcatcggagcgccatacggtacgt

SEQ ID NO: 1510 - DNA, 24 bp, Artificial
  synthetic DNA
gcaagaggaatgaacgaagtgatt

SEQ ID NO: 1511 - DNA, 24 bp, Artificial
  synthetic DNA
ggctgattgacatcctgacttagt

SEQ ID NO: 1512 - DNA, 24 bp, Artificial
  synthetic DNA
aaggcgctagattggattaacgta

SEQ ID NO: 1513 - DNA, 24 bp, Artificial
  synthetic DNA
gctagctagaagaataggattcgt

SEQ ID NO: 1514 - DNA, 24 bp, Artificial
  synthetic DNA
caggtgacggcctctataactcat

SEQ ID NO: 1515 - DNA, 24 bp, Artificial
  synthetic DNA
caggttacacataccactatcttc

SEQ ID NO: 1516 - DNA, 24 bp, Artificial
  synthetic DNA
ttgctacgtaccgtcttaatccgt

SEQ ID NO: 1517 - DNA, 24 bp, Artificial
  synthetic DNA
ctcaacatgtcttgcaagcttcga

SEQ ID NO: 1518 - DNA, 24 bp, Artificial
  synthetic DNA
ggtgcggtacgtagaaccagatca

SEQ ID NO: 1519 - DNA, 24 bp, Artificial
  synthetic DNA
aatgctctccaagatcctgaccta

SEQ ID NO: 1520 - DNA, 24 bp, Artificial
  synthetic DNA
gcttcgcaggtctggatgatggag

SEQ ID NO: 1521 - DNA, 24 bp, Artificial
  synthetic DNA
acattgaccagacagcaccttgcg

SEQ ID NO: 1522 - DNA, 24 bp, Artificial
  synthetic DNA
aggtatcaatgtgcttaataggcg

SEQ ID NO: 1523 - DNA, 24 bp, Artificial
  synthetic DNA
tccggacacacgattagtaacgga

SEQ ID NO: 1524 - DNA, 24 bp, Artificial
  synthetic DNA
tacgaagtactacagatcggtcag

SEQ ID NO: 1525 - DNA, 24 bp, Artificial
  synthetic DNA
aattgtcagacgaatactgctgga

SEQ ID NO: 1526 - DNA, 24 bp, Artificial
  synthetic DNA
tgaatcatgagccagaggttatgc

SEQ ID NO: 1527 - DNA, 24 bp, Artificial
  synthetic DNA
cacaagacacgtcattaacatcaa

SEQ ID NO: 1528 - DNA, 24 bp, Artificial
  synthetic DNA
gaatgactacattactccgccagg

SEQ ID NO: 1529 - DNA, 24 bp, Artificial
  synthetic DNA
agccagagatactggaacttgact

SEQ ID NO: 1530 - DNA, 24 bp, Artificial
  synthetic DNA
tatcagacacatcacaatggatac

SEQ ID NO: 1531 - DNA, 24 bp, Artificial
  synthetic DNA
ctaggacaccgctagtcggttgaa

SEQ ID NO: 1532 - DNA, 24 bp, Artificial
  synthetic DNA
gtataactgcgtgtcctggtgtat

SEQ ID NO: 1533 - DNA, 24 bp, Artificial
  synthetic DNA
atgcaatactaaggtggacctccg

SEQ ID NO: 1534 - DNA, 24 bp, Artificial
  synthetic DNA
atgcagacgcttgcgataagtcat

SEQ ID NO: 1535 - DNA, 24 bp, Artificial
  synthetic DNA
ttgctcgatacacgtagaccagtg

SEQ ID NO: 1536 - DNA, 24 bp, Artificial
  synthetic DNA
tactggaggacgattgtctatcat

SEQ ID NO: 1537 - DNA, 26 bp, Artificial
  synthetic DNA
actaaggcacgctgattcgagcatta

SEQ ID NO: 1538 - DNA, 26 bp, Artificial
  synthetic DNA
cggattctggcacgtacaagtagcag

SEQ ID NO: 1539 - DNA, 26 bp, Artificial
  synthetic DNA
ttatggctccagatctagtcaccagc

SEQ ID NO: 1540 - DNA, 26 bp, Artificial
  synthetic DNA
catacactccaggcatgtatgatagg

SEQ ID NO: 1541 - DNA, 26 bp, Artificial
  synthetic DNA
agttgtaagccaacgagtgtagcgta

SEQ ID NO: 1542 - DNA, 26 bp, Artificial
  synthetic DNA
gtatcagctccttcctctgattccgg

SEQ ID NO: 1543 - DNA, 26 bp, Artificial
  synthetic DNA
aacatacagaatgtctatggtcagct

SEQ ID NO: 1544 - DNA, 26 bp, Artificial
  synthetic DNA
gactcatattcatgttcagtatagag

SEQ ID NO: 1545 - DNA, 26 bp, Artificial
  synthetic DNA
agagtgaacgaacgtgaccgacgctc

SEQ ID NO: 1546 - DNA, 26 bp, Artificial
  synthetic DNA
aattggcgtccttgccacaacatctt

SEQ ID NO: 1547 - DNA, 26 bp, Artificial
  synthetic DNA
tcgtagacgcctcgtacatccgagat

SEQ ID NO: 1548 - DNA, 26 bp, Artificial
  synthetic DNA
ccggctcgtgaggcgataatcatata

SEQ ID NO: 1549 - DNA, 26 bp, Artificial
  synthetic DNA
agtcctgatcacgaccacgactcacg

SEQ ID NO: 1550 - DNA, 26 bp, Artificial
  synthetic DNA
ggcactcaatcctccatggagaagct

SEQ ID NO: 1551 - DNA, 26 bp, Artificial
  synthetic DNA
tcatcattcctcacgttcaccggtga

SEQ ID NO: 1552 - DNA, 26 bp, Artificial
  synthetic DNA
tcaactctgtgctaaccggtcgtaca

SEQ ID NO: 1553 - DNA, 26 bp, Artificial
  synthetic DNA
tgttcttatgcattaatgccaggctt

SEQ ID NO: 1554 - DNA, 26 bp, Artificial
  synthetic DNA
gattcacgacctcaacagcatcactc

SEQ ID NO: 1555 - DNA, 26 bp, Artificial
  synthetic DNA
ggcgagttcgaccagaatgctggaca

SEQ ID NO: 1556 - DNA, 26 bp, Artificial
  synthetic DNA
ttccgtatacaatgcgattaagatct

SEQ ID NO: 1557 - DNA, 26 bp, Artificial
  synthetic DNA
gagtaatccgtaaccggccaacgttg

SEQ ID NO: 1558 - DNA, 26 bp, Artificial
  synthetic DNA
cgcttccatcatggtacggtacgtat

SEQ ID NO: 1559 - DNA, 26 bp, Artificial
  synthetic DNA
ccgtcgtggtgtgttgactggtcaac

SEQ ID NO: 1560 - DNA, 26 bp, Artificial
  synthetic DNA
tattcgcatctccgtattagttgtag

SEQ ID NO: 1561 - DNA, 26 bp, Artificial
  synthetic DNA
tattattgtattctaggcggtgcaac

SEQ ID NO: 1562 - DNA, 26 bp, Artificial
  synthetic DNA
aggctgcctacttcctcgtcatctcg

SEQ ID NO: 1563 - DNA, 26 bp, Artificial
  synthetic DNA
gtaacatacggctcatcgaatgcatc

SEQ ID NO: 1564 - DNA, 26 bp, Artificial
  synthetic DNA
ttatggcacggatattaccgtacgcc

SEQ ID NO: 1565 - DNA, 26 bp, Artificial
  synthetic DNA
atagcacttcctctaatgctctgctg

SEQ ID NO: 1566 - DNA, 26 bp, Artificial
  synthetic DNA
tcacaggcaatagcctaatattatat

SEQ ID NO: 1567 - DNA, 26 bp, Artificial
  synthetic DNA
ggcggatgttcgttaatattataagg

SEQ ID NO: 1568 - DNA, 26 bp, Artificial
  synthetic DNA
tgcaatagccgttgtctctgccagcg

SEQ ID NO: 1569 - DNA, 26 bp, Artificial
  synthetic DNA
tacagcgcgttggcgagtactgatag

SEQ ID NO: 1570 - DNA, 26 bp, Artificial
  synthetic DNA
tgcagttagtaccttctcacgccaac

SEQ ID NO: 1571 - DNA, 26 bp, Artificial
  synthetic DNA
ccattggctacctagcagactctacc

SEQ ID NO: 1572 - DNA, 26 bp, Artificial
  synthetic DNA
aacagtagctcgcgtcttgctctcgt

SEQ ID NO: 1573 - DNA, 26 bp, Artificial
  synthetic DNA
gcagtccatcagctctcgcttataga

SEQ ID NO: 1574 - DNA, 26 bp, Artificial
  synthetic DNA
tatctctctgtcgccagcttgaccaa

SEQ ID NO: 1575 - DNA, 26 bp, Artificial
  synthetic DNA
cagactgttcaagcttgctgtaggag

SEQ ID NO: 1576 - DNA, 26 bp, Artificial
  synthetic DNA
taaccggaactcgttcagcaacattc

SEQ ID NO: 1577 - DNA, 26 bp, Artificial
  synthetic DNA
tcaattatgcatgtcgtccgatctct

SEQ ID NO: 1578 - DNA, 26 bp, Artificial
  synthetic DNA
ttgtctaagtcaacctgtggataatc

SEQ ID NO: 1579 - DNA, 26 bp, Artificial
  synthetic DNA
tctaagagtggtatgaccaggagtcc

SEQ ID NO: 1580 - DNA, 26 bp, Artificial
  synthetic DNA
tcgtagtactactggaacaggtaatc

SEQ ID NO: 1581 - DNA, 26 bp, Artificial
  synthetic DNA
atgtcaacattctaatcatctctcgg

SEQ ID NO: 1582 - DNA, 26 bp, Artificial
  synthetic DNA
agcgcgcaactgttacggtgatccga

SEQ ID NO: 1583 - DNA, 26 bp, Artificial
  synthetic DNA
gcgatagaataatggtgtcacacacg

SEQ ID NO: 1584 - DNA, 26 bp, Artificial
  synthetic DNA
aaggctgcgatgagaggcgtacatcg

SEQ ID NO: 1585 - DNA, 26 bp, Artificial
  synthetic DNA
ggttcatggtctcagtcgtgatcgcg

SEQ ID NO: 1586 - DNA, 26 bp, Artificial
  synthetic DNA
tagtgactctatgtcacctcggagcc

SEQ ID NO: 1587 - DNA, 26 bp, Artificial
  synthetic DNA
atgtgatagcaatggcacctctagtc

SEQ ID NO: 1588 - DNA, 26 bp, Artificial
  synthetic DNA
tcgcgaagtgtaatgcatcatccgct

SEQ ID NO: 1589 - DNA, 26 bp, Artificial
  synthetic DNA
atgtggcgacgatccaagttcaacgc

SEQ ID NO: 1590 - DNA, 26 bp, Artificial
  synthetic DNA
accttgtatgagtcggagtgtccggc

SEQ ID NO: 1591 - DNA, 26 bp, Artificial
  synthetic DNA
acctcaagagagtagacagttgagtt

SEQ ID NO: 1592 - DNA, 26 bp, Artificial
  synthetic DNA
ggtgtaatcctgtgtgcgaagctggt

SEQ ID NO: 1593 - DNA, 26 bp, Artificial
  synthetic DNA
atagcggaactgtacgacgctccagt

SEQ ID NO: 1594 - DNA, 26 bp, Artificial
  synthetic DNA
aagcacgagtcgaccattagcctgga

SEQ ID NO: 1595 - DNA, 26 bp, Artificial
  synthetic DNA
attccggtaacatcagaaggtacaat

SEQ ID NO: 1596 - DNA, 26 bp, Artificial
  synthetic DNA
gtgcaacggcagtccagtatcctggt

SEQ ID NO: 1597 - DNA, 26 bp, Artificial
  synthetic DNA
ccatcttatacacggtgaccgaagat

SEQ ID NO: 1598 - DNA, 26 bp, Artificial
  synthetic DNA
gcacttaatcaagcttgagtgatgct

SEQ ID NO: 1599 - DNA, 26 bp, Artificial
  synthetic DNA
agtattacgtgagtacgaagatagca

SEQ ID NO: 1600 - DNA, 26 bp, Artificial
  synthetic DNA
ttcttaggttaagttccttctggacc

SEQ ID NO: 1601 - DNA, 26 bp, Artificial
  synthetic DNA
gtccttgctagacactgaccgttgct

SEQ ID NO: 1602 - DNA, 26 bp, Artificial
  synthetic DNA
gccgctatgtgtgctgcatcctaagc

SEQ ID NO: 1603 - DNA, 26 bp, Artificial
  synthetic DNA
ccatcaataacagacttatgttgtga

SEQ ID NO: 1604 - DNA, 26 bp, Artificial
  synthetic DNA
cgcgtgtgcttacaagtgctaacaag

SEQ ID NO: 1605 - DNA, 26 bp, Artificial
  synthetic DNA
cgatatgtgttcgcaataagagagcc

SEQ ID NO: 1606 - DNA, 26 bp, Artificial
  synthetic DNA
cgcggatgtgagcggctcaattagca

SEQ ID NO: 1607 - DNA, 26 bp, Artificial
  synthetic DNA
gctgcatgactatcggatggaggcat

SEQ ID NO: 1608 - DNA, 26 bp, Artificial
  synthetic DNA
ctatgccgtgtatggtacgagtggcg

SEQ ID NO: 1609 - DNA, 26 bp, Artificial
  synthetic DNA
ccggctggagttcattacgtaggctg

SEQ ID NO: 1610 - DNA, 26 bp, Artificial
  synthetic DNA
tgtaggcctactgagctagtattaga

SEQ ID NO: 1611 - DNA, 26 bp, Artificial
  synthetic DNA
ccgtcaagtgactattcttctaatct

SEQ ID NO: 1612 - DNA, 26 bp, Artificial
  synthetic DNA
ggtcttacgccagagactgcgcttct

SEQ ID NO: 1613 - DNA, 26 bp, Artificial
  synthetic DNA
cgaagtgtgattattaactgtaatct

SEQ ID NO: 1614 - DNA, 26 bp, Artificial
  synthetic DNA
gcacgcgtggccgtaagcatcgatta

SEQ ID NO: 1615 - DNA, 26 bp, Artificial
  synthetic DNA
atcctgcgtcggaacgtactatagct

SEQ ID NO: 1616 - DNA, 26 bp, Artificial
  synthetic DNA
agtatcatcatatccattcgcagtac

SEQ ID NO: 1617 - DNA, 26 bp, Artificial
  synthetic DNA
agtcctgacgttcatatatagactcc

SEQ ID NO: 1618 - DNA, 26 bp, Artificial
  synthetic DNA
cttgcagtaatctgaatctgaaggtt

SEQ ID NO: 1619 - DNA, 26 bp, Artificial
  synthetic DNA
ataacttggttccagtaacgcatagt

SEQ ID NO: 1620 - DNA, 26 bp, Artificial
  synthetic DNA
gataaggatatggctgtagcgaagtg

SEQ ID NO: 1621 - DNA, 26 bp, Artificial
  synthetic DNA
gtggagcgttacagacatgctgaaca

SEQ ID NO: 1622 - DNA, 26 bp, Artificial
  synthetic DNA
cgcttccggcaggcgtcatataagtc

SEQ ID NO: 1623 - DNA, 26 bp, Artificial
  synthetic DNA
ataacattctaacctctataagccga

SEQ ID NO: 1624 - DNA, 26 bp, Artificial
  synthetic DNA
acgatctatgatccatatggacttcc

SEQ ID NO: 1625 - DNA, 26 bp, Artificial
  synthetic DNA
tgaagctcagatatcatgcctcgagc

SEQ ID NO: 1626 - DNA, 26 bp, Artificial
  synthetic DNA
agacttcaccgcaataactcgtagat

SEQ ID NO: 1627 - DNA, 26 bp, Artificial
  synthetic DNA
agactaagacatacgccatcaccgct

SEQ ID NO: 1628 - DNA, 26 bp, Artificial
  synthetic DNA
tgtagcgtgatgtatcgtaattctgt

SEQ ID NO: 1629 - DNA, 26 bp, Artificial
  synthetic DNA
tgtgctattggcacctcacgctgacc

SEQ ID NO: 1630 - DNA, 26 bp, Artificial
  synthetic DNA
tgtagataagtatccagcgactctct

SEQ ID NO: 1631 - DNA, 26 bp, Artificial
  synthetic DNA
aattcgccaattgtgtgtaggcgcaa

SEQ ID NO: 1632 - DNA, 26 bp, Artificial
  synthetic DNA
cgattatgagtacttgtagaccagct

SEQ ID NO: 1633 - DNA, 28 bp, Artificial
  synthetic DNA
ttgcaagaacaacgtatctcatatgaac

SEQ ID NO: 1634 - DNA, 28 bp, Artificial
  synthetic DNA
caccgtgctgttattacttggtattcgg

SEQ ID NO: 1635 - DNA, 28 bp, Artificial
  synthetic DNA
cacgtgtattgttgcaccagaacgacaa

SEQ ID NO: 1636 - DNA, 28 bp, Artificial
  synthetic DNA
atgcacgtaattacttccggagaagacg

SEQ ID NO: 1637 - DNA, 28 bp, Artificial
  synthetic DNA
tatgttgtctgatatggttcatgtggca

SEQ ID NO: 1638 - DNA, 28 bp, Artificial
  synthetic DNA
agcgcgactagttgatgccaacattgta

SEQ ID NO: 1639 - DNA, 28 bp, Artificial
  synthetic DNA
ataggcaggtccaggctcggaacaagtc

SEQ ID NO: 1640 - DNA, 28 bp, Artificial
  synthetic DNA
gcggtagtcggtcaagaactagaaccgt

SEQ ID NO: 1641 - DNA, 28 bp, Artificial
  synthetic DNA
actatacactctagctattaggaagcat

SEQ ID NO: 1642 - DNA, 28 bp, Artificial
  synthetic DNA
gatcatcttgcttctcctgtggagataa

SEQ ID NO: 1643 - DNA, 28 bp, Artificial
  synthetic DNA
ctactacgagtccataactgatagcctc

SEQ ID NO: 1644 - DNA, 28 bp, Artificial
  synthetic DNA
gcacagacacctgtcctatctagcagga

SEQ ID NO: 1645 - DNA, 28 bp, Artificial
  synthetic DNA
aagcgaggcgcgaaggagatggaaggat

SEQ ID NO: 1646 - DNA, 28 bp, Artificial
  synthetic DNA
ctgaagacgccagtctggataggtgcct

SEQ ID NO: 1647 - DNA, 28 bp, Artificial
  synthetic DNA
gtaagctctgtccttcgagattgataag

SEQ ID NO: 1648 - DNA, 28 bp, Artificial
  synthetic DNA
ggttagagagattattgtgcgcatccat

SEQ ID NO: 1649 - DNA, 28 bp, Artificial
  synthetic DNA
ccaggaggacctatgatcttgccgccat

SEQ ID NO: 1650 - DNA, 28 bp, Artificial
  synthetic DNA
actattcgagctactgtatgtgtatccg

SEQ ID NO: 1651 - DNA, 28 bp, Artificial
  synthetic DNA
gacatcgcgatacgtaactccggagtgt

SEQ ID NO: 1652 - DNA, 28 bp, Artificial
  synthetic DNA
ccgcaattcgtctatatattctagcata

SEQ ID NO: 1653 - DNA, 28 bp, Artificial
  synthetic DNA
ctacacttgaggttgatgctcaagatca

SEQ ID NO: 1654 - DNA, 28 bp, Artificial
  synthetic DNA
cgatcagttctagttcaccgcggacaat

SEQ ID NO: 1655 - DNA, 28 bp, Artificial
  synthetic DNA
aagaatgatgattggccgcgaaccaagc

SEQ ID NO: 1656 - DNA, 28 bp, Artificial
  synthetic DNA
cacgaccggaactagactcctaccaatt

SEQ ID NO: 1657 - DNA, 28 bp, Artificial
  synthetic DNA
agttgcctgtgagtgaggctactatctc

SEQ ID NO: 1658 - DNA, 28 bp, Artificial
  synthetic DNA
gattcttccgatgatcatgccactacaa

SEQ ID NO: 1659 - DNA, 28 bp, Artificial
  synthetic DNA
cgctgaagtgaactatgcaagcaccgca

SEQ ID NO: 1660 - DNA, 28 bp, Artificial
  synthetic DNA
attatcgtgatggtgagactgagctcgt

SEQ ID NO: 1661 - DNA, 28 bp, Artificial
  synthetic DNA
cgaggccactctgagccaggtaagtatc

SEQ ID NO: 1662 - DNA, 28 bp, Artificial
  synthetic DNA
tgccgaggacagccgatcacatcttcgt

SEQ ID NO: 1663 - DNA, 28 bp, Artificial
  synthetic DNA
gttgacatgaaggttatcgtcgatattc

SEQ ID NO: 1664 - DNA, 28 bp, Artificial
  synthetic DNA
gtggtccaggtcaagctctgatcgaatg

SEQ ID NO: 1665 - DNA, 28 bp, Artificial
  synthetic DNA
ccagtccggtgtactcagacctaataac

SEQ ID NO: 1666 - DNA, 28 bp, Artificial
  synthetic DNA
cgagacactgcatgagcgtagtcttatt

SEQ ID NO: 1667 - DNA, 28 bp, Artificial
  synthetic DNA
gacggcttgtatacttctctacggtctg

SEQ ID NO: 1668 - DNA, 28 bp, Artificial
  synthetic DNA
ttagctggatggaagccatattccgtag

SEQ ID NO: 1669 - DNA, 28 bp, Artificial
  synthetic DNA
cagcctacacttgattactcaacaactc

SEQ ID NO: 1670 - DNA, 28 bp, Artificial
  synthetic DNA
gtacgtagtgtcacgcgcctacgttcgt

SEQ ID NO: 1671 - DNA, 28 bp, Artificial
  synthetic DNA
ctacaacttctcaatcatgcctctgttg

SEQ ID NO: 1672 - DNA, 28 bp, Artificial
  synthetic DNA
cgaggacagaattcgacataaggagaga

SEQ ID NO: 1673 - DNA, 28 bp, Artificial
  synthetic DNA
gccgaacgacacagtgagttgataggta

SEQ ID NO: 1674 - DNA, 28 bp, Artificial
  synthetic DNA
gaacactatatgctgtcgctgtctgagg

SEQ ID NO: 1675 - DNA, 28 bp, Artificial
  synthetic DNA
gttaagttcttcggcggtcatgctcatt

SEQ ID NO: 1676 - DNA, 28 bp, Artificial
  synthetic DNA
ttgcttacagatcgcgtatccatagtat

SEQ ID NO: 1677 - DNA, 28 bp, Artificial
  synthetic DNA
gaggaccacctctgcgaagttcactgtg

SEQ ID NO: 1678 - DNA, 28 bp, Artificial
  synthetic DNA
aatcctagcatatcgagaacgacactga

SEQ ID NO: 1679 - DNA, 28 bp, Artificial
  synthetic DNA
tgaatactatagccatagtcgacttccg

SEQ ID NO: 1680 - DNA, 28 bp, Artificial
  synthetic DNA
gacatccacgaagctggtaatcggaacc

SEQ ID NO: 1681 - DNA, 28 bp, Artificial
  synthetic DNA
ttagccgtcttagaagtgtctgaccggc

SEQ ID NO: 1682 - DNA, 28 bp, Artificial
  synthetic DNA
ctattctgccgtaattgattccttcgtt

SEQ ID NO: 1683 - DNA, 28 bp, Artificial
  synthetic DNA
acgcctctggtcgaaggtagattagctc

SEQ ID NO: 1684 - DNA, 28 bp, Artificial
  synthetic DNA
cagcctattgatcgtaagtagatggtcc

SEQ ID NO: 1685 - DNA, 28 bp, Artificial
  synthetic DNA
ttaagtgaggtggacaaccatcaacttc

SEQ ID NO: 1686 - DNA, 28 bp, Artificial
  synthetic DNA
aaggccttgcggctaagtagtattcatc

SEQ ID NO: 1687 - DNA, 28 bp, Artificial
  synthetic DNA
ttgtgatactaattcttctcaagagtca

SEQ ID NO: 1688 - DNA, 28 bp, Artificial
  synthetic DNA
gcattaggtgacgaccttagtccatcac

SEQ ID NO: 1689 - DNA, 28 bp, Artificial
  synthetic DNA
gcggatggacgtatacagtgagtcgtgc

SEQ ID NO: 1690 - DNA, 28 bp, Artificial
  synthetic DNA
gaacatgccagcctcaactaggctaaga

SEQ ID NO: 1691 - DNA, 28 bp, Artificial
  synthetic DNA
tccgtcattagagtatgagtgactacta

SEQ ID NO: 1692 - DNA, 28 bp, Artificial
  synthetic DNA
aacacttagtaaccagttcggactggac

SEQ ID NO: 1693 - DNA, 28 bp, Artificial
  synthetic DNA
cgctaactattgcgtatattcgcggctt

SEQ ID NO: 1694 - DNA, 28 bp, Artificial
  synthetic DNA
gccatctacgatcttcggcttatcctag

SEQ ID NO: 1695 - DNA, 28 bp, Artificial
  synthetic DNA
cctgagaatgttgactaagatcttgtga

SEQ ID NO: 1696 - DNA, 28 bp, Artificial
  synthetic DNA
tcggttagtctaatcatcacgcaacgga

SEQ ID NO: 1697 - DNA, 28 bp, Artificial
  synthetic DNA
attatctattgaagcagtgacagcgatc

SEQ ID NO: 1698 - DNA, 28 bp, Artificial
  synthetic DNA
gaggagaatcacggaacacggtcacatg

SEQ ID NO: 1699 - DNA, 28 bp, Artificial
  synthetic DNA
gctgcaagcattatgaccatggcatctg

SEQ ID NO: 1700 - DNA, 28 bp, Artificial
  synthetic DNA
gaacaacctataacgacgttgtggacaa

SEQ ID NO: 1701 - DNA, 28 bp, Artificial
  synthetic DNA
ttaatcatcgatagacgacatggaatca

SEQ ID NO: 1702 - DNA, 28 bp, Artificial
  synthetic DNA
tcgagtgtaagcacactacgatctggaa

SEQ ID NO: 1703 - DNA, 28 bp, Artificial
  synthetic DNA
gctacgcacagtctctgcacagctacac

SEQ ID NO: 1704 - DNA, 28 bp, Artificial
  synthetic DNA
cctgtatgtacgttctggctaatacctt

SEQ ID NO: 1705 - DNA, 28 bp, Artificial
  synthetic DNA
tgaagcaccggtacatggtgtatccgga

SEQ ID NO: 1706 - DNA, 28 bp, Artificial
  synthetic DNA
tgctggaacctaactcggtgatgacgat

SEQ ID NO: 1707 - DNA, 28 bp, Artificial
  synthetic DNA
cgctatcttactgccaagttctcatata

SEQ ID NO: 1708 - DNA, 28 bp, Artificial
  synthetic DNA
aacgcgcgcgtatcggcaataatctcaa

SEQ ID NO: 1709 - DNA, 28 bp, Artificial
  synthetic DNA
ccattaggatgaccatcgactattagag

SEQ ID NO: 1710 - DNA, 28 bp, Artificial
  synthetic DNA
tactgctagactgcgtgcattcatggcg

SEQ ID NO: 1711 - DNA, 28 bp, Artificial
  synthetic DNA
cattgcgcgctccacgaactctattgtc

SEQ ID NO: 1712 - DNA, 28 bp, Artificial
  synthetic DNA
gacgcgcctagaactgtatagctctacg

SEQ ID NO: 1713 - DNA, 28 bp, Artificial
  synthetic DNA
cattgcaacttgtcggtgatggcaatcc

SEQ ID NO: 1714 - DNA, 28 bp, Artificial
  synthetic DNA
ttaatgcacatgcagtacggcaccacag

SEQ ID NO: 1715 - DNA, 28 bp, Artificial
  synthetic DNA
agcggtacgtggacgagtggtaattaat

SEQ ID NO: 1716 - DNA, 28 bp, Artificial
  synthetic DNA
gacgtattgctatgcattggaagatgct

SEQ ID NO: 1717 - DNA, 28 bp, Artificial
  synthetic DNA
aacacttcgaccattgcgcctcaatggt

SEQ ID NO: 1718 - DNA, 28 bp, Artificial
  synthetic DNA
cggtacgctctagcggtcataagatgca

SEQ ID NO: 1719 - DNA, 28 bp, Artificial
  synthetic DNA
cctgaataacagccgcgcctaattagat

SEQ ID NO: 1720 - DNA, 28 bp, Artificial
  synthetic DNA
aagcgtctaatgtgccttaagtcacatg

SEQ ID NO: 1721 - DNA, 28 bp, Artificial
  synthetic DNA
gctctccaagaaccagaagtaagcatcg

SEQ ID NO: 1722 - DNA, 28 bp, Artificial
  synthetic DNA
gaggagagttgtccgagtggtgtgatgt

SEQ ID NO: 1723 - DNA, 28 bp, Artificial
  synthetic DNA
taacgagtggtgcgtctaagcaattgag

SEQ ID NO: 1724 - DNA, 28 bp, Artificial
  synthetic DNA
ccaacagtatgctgacataactatgata

SEQ ID NO: 1725 - DNA, 28 bp, Artificial
  synthetic DNA
gatccttgccacgcctatgagatatcgc

SEQ ID NO: 1726 - DNA, 28 bp, Artificial
  synthetic DNA
aacgcgctaccgtccttgtgcatagagg

SEQ ID NO: 1727 - DNA, 28 bp, Artificial
  synthetic DNA
ctacatgtgccttatagtacagaggaac

SEQ ID NO: 1728 - DNA, 28 bp, Artificial
  synthetic DNA
cagcctcgtagttagcgtgattcatgcg

SEQ ID NO: 1729 - DNA, 29 bp, Artificial
  synthetic DNA
ctcctcgccgattgaagtgcgtagaacta

SEQ ID NO: 1730 - DNA, 29 bp, Artificial
  synthetic DNA
cagcaggcctcaataggataagccaacta

SEQ ID NO: 1731 - DNA, 29 bp, Artificial
  synthetic DNA
gaccatcaatctcgaagactacgctctgt

SEQ ID NO: 1732 - DNA, 29 bp, Artificial
  synthetic DNA
ggttgctccgtctgttcagcacactgtta

SEQ ID NO: 1733 - DNA, 29 bp, Artificial
  synthetic DNA
aatgtcgactggccattatcgccaagtgt

SEQ ID NO: 1734 - DNA, 29 bp, Artificial
  synthetic DNA
gatagcttgccatgcgaatggatctccag

SEQ ID NO: 1735 - DNA, 29 bp, Artificial
  synthetic DNA
ccagaccggagccaattggctgccaatat

SEQ ID NO: 1736 - DNA, 29 bp, Artificial
  synthetic DNA
aacgtcgctccatacgttacctaatgcag

SEQ ID NO: 1737 - DNA, 29 bp, Artificial
  synthetic DNA
gaatatgacgcgaacagtctattcggatc

SEQ ID NO: 1738 - DNA, 29 bp, Artificial
  synthetic DNA
gacgagaatgtattaaggataagcaaggt

SEQ ID NO: 1739 - DNA, 29 bp, Artificial
  synthetic DNA
aagtcgtatgaatcgctatcacatgagtc

SEQ ID NO: 1740 - DNA, 29 bp, Artificial
  synthetic DNA
gtcgtggagactacaattctcctcacgtt

SEQ ID NO: 1741 - DNA, 29 bp, Artificial
  synthetic DNA
gttgccaccgttacacgactatcgacagt

SEQ ID NO: 1742 - DNA, 29 bp, Artificial
  synthetic DNA
aggataggctacgccttactctcctaagc

SEQ ID NO: 1743 - DNA, 29 bp, Artificial
  synthetic DNA
taatcatcctgttcgcctcgaggttgtta

SEQ ID NO: 1744 - DNA, 29 bp, Artificial
  synthetic DNA
gacaagcagtaataattactgagtggacg

SEQ ID NO: 1745 - DNA, 29 bp, Artificial
  synthetic DNA
tacagcgttacgcaggtatatcaaggtag

SEQ ID NO: 1746 - DNA, 29 bp, Artificial
  synthetic DNA
ctaacatcacttactattagcggtctcgt

SEQ ID NO: 1747 - DNA, 29 bp, Artificial
  synthetic DNA
ccgcgcttcttgacacgttctccactagg

SEQ ID NO: 1748 - DNA, 29 bp, Artificial
  synthetic DNA
caagtaacatgagatgctatcggtacatt

SEQ ID NO: 1749 - DNA, 29 bp, Artificial
  synthetic DNA
cgaccactaggctgtgaccacgatacgct

SEQ ID NO: 1750 - DNA, 29 bp, Artificial
  synthetic DNA
caggtcatgtgacgcagtcggcagtcaac

SEQ ID NO: 1751 - DNA, 29 bp, Artificial
  synthetic DNA
actccatcgttagttcttccgccgtgctg

SEQ ID NO: 1752 - DNA, 29 bp, Artificial
  synthetic DNA
ctcaccacgtatgcgtcactcggttacgt

SEQ ID NO: 1753 - DNA, 29 bp, Artificial
  synthetic DNA
tgcctatgctatggaccttgcgcgactct

SEQ ID NO: 1754 - DNA, 29 bp, Artificial
  synthetic DNA
aatgaaggtcaacgctctgtagttacgcg

SEQ ID NO: 1755 - DNA, 29 bp, Artificial
  synthetic DNA
caccattgattcatggcttccatcactgc

SEQ ID NO: 1756 - DNA, 29 bp, Artificial
  synthetic DNA
gacacgcaaggtaattcgagattgcagca

SEQ ID NO: 1757 - DNA, 29 bp, Artificial
  synthetic DNA
caccgagaggaaggttcgatcgcttctcg

SEQ ID NO: 1758 - DNA, 29 bp, Artificial
  synthetic DNA
cagttatcggattgtgatattcactcctg

SEQ ID NO: 1759 - DNA, 29 bp, Artificial
  synthetic DNA
atactgtaacgcctcaacctatgctgact

SEQ ID NO: 1760 - DNA, 29 bp, Artificial
  synthetic DNA
atctgtcttattctggcacactcagactt

SEQ ID NO: 1761 - DNA, 29 bp, Artificial
  synthetic DNA
tccaaccggtgacgtgctcttgatccaac

SEQ ID NO: 1762 - DNA, 29 bp, Artificial
  synthetic DNA
cacactcagttcggctatctctgcgatag

SEQ ID NO: 1763 - DNA, 29 bp, Artificial
  synthetic DNA
agctgtaagtcaggtctacgactcgtact

SEQ ID NO: 1764 - DNA, 29 bp, Artificial
  synthetic DNA
gtcggcggcacgcacagctaacattcgta

SEQ ID NO: 1765 - DNA, 29 bp, Artificial
  synthetic DNA
atatggtagccagccacgtatactgaaca

SEQ ID NO: 1766 - DNA, 29 bp, Artificial
  synthetic DNA
tggacaatccgactctaacacagaggtag

SEQ ID NO: 1767 - DNA, 29 bp, Artificial
  synthetic DNA
tccgccgctgacagttcaatctatcaatt

SEQ ID NO: 1768 - DNA, 29 bp, Artificial
  synthetic DNA
ggttccttagaatatgcacctatcagcga

SEQ ID NO: 1769 - DNA, 29 bp, Artificial
  synthetic DNA
cggctgtacgacatggatcataagagtgt

SEQ ID NO: 1770 - DNA, 29 bp, Artificial
  synthetic DNA
tgcagatgtacgctgtggccagtggagag

SEQ ID NO: 1771 - DNA, 29 bp, Artificial
  synthetic DNA
cctactcacttaacaataatcggttcggt

SEQ ID NO: 1772 - DNA, 29 bp, Artificial
  synthetic DNA
cgcttcctactgcctgtgccgcgacataa

SEQ ID NO: 1773 - DNA, 29 bp, Artificial
  synthetic DNA
ctagaccgaccggttatgcgctattgttc

SEQ ID NO: 1774 - DNA, 29 bp, Artificial
  synthetic DNA
ttgtgagcacgtctgcggcaagcctatgg

SEQ ID NO: 1775 - DNA, 29 bp, Artificial
  synthetic DNA
tcatcggccggcgctgttgttgttaccat

SEQ ID NO: 1776 - DNA, 29 bp, Artificial
  synthetic DNA
gcggttaggtgcagttaggaagactatca

SEQ ID NO: 1777 - DNA, 29 bp, Artificial
  synthetic DNA
tatgcggtcgtgaggcgtagcattctaga

SEQ ID NO: 1778 - DNA, 29 bp, Artificial
  synthetic DNA
ccatctattcgtcgaactctcagctcgta

SEQ ID NO: 1779 - DNA, 29 bp, Artificial
  synthetic DNA
atcagatctactgatcgcggtagagtatc

SEQ ID NO: 1780 - DNA, 29 bp, Artificial
  synthetic DNA
tacacataggcggcgcagccttctaatta

SEQ ID NO: 1781 - DNA, 29 bp, Artificial
  synthetic DNA
ttaaccgtagttcttagcttacgccgctc

SEQ ID NO: 1782 - DNA, 29 bp, Artificial
  synthetic DNA
actatagaggacatggcactcctcttcta

SEQ ID NO: 1783 - DNA, 29 bp, Artificial
  synthetic DNA
cagttcgtattaagattgaatgtagcggt

SEQ ID NO: 1784 - DNA, 29 bp, Artificial
  synthetic DNA
agttatcggtatccgcttatccgtacgta

SEQ ID NO: 1785 - DNA, 29 bp, Artificial
  synthetic DNA
agcttattcatacactgcaccacagcaag

SEQ ID NO: 1786 - DNA, 29 bp, Artificial
  synthetic DNA
ccgtcggctagtctatcctctaattagaa

SEQ ID NO: 1787 - DNA, 29 bp, Artificial
  synthetic DNA
gtccgcttccatgcctgctgtacgaacac

SEQ ID NO: 1788 - DNA, 29 bp, Artificial
  synthetic DNA
tctcttcctccttcattgttcgctagctc

SEQ ID NO: 1789 - DNA, 29 bp, Artificial
  synthetic DNA
tctcttgagcggtcctcatacaggtctgc

SEQ ID NO: 1790 - DNA, 29 bp, Artificial
  synthetic DNA
gaccaagtgtaggtgatatcaccggtact

SEQ ID NO: 1791 - DNA, 29 bp, Artificial
  synthetic DNA
aagattgtgataggttggtagttaccaca

SEQ ID NO: 1792 - DNA, 29 bp, Artificial
  synthetic DNA
tcgcctccgaagagtatagcatcggcaga

SEQ ID NO: 1793 - DNA, 29 bp, Artificial
  synthetic DNA
gaggtagttatgagcatcgaggtcctgtt

SEQ ID NO: 1794 - DNA, 29 bp, Artificial
  synthetic DNA
ggacgcaagatcgcaggtacttgtaagct

SEQ ID NO: 1795 - DNA, 29 bp, Artificial
  synthetic DNA
actcgtacacgtcatcgtgcaggtctcag

SEQ ID NO: 1796 - DNA, 29 bp, Artificial
  synthetic DNA
taatccgtcaggagtgagatggctcgaca

SEQ ID NO: 1797 - DNA, 29 bp, Artificial
  synthetic DNA
aagatggttccgcgcattgactagcaagt

SEQ ID NO: 1798 - DNA, 29 bp, Artificial
  synthetic DNA
tccgcgatctgcggatcttgaatgctcac

SEQ ID NO: 1799 - DNA, 29 bp, Artificial
  synthetic DNA
ttcacgagagtcaactgctagtatcctag

SEQ ID NO: 1800 - DNA, 29 bp, Artificial
  synthetic DNA
ttccaactggattcttccaactcctcgaa

SEQ ID NO: 1801 - DNA, 29 bp, Artificial
  synthetic DNA
cactactactcaagttatacggtgttgac

SEQ ID NO: 1802 - DNA, 29 bp, Artificial
  synthetic DNA
caactggattctcaggatgcgtctctagc

SEQ ID NO: 1803 - DNA, 29 bp, Artificial
  synthetic DNA
tggactagagtggagcgattacgtaatat

SEQ ID NO: 1804 - DNA, 29 bp, Artificial
  synthetic DNA
gaggtcattcaactggactcgccacggac

SEQ ID NO: 1805 - DNA, 29 bp, Artificial
  synthetic DNA
caggtgtgtaacgctgcaatcacatgaat

SEQ ID NO: 1806 - DNA, 29 bp, Artificial
  synthetic DNA
tatgctgaggtattagttctaactatgcg

SEQ ID NO: 1807 - DNA, 29 bp, Artificial
  synthetic DNA
cgtctgagtcggataaggaaggttaccgc

SEQ ID NO: 1808 - DNA, 29 bp, Artificial
  synthetic DNA
gtactatcgtcgcaggcactatctctgcc

SEQ ID NO: 1809 - DNA, 29 bp, Artificial
  synthetic DNA
gcttcctccttgcaacttcattgcttcga

SEQ ID NO: 1810 - DNA, 29 bp, Artificial
  synthetic DNA
tgtctacgaagtagaagacacgaataatg

SEQ ID NO: 1811 - DNA, 29 bp, Artificial
  synthetic DNA
ccgtcatctaaggcagagtacatccgcga

SEQ ID NO: 1812 - DNA, 29 bp, Artificial
  synthetic DNA
ccggaggcgtactaactgaccacaacacc

SEQ ID NO: 1813 - DNA, 29 bp, Artificial
  synthetic DNA
aactcgtcgctgcctgaataggtcagagt

SEQ ID NO: 1814 - DNA, 29 bp, Artificial
  synthetic DNA
ttataagattaatgtcggtcagtgtcgga

SEQ ID NO: 1815 - DNA, 29 bp, Artificial
  synthetic DNA
cgtctcgatggatccacacgaacctgttg

SEQ ID NO: 1816 - DNA, 29 bp, Artificial
  synthetic DNA
atgccatcatggtcgtcctatcttaaggc

SEQ ID NO: 1817 - DNA, 29 bp, Artificial
  synthetic DNA
gcgcttcagcgattcgtcatgcaaggcac

SEQ ID NO: 1818 - DNA, 29 bp, Artificial
  synthetic DNA
ccaagcgataccgaggtacggttaacgag

SEQ ID NO: 1819 - DNA, 29 bp, Artificial
  synthetic DNA
atatgacagacaggtggacctaagcaagc

SEQ ID NO: 1820 - DNA, 29 bp, Artificial
  synthetic DNA
cactacatcgtcaggcctggaagcctcag

SEQ ID NO: 1821 - DNA, 29 bp, Artificial
  synthetic DNA
gccgtgtagacgaggacattatgtcgtat

SEQ ID NO: 1822 - DNA, 29 bp, Artificial
  synthetic DNA
caacgtatatacacaccttgtgaagagaa

SEQ ID NO: 1823 - DNA, 29 bp, Artificial
  synthetic DNA
tccaacgtaattccgccgtctgtcgagac

SEQ ID NO: 1824 - DNA, 29 bp, Artificial
  synthetic DNA
aattcgtgcttcgatcaccgtagactcag

SEQ ID NO: 1825 - DNA, 30 bp, Artificial
  synthetic DNA
actatattgtattcacgtccgacgactcgc

SEQ ID NO: 1826 - DNA, 30 bp, Artificial
  synthetic DNA
gacgagcttgtggtacactatacctatgag

SEQ ID NO: 1827 - DNA, 30 bp, Artificial
  synthetic DNA
tgattcaagcaccaggcatgcttaagctag

SEQ ID NO: 1828 - DNA, 30 bp, Artificial
  synthetic DNA
cggtctcctataggaaggctcattctgacg

SEQ ID NO: 1829 - DNA, 30 bp, Artificial
  synthetic DNA
agtcagtgtcgaatcaatcaaggcgtcctt

SEQ ID NO: 1830 - DNA, 30 bp, Artificial
  synthetic DNA
cgaacgtaatggccatcacgcgctggccta

SEQ ID NO: 1831 - DNA, 30 bp, Artificial
  synthetic DNA
cgaacctggaccacctggcattaccattac

SEQ ID NO: 1832 - DNA, 30 bp, Artificial
  synthetic DNA
acattaggttcctgtaatgtcttatcaacg

SEQ ID NO: 1833 - DNA, 30 bp, Artificial
  synthetic DNA
cgtctaatgcaccgtatcgtcttcgcgcat

SEQ ID NO: 1834 - DNA, 30 bp, Artificial
  synthetic DNA
tctatgacttacaacggaatcttacttcgt

SEQ ID NO: 1835 - DNA, 30 bp, Artificial
  synthetic DNA
gtaaccgatcggtaccgtctgctattgttc

SEQ ID NO: 1836 - DNA, 30 bp, Artificial
  synthetic DNA
ggtgattgataagcaacacatattaggagg

SEQ ID NO: 1837 - DNA, 30 bp, Artificial
  synthetic DNA
aattatcgacgctaataggcgagctgttca

SEQ ID NO: 1838 - DNA, 30 bp, Artificial
  synthetic DNA
ggaggtacatgacgagtggacagacagacc

SEQ ID NO: 1839 - DNA, 30 bp, Artificial
  synthetic DNA
ctctaatccgttatgcggtgatgtaatccg

SEQ ID NO: 1840 - DNA, 30 bp, Artificial
  synthetic DNA
gcaagcacgcggcttggcgaacttctatgc

SEQ ID NO: 1841 - DNA, 30 bp, Artificial
  synthetic DNA
tagatgtaggcctggtaggcagaggagtaa

SEQ ID NO: 1842 - DNA, 30 bp, Artificial
  synthetic DNA
ccgagtggcgaccacacaggtacgcattaa

SEQ ID NO: 1843 - DNA, 30 bp, Artificial
  synthetic DNA
gtcctggctcagattagtgcacttagttat

SEQ ID NO: 1844 - DNA, 30 bp, Artificial
  synthetic DNA
gcggtacctacatgttatgactcagacgac

SEQ ID NO: 1845 - DNA, 30 bp, Artificial
  synthetic DNA
tctctgccaatgctggtctcatcgaatcca

SEQ ID NO: 1846 - DNA, 30 bp, Artificial
  synthetic DNA
tctctacacagctacatactatactgtaac

SEQ ID NO: 1847 - DNA, 30 bp, Artificial
  synthetic DNA
tacgacggacgctggtggtgtaagagaagg

SEQ ID NO: 1848 - DNA, 30 bp, Artificial
  synthetic DNA
gcctcgatatatctacgtatagttcaagtt

SEQ ID NO: 1849 - DNA, 30 bp, Artificial
  synthetic DNA
ggctcctgcattcattgaaggtcggccttg

SEQ ID NO: 1850 - DNA, 30 bp, Artificial
  synthetic DNA
cagttcggtgattcaagagaacaatggtgg

SEQ ID NO: 1851 - DNA, 30 bp, Artificial
  synthetic DNA
tataacgaagccggctggaacggtaactca

SEQ ID NO: 1852 - DNA, 30 bp, Artificial
  synthetic DNA
ctgtatcaattcaagtgacagtggcacgtc

SEQ ID NO: 1853 - DNA, 30 bp, Artificial
  synthetic DNA
agcaattgcggttcataggcgtaattatat

SEQ ID NO: 1854 - DNA, 30 bp, Artificial
  synthetic DNA
catatggacctggagatcaccgttcagtcc

SEQ ID NO: 1855 - DNA, 30 bp, Artificial
  synthetic DNA
gaaggccgttggtctatctcttactggagc

SEQ ID NO: 1856 - DNA, 30 bp, Artificial
  synthetic DNA
gtgcgttcatctagcctaagacgctgacct

SEQ ID NO: 1857 - DNA, 30 bp, Artificial
  synthetic DNA
gagtaacttatatcctctctacgacatcga

SEQ ID NO: 1858 - DNA, 30 bp, Artificial
  synthetic DNA
attctacgctgatgtctccgctgaacagga

SEQ ID NO: 1859 - DNA, 30 bp, Artificial
  synthetic DNA
tcatcaacgttactcactagtaccacggct

SEQ ID NO: 1860 - DNA, 30 bp, Artificial
  synthetic DNA
aaccattcttgaacgttgagaacctggtgg

SEQ ID NO: 1861 - DNA, 30 bp, Artificial
  synthetic DNA
acgacacctccgcggaacatacctgattag

SEQ ID NO: 1862 - DNA, 30 bp, Artificial
  synthetic DNA
gcgcacttattgaagtaatctcatggccaa

SEQ ID NO: 1863 - DNA, 30 bp, Artificial
  synthetic DNA
gcgccaattcagccagttagcgtctccgtg

SEQ ID NO: 1864 - DNA, 30 bp, Artificial
  synthetic DNA
agcaacaagtcgctgtatatcgactggccg

SEQ ID NO: 1865 - DNA, 30 bp, Artificial
  synthetic DNA
ccttacaatagacctcgcggcgttcatgcc

SEQ ID NO: 1866 - DNA, 30 bp, Artificial
  synthetic DNA
ggatccaacttcagcgaagcaccaacgtcg

SEQ ID NO: 1867 - DNA, 30 bp, Artificial
  synthetic DNA
gcgccagttctcgtactctcgagaagcgac

SEQ ID NO: 1868 - DNA, 30 bp, Artificial
  synthetic DNA
gagtgcggccaatctggaactcatgacgtt

SEQ ID NO: 1869 - DNA, 30 bp, Artificial
  synthetic DNA
cctgagagtgattcgtgtctgcgaagatgc

SEQ ID NO: 1870 - DNA, 30 bp, Artificial
  synthetic DNA
gtgactggttaaggcaatattggtcgaccg

SEQ ID NO: 1871 - DNA, 30 bp, Artificial
  synthetic DNA
ctatcaagccttacaaggtcacgtccacta

SEQ ID NO: 1872 - DNA, 30 bp, Artificial
  synthetic DNA
actgcgtccttgcgtcggaactccttgtgt

SEQ ID NO: 1873 - DNA, 30 bp, Artificial
  synthetic DNA
tgcaactcagtggcggcgacaccaagagct

SEQ ID NO: 1874 - DNA, 30 bp, Artificial
  synthetic DNA
ttcggttctactaggatctctatctgagct

SEQ ID NO: 1875 - DNA, 30 bp, Artificial
  synthetic DNA
agctaatctattaagacagattagacagga

SEQ ID NO: 1876 - DNA, 30 bp, Artificial
  synthetic DNA
ggaccgctcttaggttatgcacctgcgtat

SEQ ID NO: 1877 - DNA, 30 bp, Artificial
  synthetic DNA
ctctaatactagtccacaggttagtacgaa

SEQ ID NO: 1878 - DNA, 30 bp, Artificial
  synthetic DNA
atccatatatgctcgtcgtcagccagtgtt

SEQ ID NO: 1879 - DNA, 30 bp, Artificial
  synthetic DNA
gctattactgtgttgatgtccacaggagaa

SEQ ID NO: 1880 - DNA, 30 bp, Artificial
  synthetic DNA
gctacggcgcagatctagacaactggaagt

SEQ ID NO: 1881 - DNA, 30 bp, Artificial
  synthetic DNA
gcctcttgtgttagccgaataccaatgacc

SEQ ID NO: 1882 - DNA, 30 bp, Artificial
  synthetic DNA
tgaggacgataacattacctctcgagtcgc

SEQ ID NO: 1883 - DNA, 30 bp, Artificial
  synthetic DNA
cgattaccaatccgacgacttcgcagcagc

SEQ ID NO: 1884 - DNA, 30 bp, Artificial
  synthetic DNA
atgacacgagtccagtacatatgcgaagac

SEQ ID NO: 1885 - DNA, 30 bp, Artificial
  synthetic DNA
gcgctcgcatgcactagtgtagactgacga

SEQ ID NO: 1886 - DNA, 30 bp, Artificial
  synthetic DNA
gcacatctcagaattgatggtctatgtcgc

SEQ ID NO: 1887 - DNA, 30 bp, Artificial
  synthetic DNA
ttcttcgacgccgcgtactaataggtcaat

SEQ ID NO: 1888 - DNA, 30 bp, Artificial
  synthetic DNA
ggaagcgcctctaacaaccgatgcttgtgg

SEQ ID NO: 1889 - DNA, 30 bp, Artificial
  synthetic DNA
ctctagacgcgtcgtgactccaatctgttg

SEQ ID NO: 1890 - DNA, 30 bp, Artificial
  synthetic DNA
gtagttcgtcggagtgacctcgtactcact

SEQ ID NO: 1891 - DNA, 30 bp, Artificial
  synthetic DNA
atgctgtcgagtgtccggcatagagcacac

SEQ ID NO: 1892 - DNA, 30 bp, Artificial
  synthetic DNA
gcgcatcttgcagcgtcctgtagttctgaa

SEQ ID NO: 1893 - DNA, 30 bp, Artificial
  synthetic DNA
gcgattgttgaggaaccacagcggcaccta

SEQ ID NO: 1894 - DNA, 30 bp, Artificial
  synthetic DNA
cacgcgtactctgcttgctgtgtggtcggt

SEQ ID NO: 1895 - DNA, 30 bp, Artificial
  synthetic DNA
catccaacgcaggacctagtagtcatgctt

SEQ ID NO: 1896 - DNA, 30 bp, Artificial
  synthetic DNA
ttctagttgtgatgagaatcgctagcgtgc

SEQ ID NO: 1897 - DNA, 30 bp, Artificial
  synthetic DNA
cattctgaatctggtctctctcgatcatcc

SEQ ID NO: 1898 - DNA, 30 bp, Artificial
  synthetic DNA
attaatgtagaggatagttccgttctctcc

SEQ ID NO: 1899 - DNA, 30 bp, Artificial
  synthetic DNA
gtatcgcgcttacgaatgaggtgtggcttc

SEQ ID NO: 1900 - DNA, 30 bp, Artificial
  synthetic DNA
gctggtgagagagccagattatcggtggag

SEQ ID NO: 1901 - DNA, 30 bp, Artificial
  synthetic DNA
ggcacgagcaggtagaactagaacctagat

SEQ ID NO: 1902 - DNA, 30 bp, Artificial
  synthetic DNA
tgtattatctcgaagcggtgcgttagagtc

SEQ ID NO: 1903 - DNA, 30 bp, Artificial
  synthetic DNA
cacgtgttctagctactaatggcgtcaatt

SEQ ID NO: 1904 - DNA, 30 bp, Artificial
  synthetic DNA
cgcgctacattacttcctacaccatgcgta

SEQ ID NO: 1905 - DNA, 30 bp, Artificial
  synthetic DNA
tgaggcaactagtgttcgcaagatgacgga

SEQ ID NO: 1906 - DNA, 30 bp, Artificial
  synthetic DNA
ttattattgtctgtggaacgcacgccagtc

SEQ ID NO: 1907 - DNA, 30 bp, Artificial
  synthetic DNA
gctatagtattatccatgaattccgtcggc

SEQ ID NO: 1908 - DNA, 30 bp, Artificial
  synthetic DNA
gtatcaatagctcaattcgtcagagttgtg

SEQ ID NO: 1909 - DNA, 30 bp, Artificial
  synthetic DNA
tagtccatgcgtggatatattgagagctga

SEQ ID NO: 1910 - DNA, 30 bp, Artificial
  synthetic DNA
gcacagtacgacttataacaggtctagatc

SEQ ID NO: 1911 - DNA, 30 bp, Artificial
  synthetic DNA
actcaatggtggcacgctcggcgcagcata

SEQ ID NO: 1912 - DNA, 30 bp, Artificial
  synthetic DNA
gtagtaccactccgccttaggcagcttaag

SEQ ID NO: 1913 - DNA, 30 bp, Artificial
  synthetic DNA
cgctcaactgatgcgtgcaaccaatgttat

SEQ ID NO: 1914 - DNA, 30 bp, Artificial
  synthetic DNA
gcagcttgactgcctagacagcagttacag

SEQ ID NO: 1915 - DNA, 30 bp, Artificial
  synthetic DNA
gcaacttcttagtacgaattcatcgtccaa

SEQ ID NO: 1916 - DNA, 30 bp, Artificial
  synthetic DNA
atccgtatgctgcggcagtggaggtggctt

SEQ ID NO: 1917 - DNA, 30 bp, Artificial
  synthetic DNA
tgcggatcaatccagttctgtgtactgtga

SEQ ID NO: 1918 - DNA, 30 bp, Artificial
  synthetic DNA
ttatgattatcaccggcgtaacattccgaa

SEQ ID NO: 1919 - DNA, 30 bp, Artificial
  synthetic DNA
gctacctagattcttcaactcatcgctacc

SEQ ID NO: 1920 - DNA, 30 bp, Artificial
  synthetic DNA
cagtgttagaatggcggtgtgtagccgcta

SEQ ID NO: 1921 - DNA, 35 bp, Artificial
  synthetic DNA
gcttatagactacagctgcgaggtataaggtcact

SEQ ID NO: 1922 - DNA, 35 bp, Artificial
  synthetic DNA
cgctcagcaggatgctatcctaagttaatgtggtg

SEQ ID NO: 1923 - DNA, 35 bp, Artificial
  synthetic DNA
gaactgagcggacatcagctaggcctacaatacat

SEQ ID NO: 1924 - DNA, 35 bp, Artificial
  synthetic DNA
tcgtgaacttctgcgttggtctctaccaaggcggt

SEQ ID NO: 1925 - DNA, 35 bp, Artificial
  synthetic DNA
taagtcaggtatcttatcagtggtacacggtacga

SEQ ID NO: 1926 - DNA, 35 bp, Artificial
  synthetic DNA
taataatgttgcgcgtgaccgaggaggaatccact

SEQ ID NO: 1927 - DNA, 35 bp, Artificial
  synthetic DNA
ctaggagttctcgtaagctggagtaccgtaacgtg

SEQ ID NO: 1928 - DNA, 35 bp, Artificial
  synthetic DNA
ggactctcctcagaggatccttcttgcgcaggcat

SEQ ID NO: 1929 - DNA, 35 bp, Artificial
  synthetic DNA
gctagaggcctgagtacaccttctcgcatcaggat

SEQ ID NO: 1930 - DNA, 35 bp, Artificial
  synthetic DNA
atatcgcgagcactaacgtcgttgtcgttctagga

SEQ ID NO: 1931 - DNA, 35 bp, Artificial
  synthetic DNA
agcggttactatacctggcggctgacgttgttagt

SEQ ID NO: 1932 - DNA, 35 bp, Artificial
  synthetic DNA
gagctaggtagatctccaagtgtagctaagaagag

SEQ ID NO: 1933 - DNA, 35 bp, Artificial
  synthetic DNA
ggagtcgctggtgacgtatgccgaggatgagcttc

SEQ ID NO: 1934 - DNA, 35 bp, Artificial
  synthetic DNA
cgccgacctcctgttcacgaagccgcctgatgtaa

SEQ ID NO: 1935 - DNA, 35 bp, Artificial
  synthetic DNA
agtaggcacttagttatcgattacgttagttagtc

SEQ ID NO: 1936 - DNA, 35 bp, Artificial
  synthetic DNA
ggatgacgtctcagtctacctcgcagtgtcgtcta

SEQ ID NO: 1937 - DNA, 35 bp, Artificial
  synthetic DNA
ctggttcgcgttagcaatactaaggcagtcaggag

SEQ ID NO: 1938 - DNA, 35 bp, Artificial
  synthetic DNA
atatggtcatattggcctcttcgaacacagactgt

SEQ ID NO: 1939 - DNA, 35 bp, Artificial
  synthetic DNA
tatcagaggatagcaggtctgagttgcaaggctaa

SEQ ID NO: 1940 - DNA, 35 bp, Artificial
  synthetic DNA
ggtggtctgaccatagctgttcttctcacagagac

SEQ ID NO: 1941 - DNA, 35 bp, Artificial
  synthetic DNA
gcaataccaacgagatgagtattcgttgaagctct

SEQ ID NO: 1942 - DNA, 35 bp, Artificial
  synthetic DNA
ccaagtcgacgctgcatgaatgagcgctattcact

SEQ ID NO: 1943 - DNA, 35 bp, Artificial
  synthetic DNA
ccattagatcgcttcgagacaattaggagacatga

SEQ ID NO: 1944 - DNA, 35 bp, Artificial
  synthetic DNA
gatgactgtacctcctatcattgagtgtggaccaa

SEQ ID NO: 1945 - DNA, 35 bp, Artificial
  synthetic DNA
atatctggatgaatagtggttaggtaagcaagtaa

SEQ ID NO: 1946 - DNA, 35 bp, Artificial
  synthetic DNA
accgactatgttaattcgtgtctggatggcagaat

SEQ ID NO: 1947 - DNA, 35 bp, Artificial
  synthetic DNA
gtggcagtcttgctagtatcttagaccatcaccaa

SEQ ID NO: 1948 - DNA, 35 bp, Artificial
  synthetic DNA
cgctatcttagtcgagcacaatgtcttcgtatagg

SEQ ID NO: 1949 - DNA, 35 bp, Artificial
  synthetic DNA
attagtacggcacgaaccggccattcatggcagct

SEQ ID NO: 1950 - DNA, 35 bp, Artificial
  synthetic DNA
agtacgactatcaagactccagcgctctccttgga

SEQ ID NO: 1951 - DNA, 35 bp, Artificial
  synthetic DNA
atgagcctcggagcgaacgttatcgatcaggctgt

SEQ ID NO: 1952 - DNA, 35 bp, Artificial
  synthetic DNA
ttgcgtgcagtagcaccgatacacagcgcttgtat

SEQ ID NO: 1953 - DNA, 35 bp, Artificial
  synthetic DNA
aacggctgcatcacctacactatactcaacatcta

SEQ ID NO: 1954 - DNA, 35 bp, Artificial
  synthetic DNA
gtcgctatgcgagaagtggcgtggaatgctatggt

SEQ ID NO: 1955 - DNA, 35 bp, Artificial
  synthetic DNA
catggatacctactgacttgacttctagaggaccg

SEQ ID NO: 1956 - DNA, 35 bp, Artificial
  synthetic DNA
gagtgacgcagacaccgtaacgtcgaatcttctag

SEQ ID NO: 1957 - DNA, 35 bp, Artificial
  synthetic DNA
agtaccgtctgtgtgaatattgttcctacgttaca

SEQ ID NO: 1958 - DNA, 35 bp, Artificial
  synthetic DNA
ggctaatcgatagtgacgagttctgcacgcctgaa

SEQ ID NO: 1959 - DNA, 35 bp, Artificial
  synthetic DNA
ggcgagcgctcgtggttctgagtcgctgttagatg

SEQ ID NO: 1960 - DNA, 35 bp, Artificial
  synthetic DNA
tatctccagcgttataagctactggagccgctcgg

SEQ ID NO: 1961 - DNA, 35 bp, Artificial
  synthetic DNA
ccttctgcgcaagtcaaggattcgcttagatggac

SEQ ID NO: 1962 - DNA, 35 bp, Artificial
  synthetic DNA
gttgctgacagccgttgcgtacttgccttaagaac

SEQ ID NO: 1963 - DNA, 35 bp, Artificial
  synthetic DNA
gtggcctaatcactcgcgcttcataggccgatagg

SEQ ID NO: 1964 - DNA, 35 bp, Artificial
  synthetic DNA
tgcatctagcctacatcggaccttgttatggtaat

SEQ ID NO: 1965 - DNA, 35 bp, Artificial
  synthetic DNA
ggacagctactggacaccaccgaactggtagtgtc

SEQ ID NO: 1966 - DNA, 35 bp, Artificial
  synthetic DNA
aactggcgatggacggccgctcttccgctacatag

SEQ ID NO: 1967 - DNA, 35 bp, Artificial
  synthetic DNA
ggagcagttagctatggagcaggccgataacctga

SEQ ID NO: 1968 - DNA, 35 bp, Artificial
  synthetic DNA
actctacggtgcacctcagccttcatgcaataggc

SEQ ID NO: 1969 - DNA, 35 bp, Artificial
  synthetic DNA
cttgtagcacaatacattactctccacgtgatagc

SEQ ID NO: 1970 - DNA, 35 bp, Artificial
  synthetic DNA
ggacgctatcgataccgttattcctactctgtcgg

SEQ ID NO: 1971 - DNA, 35 bp, Artificial
  synthetic DNA
ggatgatcgtcaacgatcaactgacagttagtcga

SEQ ID NO: 1972 - DNA, 35 bp, Artificial
  synthetic DNA
tgacagtagcaatgtctcacgtctgcacaacggaa

SEQ ID NO: 1973 - DNA, 35 bp, Artificial
  synthetic DNA
gtcgcaggacctcacggatagtagtgcgaggtcta

SEQ ID NO: 1974 - DNA, 35 bp, Artificial
  synthetic DNA
atatcggcggacgcaatgacagttgttggctgatg

SEQ ID NO: 1975 - DNA, 35 bp, Artificial
  synthetic DNA
aagcaccaaggaggtatgttccatcgaggcgctcg

SEQ ID NO: 1976 - DNA, 35 bp, Artificial
  synthetic DNA
gaccgcaccttatagctatatcctggtctagtact

SEQ ID NO: 1977 - DNA, 35 bp, Artificial
  synthetic DNA
tctcagaggaaggttgagcgtctgaccaggttggc

SEQ ID NO: 1978 - DNA, 35 bp, Artificial
  synthetic DNA
tggacctagagacctagctcgtctcttcgcgatcg

SEQ ID NO: 1979 - DNA, 35 bp, Artificial
  synthetic DNA
cggagtggttccacgcgacctcgcaactaatcctt

SEQ ID NO: 1980 - DNA, 35 bp, Artificial
  synthetic DNA
ggagccgcgcgcagactgaccttgcttgatctact

SEQ ID NO: 1981 - DNA, 35 bp, Artificial
  synthetic DNA
actctaagtatatgcgcagttagtatactgaacca

SEQ ID NO: 1982 - DNA, 35 bp, Artificial
  synthetic DNA
gagcattgcttcgcttcgatgtctattctgatcag

SEQ ID NO: 1983 - DNA, 35 bp, Artificial
  synthetic DNA
gcttgtattgccactcgagtaggtcgtggcagtag

SEQ ID NO: 1984 - DNA, 35 bp, Artificial
  synthetic DNA
atctggacattgcattcggtgtgtatacagaaggc

SEQ ID NO: 1985 - DNA, 35 bp, Artificial
  synthetic DNA
ggttgcgatcagcttgatagcaggtcatatcctca

SEQ ID NO: 1986 - DNA, 35 bp, Artificial
  synthetic DNA
gcaggtactaacctgagatgcgtagctaacacagg

SEQ ID NO: 1987 - DNA, 35 bp, Artificial
  synthetic DNA
atctgcaaggacgtaacgtcctcggaaggtgaggt

SEQ ID NO: 1988 - DNA, 35 bp, Artificial
  synthetic DNA
ataatcttacgagcctccagtgaataatgcaagca

SEQ ID NO: 1989 - DNA, 35 bp, Artificial
  synthetic DNA
caatctccgcacagtcttgttcaggtacagactta

SEQ ID NO: 1990 - DNA, 35 bp, Artificial
  synthetic DNA
atgtgcgcaattcagcgtaagtgcctattcataat

SEQ ID NO: 1991 - DNA, 35 bp, Artificial
  synthetic DNA
tcggacgcacacatcctgttgtcgagaagaggaag

SEQ ID NO: 1992 - DNA, 35 bp, Artificial
  synthetic DNA
tcggaagcatcacatgagcatcaggagttcattgc

SEQ ID NO: 1993 - DNA, 35 bp, Artificial
  synthetic DNA
atctggttgtggacttctatacagtaccagagtgg

SEQ ID NO: 1994 - DNA, 35 bp, Artificial
  synthetic DNA
cgtctgaatatagttagctagtagtgtaatccagg

SEQ ID NO: 1995 - DNA, 35 bp, Artificial
  synthetic DNA
taatatctgatccgacctattatctaggactactc

SEQ ID NO: 1996 - DNA, 35 bp, Artificial
  synthetic DNA
tatgcggccgtccgtacctcgtctgcttcagttgg

SEQ ID NO: 1997 - DNA, 35 bp, Artificial
  synthetic DNA
tggctcaagttccatattgccaagacgacctggag

SEQ ID NO: 1998 - DNA, 35 bp, Artificial
  synthetic DNA
gcagttctgctaggcggtccgaggcaattgaagag

SEQ ID NO: 1999 - DNA, 35 bp, Artificial
  synthetic DNA
catggcacagacgaagtatgcaccacgctcattaa

SEQ ID NO: 2000 - DNA, 35 bp, Artificial
  synthetic DNA
ggagcgtactacgaccattcaaccgaatatgttac

SEQ ID NO: 2001 - DNA, 35 bp, Artificial
  synthetic DNA
gcgtagatctcgcgacagagacaaggtgcgaatgg

SEQ ID NO: 2002 - DNA, 35 bp, Artificial
  synthetic DNA
tggactgaggttctccggtctatactcctgtagga

SEQ ID NO: 2003 - DNA, 35 bp, Artificial
  synthetic DNA
tggctatagcaacggcttcttgtgatcgcattgca

SEQ ID NO: 2004 - DNA, 35 bp, Artificial
  synthetic DNA
ggcgaagaatcatgcgagacggagtagacggacgt

SEQ ID NO: 2005 - DNA, 35 bp, Artificial
  synthetic DNA
gagcattgcgagttgcacacgtgatatcagactgt

SEQ ID NO: 2006 - DNA, 35 bp, Artificial
  synthetic DNA
ctgttgacctatgccagaatcaatacctcagatta

SEQ ID NO: 2007 - DNA, 35 bp, Artificial
  synthetic DNA
gttaacaagtagatgccaagatacaacgagagacc

SEQ ID NO: 2008 - DNA, 35 bp, Artificial
  synthetic DNA
gagcaagattatagttaggaagatagttaactcgc

SEQ ID NO: 2009 - DNA, 35 bp, Artificial
  synthetic DNA
tccggagtcgagcatatgtgaccaactctcaacgc

SEQ ID NO: 2010 - DNA, 35 bp, Artificial
  synthetic DNA
ggagctgcgatgccgttaccgacgtcatcttcaag

SEQ ID NO: 2011 - DNA, 35 bp, Artificial
  synthetic DNA
gctctatcttacacattggcgtactggactcgcga

SEQ ID NO: 2012 - DNA, 35 bp, Artificial
  synthetic DNA
ttctacatattcatcgcctaccgagttgcgcgaag

SEQ ID NO: 2013 - DNA, 35 bp, Artificial
  synthetic DNA
tggacgtctgacctgtgtctacatcggtggtgcta

SEQ ID NO: 2014 - DNA, 35 bp, Artificial
  synthetic DNA
ggcaggacagctccgtgttctactcgaaccgcact

SEQ ID NO: 2015 - DNA, 35 bp, Artificial
  synthetic DNA
tgacaacctcatgtctccgaccgcaggcatacaat

SEQ ID NO: 2016 - DNA, 35 bp, Artificial
  synthetic DNA
gcaggcctaacaagtggtcacgaggagtccttatt

SEQ ID NO: 2017 - DNA, 90 bp, Artificial
  synthetic DNA
cccatacacacaccatgaagcttgaactaattaacattctcaaactaattaacaagcatgcaagcatgtttttacacaatgacaatatat

SEQ ID NO: 2018 - DNA, 90 bp, Artificial
  synthetic DNA
atgggtgagggcgcagaggcaaagacatggaggtccggaagggtagaagctcacatcaagtcgagtatgttgaatgcaatcccatatata

SEQ ID NO: 2019 - DNA, 24 bp, Artificial
  synthetic DNA
cccatacacacaccatgaagcttg

SEQ ID NO: 2020 - DNA, 24 bp, Artificial
  synthetic DNA
ggtagaagctcacatcaagtcgag

SEQ ID NO: 2021 - DNA, 90 bp, Artificial
  synthetic DNA
aatcacagaacgaggtctggacgagaacagagctggacatctacacgcaccgcatggtagtagagcatgtactgcaaaagcttgaagcgc

SEQ ID NO: 2022 - DNA, 90 bp, Artificial
  synthetic DNA
gatgctgagggcgaagttgtcagccaagtcctcaatgtcataggcgagatcgcagtagttctgtaaccattccctgctaaactggtccat

SEQ ID NO: 2023 - DNA, 24 bp, Artificial
  synthetic DNA
acgagaacagagctggacatctac

SEQ ID NO: 2024 - DNA, 24 bp, Artificial
  synthetic DNA
tcaatgtcataggcgagatcgcag

SEQ ID NO: 2025 - DNA, 90 bp, Artificial
  synthetic DNA
agaccaacaagcagcaagtagtcagagaagtacaagagaaggagagcaagaaggatagtaagttgcaagcttaccgttacaaagatgata

SEQ ID NO: 2026 - DNA, 90 bp, Artificial
  synthetic DNA
ggaggagcacaactaggcgtttatcaagatgggtcatcgagctcttggtgtcttcaaccttcttgacatcaacttctccaatcttcgtct

SEQ ID NO: 2027 - DNA, 26 bp, Artificial
  synthetic DNA
ggagagcaagaaggatagtaagttgc

SEQ ID NO: 2028 - DNA, 25 bp, Artificial
  synthetic DNA
cgagctcttggtgtcttcaaccttc

SEQ ID NO: 2029 - DNA, 90 bp, Artificial
  synthetic DNA
tggggtagtcctgaagctctaggtatgcctcttcatctccctgcacctctggtgctagcacctcctgctcttcgggcacctctaccgggg

SEQ ID NO: 2030 - DNA, 90 bp, Artificial
  synthetic DNA
ggatactgatgtagctttcacccgggagtattccaaggtatcgattttccacggggaacgcgaagtgcactagttgaggtttagattgcc

SEQ ID NO: 2031 - DNA, 25 bp, Artificial
  synthetic DNA
gaagctctaggtatgcctcttcatc

SEQ ID NO: 2032 - DNA, 25 bp, Artificial
  synthetic DNA
gtgcactagttgaggtttagattgc

SEQ ID NO: 2033 - DNA, 90 bp, Artificial
  synthetic DNA
tcgggaaaacgaacgggcgaactacagatgtcagtacgaagtagtctatggcaggaaatacgtagtccatacgtggtgccagcccaagcc

SEQ ID NO: 2034 - DNA, 90 bp, Artificial
  synthetic DNA
agcaggagggagaaaggaaacgtggcattcatcggctgtctgccattgccatgtgagacaaggaaatctacttcacccccatctatcgag

SEQ ID NO: 2035 - DNA, 24 bp, Artificial
  synthetic DNA
gggcgaactacagatgtcagtacg

SEQ ID NO: 2036 - DNA, 24 bp, Artificial
  synthetic DNA
ctgtctgccattgccatgtgagac

SEQ ID NO: 2037 - DNA, 90 bp, Artificial
  synthetic DNA
agacataagattaactatgaacaaattcacgggtccgattcctttgggatttgcagcttgcaagaaccttcaaatactcattatatcttc

SEQ ID NO: 2038 - DNA, 90 bp, Artificial
  synthetic DNA
ttaagttgcagaatttgatacgaagaacttgaagcatggtgaggttgccgagctcattggggatggttccagaaaggctattgtagctta

SEQ ID NO: 2039 - DNA, 24 bp, Artificial
  synthetic DNA
gaacaaattcacgggtccgattcc

SEQ ID NO: 2040 - DNA, 24 bp, Artificial
  synthetic DNA
cgaagaacttgaagcatggtgagg

SEQ ID NO: 2041 - DNA, 60 bp, Artificial
  synthetic DNA
cacacaccatgaagcttgaactaattaacattctcaaactaattaacaagcatgcaagca

SEQ ID NO: 2042 - DNA, 60 bp, Artificial
  synthetic DNA
caagtcctcaatgtcataggcgagatcgcagtagttctgtaaccattccctgctaaactg

SEQ ID NO: 2043 - DNA, 60 bp, Artificial
  synthetic DNA
gtttatcaagatgggtcatcgagctcttggtgtcttcaaccttcttgacatcaacttctc

SEQ ID NO: 2044 - DNA, 50 bp, Artificial
  synthetic DNA
ctgaagctctaggtatgcctcttcatctccctgcacctctggtgctagca

SEQ ID NO: 2045 - DNA, 54 bp, Artificial
  synthetic DNA
ctgtctgccattgccatgtgagacaaggaaatctacttcacccccatctatcga

SEQ ID NO: 2046 - DNA, 60 bp, Artificial
  synthetic DNA
taagattaactatgaacaaattcacgggtccgattcctttgggatttgcagcttgcaaga